European Patent Specification EP 3 570 864 B1, published February 18, 2026. Title: PEPTIDE INHIBITORS OF INTERLEUKIN-23 RECEPTOR AND THEIR USE TO TREAT INFLAMMATORY DISEASES. Applicant: Protagonist Therapeutics, Inc. Bhandari, Ashok Bourne, Gregory Thomas. The sequence listing filed with the application follows.

SEQUENCE LISTING (310 sequences)

SEQ ID NO: 1 - protein, 13 aa, Artificial Sequence
  Synthesized peptide
  MOD_RES (1)..(1): D-form arginine
  MOD_RES (2)..(2): L-Penicillamine
  MISC_FEATURE (2)..(7): Residues 2 and 7 may be linked via a disulfide bond
  MOD_RES (7)..(7): L-Penicillamine
  MOD_RES (8)..(8): 4-(2-aminoethoxy)-L-phenylalanine
  MOD_RES (9)..(9): L-2-Napthylalanine
  MOD_RES (10)..(10): 4-amino-4-carboxy-tetrahydropyran
XXQTWQXXXXENN

SEQ ID NO: 2 - protein, 12 aa, Artificial Sequence
  Synthesized peptide
  MOD_RES (1)..(1): L-Penicillamine
  MISC_FEATURE (1)..(6): Residues 1 and 6 may be linked via a disulfide bond
  MOD_RES (6)..(6): L-Penicillamine
  MOD_RES (7)..(7): 4-(2-aminoethoxy)-L-phenylalanine
  MOD_RES (8)..(8): L-2-Napthylalanine
  MOD_RES (9)..(9): 4-amino-4-carboxy-tetrahydropyran
XNDWQXXXXENN

SEQ ID NO: 3 - protein, 12 aa, Artificial Sequence
  Synthesized peptide
  MOD_RES (1)..(1): L-Penicillamine
  MISC_FEATURE (1)..(6): Residues 1 and 6 may be linked via a disulfide bond
  MOD_RES (3)..(3): L-Diaminobutyric acid
  MOD_RES (6)..(6): L-Penicillamine
  MOD_RES (7)..(7): 4-(2-aminoethoxy)-L-phenylalanine
  MOD_RES (8)..(8): L-2-Napthylalanine
  MOD_RES (9)..(9): 4-amino-4-carboxy-tetrahydropyran
XNXWQXXXXENN

SEQ ID NO: 4 - protein, 12 aa, Artificial Sequence
  Synthesized peptide
  MOD_RES (1)..(1): L-Penicillamine
  MISC_FEATURE (1)..(6): Residues 1 and 6 may be linked via a disulfide bond
  MOD_RES (4)..(4): L-1-Napthylalanine
  MOD_RES (6)..(6): L-Penicillamine
  MOD_RES (7)..(7): 4-(2-aminoethoxy)-L-phenylalanine
  MOD_RES (8)..(8): L-2-Napthylalanine
  MOD_RES (9)..(9): 4-amino-4-carboxy-tetrahydropyran
  MOD_RES (10)..(10): ACETYLATION
XNTXQXXXXKNN

SEQ ID NO: 5 - protein, 12 aa, Artificial Sequence
  Synthesized peptide
  MOD_RES (1)..(1): L-Penicillamine
  MISC_FEATURE (1)..(6): Residues 1 and 6 may be linked via a disulfide bond
  MOD_RES (4)..(4): L-2-Napthylalanine
  MOD_RES (6)..(6): L-Penicillamine
  MOD_RES (7)..(7): 4-(2-aminoethoxy)-L-phenylalanine
  MOD_RES (8)..(8): L-2-Napthylalanine
  MOD_RES (9)..(9): 4-amino-4-carboxy-tetrahydropyran
  MOD_RES (10)..(10): ACETYLATION
XNTXQXXXXKNN

SEQ ID NO: 6 - protein, 12 aa, Artificial Sequence
  Synthesized peptide
  MOD_RES (1)..(1): L-Penicillamine
  MISC_FEATURE (1)..(6): Residues 1 and 6 may be linked via a disulfide bond
  MOD_RES (6)..(6): L-Penicillamine
  MOD_RES (7)..(7): 4-(2-aminoethoxy)-L-phenylalanine
  MOD_RES (8)..(8): L-2-Napthylalanine
  MOD_RES (9)..(9): 4-amino-4-carboxy-tetrahydropyran
  MOD_RES (10)..(10): ACETYLATION
XNTWEXXXXKNN

SEQ ID NO: 7 - protein, 12 aa, Artificial Sequence
  Synthesized peptide
  MOD_RES (1)..(1): L-Penicillamine
  MISC_FEATURE (1)..(6): Residues 1 and 6 may be linked via a disulfide bond
  MOD_RES (6)..(6): L-Penicillamine
  MOD_RES (7)..(7): 4-(2-aminoethoxy)-L-phenylalanine
  MOD_RES (8)..(8): L-2-Napthylalanine
  MOD_RES (9)..(9): 4-amino-4-carboxy-tetrahydropyran
  MOD_RES (10)..(10): ACETYLATION
XNTWFXXXXKNN

SEQ ID NO: 8 - protein, 12 aa, Artificial Sequence
  Synthesized peptide
  MOD_RES (1)..(1): L-Penicillamine
  MISC_FEATURE (1)..(6): Residues 1 and 6 may be linked via a disulfide bond
  MOD_RES (6)..(6): L-Penicillamine
  MOD_RES (7)..(7): 4-(2-aminoethoxy)-L-phenylalanine
  MOD_RES (9)..(9): 4-amino-4-carboxy-tetrahydropyran
  MOD_RES (10)..(10): ACETYLATION
XNTWQXXWXKNN

SEQ ID NO: 9 - protein, 12 aa, Artificial Sequence
  Synthesized peptide
  MOD_RES (1)..(1): L-Penicillamine
  MISC_FEATURE (1)..(6): Residues 1 and 6 may be linked via a disulfide bond
  MOD_RES (4)..(4): 5-Fluoro-L-tryptophan
  MOD_RES (6)..(6): L-Penicillamine
  MOD_RES (7)..(7): 4-(2-aminoethoxy)-L-phenylalanine
  MOD_RES (9)..(9): alpha-methyl-L-Leucine
  MOD_RES (10)..(10): ACETYLATION
XNTXQXXWXKNN

SEQ ID NO: 10 - protein, 13 aa, Artificial Sequence
  Synthesized peptide
  MOD_RES (1)..(1): L-Penicillamine
  MISC_FEATURE (1)..(6): Residues 1 and 6 may be linked via a disulfide bond
  MOD_RES (6)..(6): L-Penicillamine
  MOD_RES (7)..(7): 4-(2-aminoethoxy)-L-phenylalanine
  MOD_RES (8)..(8): L-2-Napthylalanine
  MOD_RES (9)..(9): alpha-methyl-L-Leucine
  MOD_RES (10)..(10): ACETYLATION
XNTWQXXXXKNNE

SEQ ID NO: 11 - protein, 13 aa, Artificial Sequence
  Synthesized peptide
  MOD_RES (1)..(1): L-Penicillamine
  MISC_FEATURE (1)..(6): Residues 1 and 6 may be linked via a disulfide bond
  MOD_RES (6)..(6): L-Penicillamine
  MOD_RES (7)..(7): 4-(2-aminoethoxy)-L-phenylalanine
  MOD_RES (8)..(8): L-2-Napthylalanine
  MOD_RES (9)..(9): alpha-methyl-L-Leucine
  MOD_RES (10)..(10): ACETYLATION
XNTWQXXXXKNNF

SEQ ID NO: 12 - protein, 13 aa, Artificial Sequence
  Synthesized peptide
  MOD_RES (1)..(1): L-Penicillamine
  MISC_FEATURE (1)..(6): Residues 1 and 6 may be linked via a disulfide bond
  MOD_RES (6)..(6): L-Penicillamine
  MOD_RES (7)..(7): 4-(2-aminoethoxy)-L-phenylalanine
  MOD_RES (8)..(8): L-2-Napthylalanine
  MOD_RES (9)..(9): alpha-methyl-L-Leucine
  MOD_RES (10)..(10): ACETYLATION
XNTWQXXXXKNNK

SEQ ID NO: 13 - protein, 13 aa, Artificial Sequence
  Synthesized peptide
  MOD_RES (1)..(1): L-Penicillamine
  MISC_FEATURE (1)..(6): Residues 1 and 6 may be linked via a disulfide bond
  MOD_RES (6)..(6): L-Penicillamine
  MOD_RES (7)..(7): 4-(2-aminoethoxy)-L-phenylalanine
  MOD_RES (8)..(8): L-2-Napthylalanine
  MOD_RES (9)..(9): alpha-methyl-L-Leucine
  MOD_RES (10)..(10): ACETYLATION
XNTWQXXXXKNNN

SEQ ID NO: 14 - protein, 13 aa, Artificial Sequence
  Synthesized peptide
  MOD_RES (1)..(1): L-Penicillamine
  MISC_FEATURE (1)..(6): Residues 1 and 6 may be linked via a disulfide bond
  MOD_RES (6)..(6): L-Penicillamine
  MOD_RES (7)..(7): 4-(2-aminoethoxy)-L-phenylalanine
  MOD_RES (8)..(8): L-2-Napthylalanine
  MOD_RES (9)..(9): alpha-methyl-L-Leucine
  MOD_RES (10)..(10): ACETYLATION
XNTWQXXXXKNNW

SEQ ID NO: 15 - protein, 13 aa, Artificial Sequence
  Synthesized peptide
  MOD_RES (1)..(1): L-Penicillamine
  MISC_FEATURE (1)..(6): Residues 1 and 6 may be linked via a disulfide bond
  MOD_RES (6)..(6): L-Penicillamine
  MOD_RES (7)..(7): 4-(2-aminoethoxy)-L-phenylalanine
  MOD_RES (8)..(8): L-2-Napthylalanine
  MOD_RES (9)..(9): alpha-methyl-L-Leucine
  MOD_RES (10)..(10): ACETYLATION
XNTWQXXXXKNNG

SEQ ID NO: 16 - protein, 13 aa, Artificial Sequence
  Synthesized peptide
  MOD_RES (1)..(1): L-Penicillamine
  MISC_FEATURE (1)..(6): Residues 1 and 6 may be linked via a disulfide bond
  MOD_RES (6)..(6): L-Penicillamine
  MOD_RES (7)..(7): 4-(2-aminoethoxy)-L-phenylalanine
  MOD_RES (8)..(8): L-2-Napthylalanine
  MOD_RES (9)..(9): alpha-methyl-L-Leucine
  MOD_RES (10)..(10): ACETYLATION
XNTWQXXXXKNNT

SEQ ID NO: 17 - protein, 14 aa, Artificial Sequence
  Synthesized peptide
  MOD_RES (1)..(1): L-Penicillamine
  MISC_FEATURE (1)..(6): Residues 1 and 6 may be linked via a disulfide bond
  MOD_RES (6)..(6): L-Penicillamine
  MOD_RES (7)..(7): 4-(2-aminoethoxy)-L-phenylalanine
  MOD_RES (8)..(8): L-2-Napthylalanine
  MOD_RES (9)..(9): alpha-methyl-L-Leucine
  MOD_RES (10)..(10): ACETYLATION
XNTWQXXXXKNNPK

SEQ ID NO: 18 - protein, 14 aa, Artificial Sequence
  Synthesized peptide
  MOD_RES (1)..(1): L-Penicillamine
  MISC_FEATURE (1)..(6): Residues 1 and 6 may be linked via a disulfide bond
  MOD_RES (6)..(6): L-Penicillamine
  MOD_RES (7)..(7): 4-(2-aminoethoxy)-L-phenylalanine
  MOD_RES (8)..(8): L-2-Napthylalanine
  MOD_RES (9)..(9): alpha-methyl-L-Leucine
  MOD_RES (10)..(10): ACETYLATION
XNTWQXXXXKNNPG

SEQ ID NO: 19 - protein, 14 aa, Artificial Sequence
  Synthesized peptide
  MOD_RES (1)..(1): L-Penicillamine
  MISC_FEATURE (1)..(6): Residues 1 and 6 may be linked via a disulfide bond
  MOD_RES (6)..(6): L-Penicillamine
  MOD_RES (7)..(7): 4-(2-aminoethoxy)-L-phenylalanine
  MOD_RES (8)..(8): L-2-Napthylalanine
  MOD_RES (9)..(9): alpha-methyl-L-Leucine
  MOD_RES (10)..(10): ACETYLATION
XNTWQXXXXKNNEP

SEQ ID NO: 20 - protein, 14 aa, Artificial Sequence
  Synthesized peptide
  MOD_RES (1)..(1): L-Penicillamine
  MISC_FEATURE (1)..(6): Residues 1 and 6 may be linked via a disulfide bond
  MOD_RES (6)..(6): L-Penicillamine
  MOD_RES (7)..(7): 4-(2-aminoethoxy)-L-phenylalanine
  MOD_RES (8)..(8): L-2-Napthylalanine
  MOD_RES (9)..(9): alpha-methyl-L-Leucine
  MOD_RES (10)..(10): ACETYLATION
XNTWQXXXXKNNGK

SEQ ID NO: 21 - protein, 14 aa, Artificial Sequence
  Synthesized peptide
  MOD_RES (1)..(1): L-Penicillamine
  MISC_FEATURE (1)..(6): Residues 1 and 6 may be linked via a disulfide bond
  MOD_RES (6)..(6): L-Penicillamine
  MOD_RES (7)..(7): 4-(2-aminoethoxy)-L-phenylalanine
  MOD_RES (8)..(8): L-2-Napthylalanine
  MOD_RES (9)..(9): alpha-methyl-L-Leucine
  MOD_RES (10)..(10): ACETYLATION
XNTWQXXXXKNNPT

SEQ ID NO: 22 - protein, 15 aa, Artificial Sequence
  Synthesized peptide
  MOD_RES (1)..(1): L-Penicillamine
  MISC_FEATURE (1)..(6): Residues 1 and 6 may be linked via a disulfide bond
  MOD_RES (6)..(6): L-Penicillamine
  MOD_RES (7)..(7): 4-(2-aminoethoxy)-L-phenylalanine
  MOD_RES (8)..(8): L-2-Napthylalanine
  MOD_RES (9)..(9): alpha-methyl-L-Leucine
  MOD_RES (10)..(10): ACETYLATION
XNTWQXXXXKNNKFG

SEQ ID NO: 23 - protein, 14 aa, Artificial Sequence
  Synthesized peptide
  MOD_RES (1)..(1): L-Penicillamine
  MISC_FEATURE (1)..(6): Residues 1 and 6 may be linked via a disulfide bond
  MOD_RES (6)..(6): L-Penicillamine
  MOD_RES (7)..(7): 4-(2-aminoethoxy)-L-phenylalanine
  MOD_RES (8)..(8): L-2-Napthylalanine
  MOD_RES (9)..(9): alpha-methyl-L-Leucine
  MOD_RES (10)..(10): ACETYLATION
XNTWQXXXXKNNGW

SEQ ID NO: 24 - protein, 14 aa, Artificial Sequence
  Synthesized peptide
  MOD_RES (1)..(1): L-Penicillamine
  MISC_FEATURE (1)..(6): Residues 1 and 6 may be linked via a disulfide bond
  MOD_RES (6)..(6): L-Penicillamine
  MOD_RES (7)..(7): 4-(2-aminoethoxy)-L-phenylalanine
  MOD_RES (8)..(8): L-2-Napthylalanine
  MOD_RES (9)..(9): alpha-methyl-L-Leucine
  MOD_RES (10)..(10): ACETYLATION
XNTWQXXXXKNNGQ

SEQ ID NO: 25 - protein, 15 aa, Artificial Sequence
  Synthesized peptide
  MOD_RES (1)..(1): L-Penicillamine
  MISC_FEATURE (1)..(6): Residues 1 and 6 may be linked via a disulfide bond
  MOD_RES (6)..(6): L-Penicillamine
  MOD_RES (7)..(7): 4-(2-aminoethoxy)-L-phenylalanine
  MOD_RES (8)..(8): L-2-Napthylalanine
  MOD_RES (9)..(9): alpha-methyl-L-Leucine
  MOD_RES (10)..(10): ACETYLATION
XNTWQXXXXKNNGGG

SEQ ID NO: 26 - protein, 15 aa, Artificial Sequence
  Synthesized peptide
  MOD_RES (1)..(1): L-Penicillamine
  MISC_FEATURE (1)..(6): Residues 1 and 6 may be linked via a disulfide bond
  MOD_RES (6)..(6): L-Penicillamine
  MOD_RES (7)..(7): 4-(2-aminoethoxy)-L-phenylalanine
  MOD_RES (8)..(8): L-2-Napthylalanine
  MOD_RES (9)..(9): alpha-methyl-L-Leucine
  MOD_RES (10)..(10): ACETYLATION
XNTWQXXXXKNNKKK

SEQ ID NO: 27 - protein, 15 aa, Artificial Sequence
  Synthesized peptide
  MOD_RES (1)..(1): L-Penicillamine
  MISC_FEATURE (1)..(6): Residues 1 and 6 may be linked via a disulfide bond
  MOD_RES (6)..(6): L-Penicillamine
  MOD_RES (7)..(7): 4-(2-aminoethoxy)-L-phenylalanine
  MOD_RES (8)..(8): L-2-Napthylalanine
  MOD_RES (9)..(9): alpha-methyl-L-Leucine
  MOD_RES (10)..(10): ACETYLATION
XNTWQXXXXKNNEEE

SEQ ID NO: 28 - protein, 15 aa, Artificial Sequence
  Synthesized peptide
  MOD_RES (1)..(1): L-Penicillamine
  MISC_FEATURE (1)..(6): Residues 1 and 6 may be linked via a disulfide bond
  MOD_RES (6)..(6): L-Penicillamine
  MOD_RES (7)..(7): 4-(2-aminoethoxy)-L-phenylalanine
  MOD_RES (8)..(8): L-2-Napthylalanine
  MOD_RES (9)..(9): alpha-methyl-L-Leucine
  MOD_RES (10)..(10): ACETYLATION
XNTWQXXXXKNNFFF

SEQ ID NO: 29 - protein, 15 aa, Artificial Sequence
  Synthesized peptide
  MOD_RES (1)..(1): L-Penicillamine
  MISC_FEATURE (1)..(6): Residues 1 and 6 may be linked via a disulfide bond
  MOD_RES (6)..(6): L-Penicillamine
  MOD_RES (7)..(7): 4-(2-aminoethoxy)-L-phenylalanine
  MOD_RES (8)..(8): L-2-Napthylalanine
  MOD_RES (9)..(9): alpha-methyl-L-Leucine
  MOD_RES (10)..(10): ACETYLATION
XNTWQXXXXKNNTTT

SEQ ID NO: 30 - protein, 16 aa, Artificial Sequence
  Synthesized peptide
  MOD_RES (1)..(1): L-Penicillamine
  MISC_FEATURE (1)..(6): Residues 1 and 6 may be linked via a disulfide bond
  MOD_RES (6)..(6): L-Penicillamine
  MOD_RES (7)..(7): 4-(2-aminoethoxy)-L-phenylalanine
  MOD_RES (8)..(8): L-2-Napthylalanine
  MOD_RES (9)..(9): alpha-methyl-L-Leucine
  MOD_RES (10)..(10): ACETYLATION
XNTWQXXXXKNNGGGR

SEQ ID NO: 31 - protein, 16 aa, Artificial Sequence
  Synthesized peptide
  MOD_RES (1)..(1): L-Penicillamine
  MISC_FEATURE (1)..(6): Residues 1 and 6 may be linked via a disulfide bond
  MOD_RES (6)..(6): L-Penicillamine
  MOD_RES (7)..(7): 4-(2-aminoethoxy)-L-phenylalanine
  MOD_RES (8)..(8): L-2-Napthylalanine
  MOD_RES (9)..(9): alpha-methyl-L-Leucine
  MOD_RES (10)..(10): ACETYLATION
XNTWQXXXXKNNGGGF

SEQ ID NO: 32 - protein, 16 aa, Artificial Sequence
  Synthesized peptide
  MOD_RES (1)..(1): L-Penicillamine
  MISC_FEATURE (1)..(6): Residues 1 and 6 may be linked via a disulfide bond
  MOD_RES (6)..(6): L-Penicillamine
  MOD_RES (7)..(7): 4-(2-aminoethoxy)-L-phenylalanine
  MOD_RES (8)..(8): L-2-Napthylalanine
  MOD_RES (9)..(9): alpha-methyl-L-Leucine
  MOD_RES (10)..(10): ACETYLATION
XNTWQXXXXKNNGGGE

SEQ ID NO: 33 - protein, 16 aa, Artificial Sequence
  Synthesized peptide
  MOD_RES (1)..(1): L-Penicillamine
  MISC_FEATURE (1)..(6): Residues 1 and 6 may be linked via a disulfide bond
  MOD_RES (6)..(6): L-Penicillamine
  MOD_RES (7)..(7): 4-(2-aminoethoxy)-L-phenylalanine
  MOD_RES (8)..(8): L-2-Napthylalanine
  MOD_RES (9)..(9): alpha-methyl-L-Leucine
  MOD_RES (10)..(10): ACETYLATION
XNTWQXXXXKNNGGGQ

SEQ ID NO: 34 - protein, 16 aa, Artificial Sequence
  Synthesized peptide
  MOD_RES (1)..(1): L-Penicillamine
  MISC_FEATURE (1)..(6): Residues 1 and 6 may be linked via a disulfide bond
  MOD_RES (6)..(6): L-Penicillamine
  MOD_RES (7)..(7): 4-(2-aminoethoxy)-L-phenylalanine
  MOD_RES (8)..(8): L-2-Napthylalanine
  MOD_RES (9)..(9): alpha-methyl-L-Leucine
  MOD_RES (10)..(10): ACETYLATION
XNTWQXXXXKNNGGGT

SEQ ID NO: 35 - protein, 17 aa, Artificial Sequence
  Synthesized peptide
  MOD_RES (1)..(1): L-Penicillamine
  MISC_FEATURE (1)..(6): Residues 1 and 6 may be linked via a disulfide bond
  MOD_RES (6)..(6): L-Penicillamine
  MOD_RES (7)..(7): 4-(2-aminoethoxy)-L-phenylalanine
  MOD_RES (8)..(8): L-2-Napthylalanine
  MOD_RES (9)..(9): alpha-methyl-L-Leucine
  MOD_RES (10)..(10): ACETYLATION
XNTWQXXXXKNNGGGGR

SEQ ID NO: 36 - protein, 17 aa, Artificial Sequence
  Synthesized peptide
  MOD_RES (1)..(1): L-Penicillamine
  MISC_FEATURE (1)..(6): Residues 1 and 6 may be linked via a disulfide bond
  MOD_RES (6)..(6): L-Penicillamine
  MOD_RES (7)..(7): 4-(2-aminoethoxy)-L-phenylalanine
  MOD_RES (8)..(8): L-2-Napthylalanine
  MOD_RES (9)..(9): alpha-methyl-L-Leucine
  MOD_RES (10)..(10): ACETYLATION
XNTWQXXXXKNNGGGGF

SEQ ID NO: 37 - protein, 17 aa, Artificial Sequence
  Synthesized peptide
  MOD_RES (1)..(1): L-Penicillamine
  MISC_FEATURE (1)..(6): Residues 1 and 6 may be linked via a disulfide bond
  MOD_RES (6)..(6): L-Penicillamine
  MOD_RES (7)..(7): 4-(2-aminoethoxy)-L-phenylalanine
  MOD_RES (8)..(8): L-2-Napthylalanine
  MOD_RES (9)..(9): alpha-methyl-L-Leucine
  MOD_RES (10)..(10): ACETYLATION
XNTWQXXXXKNNGGGGE

SEQ ID NO: 38 - protein, 17 aa, Artificial Sequence
  Synthesized peptide
  MOD_RES (1)..(1): L-Penicillamine
  MISC_FEATURE (1)..(6): Residues 1 and 6 may be linked via a disulfide bond
  MOD_RES (6)..(6): L-Penicillamine
  MOD_RES (7)..(7): 4-(2-aminoethoxy)-L-phenylalanine
  MOD_RES (8)..(8): L-2-Napthylalanine
  MOD_RES (9)..(9): alpha-methyl-L-Leucine
  MOD_RES (10)..(10): ACETYLATION
XNTWQXXXXKNNGGGGQ

SEQ ID NO: 39 - protein, 17 aa, Artificial Sequence
  Synthesized peptide
  MOD_RES (1)..(1): L-Penicillamine
  MISC_FEATURE (1)..(6): Residues 1 and 6 may be linked via a disulfide bond
  MOD_RES (6)..(6): L-Penicillamine
  MOD_RES (7)..(7): 4-(2-aminoethoxy)-L-phenylalanine
  MOD_RES (8)..(8): L-2-Napthylalanine
  MOD_RES (9)..(9): alpha-methyl-L-Leucine
  MOD_RES (10)..(10): ACETYLATION
XNTWQXXXXKNNGGGGT

SEQ ID NO: 40 - protein, 17 aa, Artificial Sequence
  Synthesized peptide
  MOD_RES (1)..(1): L-Penicillamine
  MISC_FEATURE (1)..(6): Residues 1 and 6 may be linked via a disulfide bond
  MOD_RES (6)..(6): L-Penicillamine
  MOD_RES (7)..(7): 4-(2-aminoethoxy)-L-phenylalanine
  MOD_RES (8)..(8): L-2-Napthylalanine
  MOD_RES (9)..(9): alpha-methyl-L-Leucine
  MOD_RES (10)..(10): ACETYLATION
XNTWQXXXXKNNRRRRR

SEQ ID NO: 41 - protein, 17 aa, Artificial Sequence
  Synthesized peptide
  MOD_RES (1)..(1): L-Penicillamine
  MISC_FEATURE (1)..(6): Residues 1 and 6 may be linked via a disulfide bond
  MOD_RES (6)..(6): L-Penicillamine
  MOD_RES (7)..(7): 4-(2-aminoethoxy)-L-phenylalanine
  MOD_RES (8)..(8): L-2-Napthylalanine
  MOD_RES (9)..(9): alpha-methyl-L-Leucine
  MOD_RES (10)..(10): ACETYLATION
XNTWQXXXXKNNFFFFF

SEQ ID NO: 42 - protein, 17 aa, Artificial Sequence
  Synthesized peptide
  MOD_RES (1)..(1): L-Penicillamine
  MISC_FEATURE (1)..(6): Residues 1 and 6 may be linked via a disulfide bond
  MOD_RES (6)..(6): L-Penicillamine
  MOD_RES (7)..(7): 4-(2-aminoethoxy)-L-phenylalanine
  MOD_RES (8)..(8): L-2-Napthylalanine
  MOD_RES (9)..(9): alpha-methyl-L-Leucine
  MOD_RES (10)..(10): ACETYLATION
XNTWQXXXXKNNEEEEE

SEQ ID NO: 43 - protein, 17 aa, Artificial Sequence
  Synthesized peptide
  MOD_RES (1)..(1): L-Penicillamine
  MISC_FEATURE (1)..(6): Residues 1 and 6 may be linked via a disulfide bond
  MOD_RES (6)..(6): L-Penicillamine
  MOD_RES (7)..(7): 4-(2-aminoethoxy)-L-phenylalanine
  MOD_RES (8)..(8): L-2-Napthylalanine
  MOD_RES (9)..(9): alpha-methyl-L-Leucine
  MOD_RES (10)..(10): ACETYLATION
XNTWQXXXXKNNQQQQQ

SEQ ID NO: 44 - protein, 17 aa, Artificial Sequence
  Synthesized peptide
  MOD_RES (1)..(1): L-Penicillamine
  MISC_FEATURE (1)..(6): Residues 1 and 6 may be linked via a disulfide bond
  MOD_RES (6)..(6): L-Penicillamine
  MOD_RES (7)..(7): 4-(2-aminoethoxy)-L-phenylalanine
  MOD_RES (8)..(8): L-2-Napthylalanine
  MOD_RES (9)..(9): alpha-methyl-L-Leucine
  MOD_RES (10)..(10): ACETYLATION
XNTWQXXXXKNNTTTTT

SEQ ID NO: 45 - protein, 15 aa, Artificial Sequence
  Synthesized peptide
  MOD_RES (4)..(4): L-Penicillamine
  MISC_FEATURE (4)..(9): Residues 1 and 6 may be linked via a disulfide bond
  MOD_RES (9)..(9): L-Penicillamine
  MOD_RES (10)..(10): 4-(2-aminoethoxy)-L-phenylalanine
  MOD_RES (11)..(11): L-2-Napthylalanine
  MOD_RES (12)..(12): alpha-methyl-L-Leucine
  MOD_RES (13)..(13): ACETYLATION
GGGXNTWQXXXXKNN

SEQ ID NO: 46 - protein, 15 aa, Artificial Sequence
  Synthesized peptide
  MOD_RES (4)..(4): L-Penicillamine
  MISC_FEATURE (4)..(9): Residues 1 and 6 may be linked via a disulfide bond
  MOD_RES (9)..(9): L-Penicillamine
  MOD_RES (10)..(10): 4-(2-aminoethoxy)-L-phenylalanine
  MOD_RES (11)..(11): L-2-Napthylalanine
  MOD_RES (12)..(12): alpha-methyl-L-Leucine
  MOD_RES (13)..(13): ACETYLATION
RRRXNTWQXXXXKNN

SEQ ID NO: 47 - protein, 15 aa, Artificial Sequence
  Synthesized peptide
  MOD_RES (4)..(4): L-Penicillamine
  MISC_FEATURE (4)..(9): Residues 1 and 6 may be linked via a disulfide bond
  MOD_RES (9)..(9): L-Penicillamine
  MOD_RES (10)..(10): 4-(2-aminoethoxy)-L-phenylalanine
  MOD_RES (11)..(11): L-2-Napthylalanine
  MOD_RES (12)..(12): alpha-methyl-L-Leucine
  MOD_RES (13)..(13): ACETYLATION
FFFXNTWQXXXXKNN

SEQ ID NO: 48 - protein, 15 aa, Artificial Sequence
  Synthesized peptide
  MOD_RES (4)..(4): L-Penicillamine
  MISC_FEATURE (4)..(9): Residues 1 and 6 may be linked via a disulfide bond
  MOD_RES (9)..(9): L-Penicillamine
  MOD_RES (10)..(10): 4-(2-aminoethoxy)-L-phenylalanine
  MOD_RES (11)..(11): L-2-Napthylalanine
  MOD_RES (12)..(12): alpha-methyl-L-Leucine
  MOD_RES (13)..(13): ACETYLATION
EEEXNTWQXXXXKNN

SEQ ID NO: 49 - protein, 15 aa, Artificial Sequence
  Synthesized peptide
  MOD_RES (4)..(4): L-Penicillamine
  MISC_FEATURE (4)..(9): Residues 1 and 6 may be linked via a disulfide bond
  MOD_RES (9)..(9): L-Penicillamine
  MOD_RES (10)..(10): 4-(2-aminoethoxy)-L-phenylalanine
  MOD_RES (11)..(11): L-2-Napthylalanine
  MOD_RES (12)..(12): alpha-methyl-L-Leucine
  MOD_RES (13)..(13): ACETYLATION
QQQXNTWQXXXXKNN

SEQ ID NO: 50 - protein, 15 aa, Artificial Sequence
  Synthesized peptide
  MOD_RES (4)..(4): L-Penicillamine
  MISC_FEATURE (4)..(9): Residues 1 and 6 may be linked via a disulfide bond
  MOD_RES (9)..(9): L-Penicillamine
  MOD_RES (10)..(10): 4-(2-aminoethoxy)-L-phenylalanine
  MOD_RES (11)..(11): L-2-Napthylalanine
  MOD_RES (12)..(12): alpha-methyl-L-Leucine
  MOD_RES (13)..(13): ACETYLATION
TTTXNTWQXXXXKNN

SEQ ID NO: 51 - protein, 14 aa, Artificial Sequence
  Synthesized peptide
  MOD_RES (3)..(3): L-Penicillamine
  MISC_FEATURE (3)..(8): Residues 1 and 6 may be linked via a disulfide bond
  MOD_RES (8)..(8): L-Penicillamine
  MOD_RES (9)..(9): 4-(2-aminoethoxy)-L-phenylalanine
  MOD_RES (10)..(10): L-2-Napthylalanine
  MOD_RES (11)..(11): alpha-methyl-L-Leucine
  MOD_RES (12)..(12): ACETYLATION
RGXNTWQXXXXKNN

SEQ ID NO: 52 - protein, 14 aa, Artificial Sequence
  Synthesized peptide
  MOD_RES (3)..(3): L-Penicillamine
  MISC_FEATURE (3)..(8): Residues 1 and 6 may be linked via a disulfide bond
  MOD_RES (8)..(8): L-Penicillamine
  MOD_RES (9)..(9): 4-(2-aminoethoxy)-L-phenylalanine
  MOD_RES (10)..(10): L-2-Napthylalanine
  MOD_RES (11)..(11): alpha-methyl-L-Leucine
  MOD_RES (12)..(12): ACETYLATION
FGXNTWQXXXXKNN

SEQ ID NO: 53 - protein, 14 aa, Artificial Sequence
  Synthesized peptide
  MOD_RES (3)..(3): L-Penicillamine
  MISC_FEATURE (3)..(8): Residues 1 and 6 may be linked via a disulfide bond
  MOD_RES (8)..(8): L-Penicillamine
  MOD_RES (9)..(9): 4-(2-aminoethoxy)-L-phenylalanine
  MOD_RES (10)..(10): L-2-Napthylalanine
  MOD_RES (11)..(11): alpha-methyl-L-Leucine
  MOD_RES (12)..(12): ACETYLATION
EGXNTWQXXXXKNN

SEQ ID NO: 54 - protein, 14 aa, Artificial Sequence
  Synthesized peptide
  MOD_RES (3)..(3): L-Penicillamine
  MISC_FEATURE (3)..(8): Residues 1 and 6 may be linked via a disulfide bond
  MOD_RES (8)..(8): L-Penicillamine
  MOD_RES (9)..(9): 4-(2-aminoethoxy)-L-phenylalanine
  MOD_RES (10)..(10): L-2-Napthylalanine
  MOD_RES (11)..(11): alpha-methyl-L-Leucine
  MOD_RES (12)..(12): ACETYLATION
QGXNTWQXXXXKNN

SEQ ID NO: 55 - protein, 14 aa, Artificial Sequence
  Synthesized peptide
  MOD_RES (3)..(3): L-Penicillamine
  MISC_FEATURE (3)..(8): Residues 1 and 6 may be linked via a disulfide bond
  MOD_RES (8)..(8): L-Penicillamine
  MOD_RES (9)..(9): 4-(2-aminoethoxy)-L-phenylalanine
  MOD_RES (10)..(10): L-2-Napthylalanine
  MOD_RES (11)..(11): alpha-methyl-L-Leucine
  MOD_RES (12)..(12): ACETYLATION
TGXNTWQXXXXKNN

SEQ ID NO: 56 - protein, 12 aa, Artificial Sequence
  Synthesized peptide
  MOD_RES (1)..(1): L-Penicillamine
  MISC_FEATURE (1)..(6): Residues 1 and 6 may be linked via a disulfide bond
  MOD_RES (6)..(6): L-Penicillamine
  MOD_RES (7)..(7): 4-(2-aminoethoxy)-L-phenylalanine
  MOD_RES (8)..(8): L-2-Napthylalanine
  MOD_RES (9)..(9): alpha-methyl-L-Leucine
  MOD_RES (10)..(10): Palmityl conjugation
XNTWQXXXXKNN

SEQ ID NO: 57 - protein, 12 aa, Artificial Sequence
  Synthesized peptide
  MOD_RES (1)..(1): L-Penicillamine
  MISC_FEATURE (1)..(6): Residues 1 and 6 may be linked via a disulfide bond
  MOD_RES (6)..(6): L-Penicillamine
  MOD_RES (7)..(7): 4-(2-aminoethoxy)-L-phenylalanine
  MOD_RES (8)..(8): L-2-Napthylalanine
  MOD_RES (9)..(9): alpha-methyl-L-Leucine
  MOD_RES (10)..(10): IsoGlu-Palmityl conjugation
XNTWQXXXXKNN

SEQ ID NO: 58 - protein, 12 aa, Artificial Sequence
  Synthesized peptide
  MOD_RES (1)..(1): L-Penicillamine
  MISC_FEATURE (1)..(6): Residues 1 and 6 may be linked via a disulfide bond
  MOD_RES (6)..(6): L-Penicillamine
  MOD_RES (7)..(7): 4-(2-aminoethoxy)-L-phenylalanine
  MOD_RES (8)..(8): L-2-Napthylalanine
  MOD_RES (9)..(9): alpha-methyl-L-Leucine
  MOD_RES (10)..(10): PEG11-Palmityl conjugation
XNTWQXXXXKNN

SEQ ID NO: 59 - protein, 12 aa, Artificial Sequence
  Synthesized peptide
  MOD_RES (1)..(1): L-Penicillamine
  MISC_FEATURE (1)..(6): Residues 1 and 6 may be linked via a disulfide bond
  MOD_RES (6)..(6): L-Penicillamine
  MOD_RES (7)..(7): 4-(2-aminoethoxy)-L-phenylalanine
  MOD_RES (8)..(8): L-2-Napthylalanine
  MOD_RES (9)..(9): alpha-methyl-L-Leucine
  MOD_RES (10)..(10): 6-aminohexanoic acid - Palmityl conjugation
XNTWQXXXXKNN

SEQ ID NO: 60 - protein, 12 aa, Artificial Sequence
  Synthesized peptide
  MOD_RES (1)..(1): L-Penicillamine
  MISC_FEATURE (1)..(6): Residues 1 and 6 may be linked via a disulfide bond
  MOD_RES (6)..(6): L-Penicillamine
  MOD_RES (7)..(7): 4-(2-aminoethoxy)-L-phenylalanine
  MOD_RES (8)..(8): L-2-Napthylalanine
  MOD_RES (9)..(9): alpha-methyl-L-Leucine
  MOD_RES (10)..(10): IsoGlu - 6-aminohexanoic acid - Palmityl conjugation
XNTWQXXXXKNN

SEQ ID NO: 61 - protein, 12 aa, Artificial Sequence
  Synthesized peptide
  MOD_RES (1)..(1): L-Penicillamine with a palmityl conjugation
  MISC_FEATURE (1)..(6): Residues 1 and 6 may be linked via a disulfide bond
  MOD_RES (6)..(6): L-Penicillamine
  MOD_RES (7)..(7): 4-(2-aminoethoxy)-L-phenylalanine
  MOD_RES (8)..(8): L-2-Napthylalanine
  MOD_RES (9)..(9): alpha-methyl-L-Leucine
  MOD_RES (10)..(10): ACETYLATION
XNTWQXXXXKNN

SEQ ID NO: 62 - protein, 12 aa, Artificial Sequence
  Synthesized peptide
  MOD_RES (1)..(1): L-Penicillamine
  MOD_RES (1)..(1): Palmityl - IsoGlu conjugation
  MISC_FEATURE (1)..(6): Residues 1 and 6 may be linked via a disulfide bond
  MOD_RES (6)..(6): L-Penicillamine
  MOD_RES (7)..(7): 4-(2-aminoethoxy)-L-phenylalanine
  MOD_RES (8)..(8): L-2-Napthylalanine
  MOD_RES (9)..(9): alpha-methyl-L-Leucine
  MOD_RES (10)..(10): ACETYLATION
XNTWQXXXXKNN

SEQ ID NO: 63 - protein, 12 aa, Artificial Sequence
  Synthesized peptide
  MOD_RES (1)..(1): L-Penicillamine
  MOD_RES (1)..(1): Palmityl - PEG11
  MISC_FEATURE (1)..(6): Residues 1 and 6 may be linked via a disulfide bond
  MOD_RES (6)..(6): L-Penicillamine
  MOD_RES (7)..(7): 4-(2-aminoethoxy)-L-phenylalanine
  MOD_RES (8)..(8): L-2-Napthylalanine
  MOD_RES (9)..(9): alpha-methyl-L-Leucine
  MOD_RES (10)..(10): ACETYLATION
XNTWQXXXXKNN

SEQ ID NO: 64 - protein, 12 aa, Artificial Sequence
  Synthesized peptide
  MOD_RES (1)..(1): L-Penicillamine
  MOD_RES (1)..(1): Palmityl - 6-aminohexanoic acid
  MISC_FEATURE (1)..(6): Residues 1 and 6 may be linked via a disulfide bond
  MOD_RES (6)..(6): L-Penicillamine
  MOD_RES (7)..(7): 4-(2-aminoethoxy)-L-phenylalanine
  MOD_RES (8)..(8): L-2-Napthylalanine
  MOD_RES (9)..(9): alpha-methyl-L-Leucine
  MOD_RES (10)..(10): ACETYLATION
XNTWQXXXXKNN

SEQ ID NO: 65 - protein, 12 aa, Artificial Sequence
  Synthesized peptide
  MOD_RES (1)..(1): L-Penicillamine
  MOD_RES (1)..(1): Palmityl - 6-aminohexanoic acid - IsoGlu conjugation
  MISC_FEATURE (1)..(6): Residues 1 and 6 may be linked via a disulfide bond
  MOD_RES (6)..(6): L-Penicillamine
  MOD_RES (7)..(7): 4-(2-aminoethoxy)-L-phenylalanine
  MOD_RES (8)..(8): L-2-Napthylalanine
  MOD_RES (9)..(9): alpha-methyl-L-Leucine
  MOD_RES (10)..(10): ACETYLATION
XNTWQXXXXKNN

SEQ ID NO: 66 - protein, 13 aa, Artificial Sequence
  Synthesized peptide
  MOD_RES (1)..(1): L-Penicillamine
  MISC_FEATURE (1)..(6): Residues 1 and 6 may be linked via a disulfide bond
  MOD_RES (6)..(6): L-Penicillamine
  MOD_RES (7)..(7): 4-(2-aminoethoxy)-L-phenylalanine
  MOD_RES (8)..(8): L-2-Napthylalanine
  MOD_RES (9)..(9): alpha-methyl-L-Leucine
  MOD_RES (10)..(10): ACETYLATION
  MOD_RES (13)..(13): Palmityl conjugation
XNTWQXXXXKNNK

SEQ ID NO: 67 - protein, 13 aa, Artificial Sequence
  Synthesized peptide
  MOD_RES (1)..(1): L-Penicillamine
  MISC_FEATURE (1)..(6): Residues 1 and 6 may be linked via a disulfide bond
  MOD_RES (6)..(6): L-Penicillamine
  MOD_RES (7)..(7): 4-(2-aminoethoxy)-L-phenylalanine
  MOD_RES (8)..(8): L-2-Napthylalanine
  MOD_RES (9)..(9): alpha-methyl-L-Leucine
  MOD_RES (10)..(10): ACETYLATION
  MOD_RES (13)..(13): IsoGlu - Palmityl conjugation
XNTWQXXXXKNNK

SEQ ID NO: 68 - protein, 13 aa, Artificial Sequence
  Synthesized peptide
  MOD_RES (1)..(1): L-Penicillamine
  MISC_FEATURE (1)..(6): Residues 1 and 6 may be linked via a disulfide bond
  MOD_RES (6)..(6): L-Penicillamine
  MOD_RES (7)..(7): 4-(2-aminoethoxy)-L-phenylalanine
  MOD_RES (8)..(8): L-2-Napthylalanine
  MOD_RES (9)..(9): alpha-methyl-L-Leucine
  MOD_RES (10)..(10): ACETYLATION
  MOD_RES (13)..(13): PEG11 - Palmityl conjugation
XNTWQXXXXKNNK

SEQ ID NO: 69 - protein, 13 aa, Artificial Sequence
  Synthesized peptide
  MOD_RES (1)..(1): L-Penicillamine
  MISC_FEATURE (1)..(6): Residues 1 and 6 may be linked via a disulfide bond
  MOD_RES (6)..(6): L-Penicillamine
  MOD_RES (7)..(7): 4-(2-aminoethoxy)-L-phenylalanine
  MOD_RES (8)..(8): L-2-Napthylalanine
  MOD_RES (9)..(9): alpha-methyl-L-Leucine
  MOD_RES (10)..(10): ACETYLATION
  MOD_RES (13)..(13): 6-aminohexanoic acid - Palmityl conjugation
XNTWQXXXXKNNK

SEQ ID NO: 70 - protein, 13 aa, Artificial Sequence
  Synthesized peptide
  MOD_RES (1)..(1): L-Penicillamine
  MISC_FEATURE (1)..(6): Residues 1 and 6 may be linked via a disulfide bond
  MOD_RES (6)..(6): L-Penicillamine
  MOD_RES (7)..(7): 4-(2-aminoethoxy)-L-phenylalanine
  MOD_RES (8)..(8): L-2-Napthylalanine
  MOD_RES (9)..(9): alpha-methyl-L-Leucine
  MOD_RES (10)..(10): ACETYLATION
  MOD_RES (13)..(13): IsoGlu - 6-aminohexanoic acid - Palmityl conjugation
XNTWQXXXXKNNK

SEQ ID NO: 71 - protein, 13 aa, Artificial Sequence
  Synthesized peptide
  MOD_RES (1)..(1): D-form arginine
  MOD_RES (1)..(1): Alexa488 - PEG4 conjugation
  MOD_RES (2)..(2): Abu
  MISC_FEATURE (2)..(7): residues cyclosized
  MOD_RES (8)..(8): 4-(2-aminoethoxy)-L-phenylalanine
  MOD_RES (9)..(9): L-2-Napthylalanine
  MOD_RES (10)..(10): 4-amino-4-carboxy-tetrahydropyran
XXQTWQCXXXENN

SEQ ID NO: 72 - protein, 13 aa, Artificial Sequence
  Synthesized peptide
  MOD_RES (1)..(1): D-form arginine
  MOD_RES (1)..(1): Alexa647 - PEG4 conjugation
  MOD_RES (2)..(2): Abu
  MISC_FEATURE (2)..(7): residues cyclosized
  MOD_RES (8)..(8): 4-(2-aminoethoxy)-L-phenylalanine
  MOD_RES (9)..(9): L-2-Napthylalanine
  MOD_RES (10)..(10): 4-amino-4-carboxy-tetrahydropyran
XXQTWQCXXXENN

SEQ ID NO: 73 - protein, 13 aa, Artificial Sequence
  Synthesized peptide
  MOD_RES (1)..(1): D-form arginine
  MOD_RES (2)..(2): Abu
  MISC_FEATURE (2)..(7): residues cyclosized
  MOD_RES (8)..(8): 4-(2-aminoethoxy)-L-phenylalanine
  MOD_RES (9)..(9): L-2-Napthylalanine
  MOD_RES (10)..(10): 4-amino-4-carboxy-tetrahydropyran
XXQTWQCXXXEND

SEQ ID NO: 74 - protein, 13 aa, Artificial Sequence
  Synthesized peptide
  MOD_RES (1)..(1): D-form arginine
  MOD_RES (2)..(2): Abu
  MISC_FEATURE (2)..(7): residues cyclosized
  MOD_RES (8)..(8): 4-(2-aminoethoxy)-L-phenylalanine
  MOD_RES (9)..(9): L-2-Napthylalanine
  MOD_RES (10)..(10): 4-amino-4-carboxy-tetrahydropyran
XXQTWQCXXXEDN

SEQ ID NO: 75 - protein, 13 aa, Artificial Sequence
  Synthesized peptide
  MOD_RES (1)..(1): D-form arginine
  MOD_RES (2)..(2): Abu
  MISC_FEATURE (2)..(7): residues cyclosized
  MOD_RES (8)..(8): 4-(2-aminoethoxy)-L-phenylalanine
  MOD_RES (9)..(9): L-2-Napthylalanine
  MOD_RES (10)..(10): 4-amino-4-carboxy-tetrahydropyran
XXQTWECXXXENN

SEQ ID NO: 76 - protein, 13 aa, Artificial Sequence
  Synthesized peptide
  MOD_RES (1)..(1): D-form arginine
  MOD_RES (2)..(2): Abu
  MISC_FEATURE (2)..(7): residues cyclosized
  MOD_RES (8)..(8): 4-(2-aminoethoxy)-L-phenylalanine
  MOD_RES (9)..(9): L-2-Napthylalanine
  MOD_RES (10)..(10): 4-amino-4-carboxy-tetrahydropyran
XXETWQCXXXENN

SEQ ID NO: 77 - protein, 13 aa, Artificial Sequence
  Synthesized peptide
  MOD_RES (1)..(1): D-form arginine
  MOD_RES (2)..(2): Abu
  MISC_FEATURE (2)..(7): residues cyclosized
  MOD_RES (8)..(8): 4-(2-aminoethoxy)-L-phenylalanine
  MOD_RES (9)..(9): L-2-Napthylalanine
  MOD_RES (10)..(10): 4-amino-4-carboxy-tetrahydropyran
XXQTWQCXXXEDD

SEQ ID NO: 78 - protein, 13 aa, Artificial Sequence
  Synthesized peptide
  MOD_RES (1)..(1): D-form arginine
  MOD_RES (2)..(2): Abu
  MISC_FEATURE (2)..(7): residues cyclosized
  MOD_RES (8)..(8): 4-(2-aminoethoxy)-L-phenylalanine
  MOD_RES (9)..(9): L-2-Napthylalanine
  MOD_RES (10)..(10): 4-amino-4-carboxy-tetrahydropyran
XXQTWECXXXEND

SEQ ID NO: 79 - protein, 13 aa, Artificial Sequence
  Synthesized peptide
  MOD_RES (1)..(1): D-form arginine
  MOD_RES (2)..(2): Abu
  MISC_FEATURE (2)..(7): residues cyclosized
  MOD_RES (8)..(8): 4-(2-aminoethoxy)-L-phenylalanine
  MOD_RES (9)..(9): L-2-Napthylalanine
  MOD_RES (10)..(10): 4-amino-4-carboxy-tetrahydropyran
XXETWQCXXXEND

SEQ ID NO: 80 - protein, 13 aa, Artificial Sequence
  Synthesized peptide
  MOD_RES (1)..(1): D-form arginine
  MOD_RES (2)..(2): Abu
  MISC_FEATURE (2)..(7): residues cyclosized
  MOD_RES (8)..(8): 4-(2-aminoethoxy)-L-phenylalanine
  MOD_RES (9)..(9): L-2-Napthylalanine
  MOD_RES (10)..(10): 4-amino-4-carboxy-tetrahydropyran
XXQTWECXXXEDN

SEQ ID NO: 81 - protein, 13 aa, Artificial Sequence
  Synthesized peptide
  MOD_RES (1)..(1): D-form arginine
  MOD_RES (2)..(2): Abu
  MISC_FEATURE (2)..(7): residues cyclosized
  MOD_RES (8)..(8): 4-(2-aminoethoxy)-L-phenylalanine
  MOD_RES (9)..(9): L-2-Napthylalanine
  MOD_RES (10)..(10): 4-amino-4-carboxy-tetrahydropyran
XXETWQCXXXEDN

SEQ ID NO: 82 - protein, 13 aa, Artificial Sequence
  Synthesized peptide
  MOD_RES (1)..(1): D-form arginine
  MOD_RES (2)..(2): Abu
  MISC_FEATURE (2)..(7): residues cyclosized
  MOD_RES (8)..(8): 4-(2-aminoethoxy)-L-phenylalanine
  MOD_RES (9)..(9): L-2-Napthylalanine
  MOD_RES (10)..(10): 4-amino-4-carboxy-tetrahydropyran
XXETWECXXXENN

SEQ ID NO: 83 - protein, 13 aa, Artificial Sequence
  Synthesized peptide
  MOD_RES (1)..(1): D-form arginine
  MOD_RES (2)..(2): Abu
  MISC_FEATURE (2)..(7): residues cyclosized
  MOD_RES (8)..(8): 4-(2-aminoethoxy)-L-phenylalanine
  MOD_RES (9)..(9): L-2-Napthylalanine
  MOD_RES (10)..(10): 4-amino-4-carboxy-tetrahydropyran
XXQTWQCXXXENN

SEQ ID NO: 84 - protein, 13 aa, Artificial Sequence
  Synthesized peptide
  MOD_RES (1)..(1): D-form arginine
  MOD_RES (2)..(2): Abu
  MISC_FEATURE (2)..(7): residues cyclosized
  MOD_RES (8)..(8): 4-(2-aminoethoxy)-L-phenylalanine
  MOD_RES (9)..(9): L-2-Napthylalanine
  MOD_RES (10)..(10): 4-amino-4-carboxy-tetrahydropyran
XXQTWQCXXXEND

SEQ ID NO: 85 - protein, 13 aa, Artificial Sequence
  Synthesized peptide
  MOD_RES (1)..(1): D-form arginine
  MOD_RES (2)..(2): Abu
  MISC_FEATURE (2)..(7): residues cyclosized
  MOD_RES (8)..(8): 4-(2-aminoethoxy)-L-phenylalanine
  MOD_RES (9)..(9): L-2-Napthylalanine
  MOD_RES (10)..(10): 4-amino-4-carboxy-tetrahydropyran
XXQTWQCXXXEDN

SEQ ID NO: 86 - protein, 13 aa, Artificial Sequence
  Synthesized peptide
  MOD_RES (1)..(1): D-form arginine
  MOD_RES (2)..(2): Abu
  MISC_FEATURE (2)..(7): residues cyclosized
  MOD_RES (8)..(8): 4-(2-aminoethoxy)-L-phenylalanine
  MOD_RES (9)..(9): L-2-Napthylalanine
  MOD_RES (10)..(10): 4-amino-4-carboxy-tetrahydropyran
XXQTWECXXXENN

SEQ ID NO: 87 - protein, 13 aa, Artificial Sequence
  Synthesized peptide
  MOD_RES (1)..(1): D-form arginine
  MOD_RES (2)..(2): Abu
  MISC_FEATURE (2)..(7): residues cyclosized
  MOD_RES (8)..(8): 4-(2-aminoethoxy)-L-phenylalanine
  MOD_RES (9)..(9): L-2-Napthylalanine
  MOD_RES (10)..(10): 4-amino-4-carboxy-tetrahydropyran
XXETWQCXXXENN

SEQ ID NO: 88 - protein, 13 aa, Artificial Sequence
  Synthesized peptide
  MOD_RES (1)..(1): D-form arginine
  MOD_RES (1)..(1): PEG4 conjugation
  MOD_RES (2)..(2): Abu
  MISC_FEATURE (2)..(7): residues cyclosized
  MOD_RES (8)..(8): 4-(2-aminoethoxy)-L-phenylalanine
  MOD_RES (9)..(9): L-2-Napthylalanine
  MOD_RES (10)..(10): 4-amino-4-carboxy-tetrahydropyran
XXETWQCXXXENN

SEQ ID NO: 89 - protein, 13 aa, Artificial Sequence
  Synthesized peptide
  MOD_RES (1)..(1): D-form arginine
  MOD_RES (1)..(1): Biotin - PEG4 conjugation
  MOD_RES (2)..(2): Abu
  MISC_FEATURE (2)..(7): residues cyclosized
  MOD_RES (8)..(8): 4-(2-aminoethoxy)-L-phenylalanine
  MOD_RES (9)..(9): L-2-Napthylalanine
  MOD_RES (10)..(10): 4-amino-4-carboxy-tetrahydropyran
XXETWQCXXXENN

SEQ ID NO: 90 - protein, 13 aa, Artificial Sequence
  Synthesized peptide
  MOD_RES (1)..(1): D-form arginine
  MOD_RES (1)..(1): PEG4 conjugation
  MOD_RES (2)..(2): Abu
  MISC_FEATURE (2)..(7): residues cyclosized
  MOD_RES (8)..(8): 4-(2-aminoethoxy)-L-phenylalanine
  MOD_RES (8)..(8): PEG4 conjugation
  MOD_RES (9)..(9): L-2-Napthylalanine
  MOD_RES (10)..(10): 4-amino-4-carboxy-tetrahydropyran
XXETWQCXXXENN

SEQ ID NO: 91 - protein, 13 aa, Artificial Sequence
  Synthesized peptide
  MOD_RES (1)..(1): D-form arginine
  MOD_RES (1)..(1): PEG4 conjugation
  MOD_RES (2)..(2): Abu
  MISC_FEATURE (2)..(7): residues cyclosized
  MOD_RES (8)..(8): 4-(2-aminoethoxy)-L-phenylalanine
  MOD_RES (8)..(8): PEG4 - Biotin conjugation
  MOD_RES (9)..(9): L-2-Napthylalanine
  MOD_RES (10)..(10): 4-amino-4-carboxy-tetrahydropyran
XXETWQCXXXENN

SEQ ID NO: 92 - protein, 13 aa, Artificial Sequence
  Synthesized peptide
  MOD_RES (1)..(1): D-form arginine
  MOD_RES (2)..(2): Abu
  MISC_FEATURE (2)..(7): residues cyclosized
  MOD_RES (7)..(7): L-Penicillamine
  MOD_RES (8)..(8): 4-(2-aminoethoxy)-L-phenylalanine
  MOD_RES (9)..(9): L-2-Napthylalanine
  MOD_RES (10)..(10): 4-amino-4-carboxy-tetrahydropyran
XXQTWQXXXXENN

SEQ ID NO: 93 - protein, 13 aa, Artificial Sequence
  Synthesized peptide
  MOD_RES (1)..(1): D-form arginine
  MOD_RES (2)..(2): Abu
  MISC_FEATURE (2)..(7): residues cyclosized
  MOD_RES (6)..(6): alpha-methyl-L-Leucine
  MOD_RES (8)..(8): 4-(2-aminoethoxy)-L-phenylalanine
  MOD_RES (9)..(9): L-2-Napthylalanine
  MOD_RES (10)..(10): 4-amino-4-carboxy-tetrahydropyran
XXQTWXCXXXENN

SEQ ID NO: 94 - protein, 13 aa, Artificial Sequence
  Synthesized peptide
  MOD_RES (1)..(1): D-form arginine
  MOD_RES (2)..(2): Abu
  MISC_FEATURE (2)..(7): residues cyclosized
  MOD_RES (6)..(6): alpha-methyl-L-Lysine
  MOD_RES (8)..(8): 4-(2-aminoethoxy)-L-phenylalanine
  MOD_RES (9)..(9): L-2-Napthylalanine
  MOD_RES (10)..(10): 4-amino-4-carboxy-tetrahydropyran
XXQTWXCXXXENN

SEQ ID NO: 95 - protein, 13 aa, Artificial Sequence
  Synthesized peptide
  MOD_RES (1)..(1): D-form arginine
  MOD_RES (2)..(2): Abu
  MISC_FEATURE (2)..(7): residues cyclosized
  MOD_RES (6)..(6): alpha-methyl-L-Lysine
  MOD_RES (6)..(6): ACETYLATION
  MOD_RES (8)..(8): 4-(2-aminoethoxy)-L-phenylalanine
  MOD_RES (9)..(9): L-2-Napthylalanine
  MOD_RES (10)..(10): 4-amino-4-carboxy-tetrahydropyran
XXQTWXCXXXENN

SEQ ID NO: 96 - protein, 13 aa, Artificial Sequence
  Synthesized peptide
  MOD_RES (1)..(1): D-form arginine
  MOD_RES (2)..(2): Abu
  MISC_FEATURE (2)..(7): residues cyclosized
  MOD_RES (6)..(6): D-form glutamine
  MOD_RES (8)..(8): 4-(2-aminoethoxy)-L-phenylalanine
  MOD_RES (9)..(9): L-2-Napthylalanine
  MOD_RES (10)..(10): 4-amino-4-carboxy-tetrahydropyran
XXQTWXCXXXENN

SEQ ID NO: 97 - protein, 13 aa, Artificial Sequence
  Synthesized peptide
  MOD_RES (1)..(1): D-form arginine
  MOD_RES (2)..(2): Abu
  MISC_FEATURE (2)..(7): residues cyclosized
  MOD_RES (6)..(6): beta homoglutamine
  MOD_RES (8)..(8): 4-(2-aminoethoxy)-L-phenylalanine
  MOD_RES (9)..(9): L-2-Napthylalanine
  MOD_RES (10)..(10): 4-amino-4-carboxy-tetrahydropyran
XXQTWXCXXXENN

SEQ ID NO: 98 - protein, 13 aa, Artificial Sequence
  Synthesized peptide
  MOD_RES (1)..(1): D-form arginine
  MOD_RES (2)..(2): Abu
  MISC_FEATURE (2)..(7): residues cyclosized
  MOD_RES (6)..(6): alpha-methyl-L-Lysine
  MOD_RES (6)..(6): ACETYLATION
  MOD_RES (8)..(8): 4-(2-aminoethoxy)-L-phenylalanine
  MOD_RES (9)..(9): L-2-Napthylalanine
  MOD_RES (10)..(10): 4-amino-4-carboxy-tetrahydropyran
XXQTWXCXXXENN

SEQ ID NO: 99 - protein, 13 aa, Artificial Sequence
  Synthesized peptide
  MOD_RES (1)..(1): D-form arginine
  MOD_RES (2)..(2): Abu
  MISC_FEATURE (2)..(7): residues cyclosized
  MOD_RES (8)..(8): 4-(2-aminoethoxy)-L-phenylalanine
  MOD_RES (9)..(9): L-2-Napthylalanine
  MOD_RES (10)..(10): 4-amino-4-carboxy-tetrahydropyran
XXQTWFCXXXENN

SEQ ID NO: 100 - protein, 13 aa, Artificial Sequence
  Synthesized peptide
  MOD_RES (1)..(1): D-form arginine
  MOD_RES (2)..(2): Abu
  MISC_FEATURE (2)..(7): residues cyclosized
  MOD_RES (8)..(8): 4-(2-aminoethoxy)-L-phenylalanine
  MOD_RES (9)..(9): L-2-Napthylalanine
  MOD_RES (10)..(10): 4-amino-4-carboxy-tetrahydropyran
XXQTWWCXXXENN

SEQ ID NO: 101 - protein, 13 aa, Artificial Sequence
  Synthesized peptide
  MOD_RES (1)..(1): D-form arginine
  MOD_RES (2)..(2): Abu
  MISC_FEATURE (2)..(7): residues cyclosized
  MOD_RES (6)..(6): Aib
  MOD_RES (8)..(8): 4-(2-aminoethoxy)-L-phenylalanine
  MOD_RES (9)..(9): L-2-Napthylalanine
  MOD_RES (10)..(10): 4-amino-4-carboxy-tetrahydropyran
XXQTWXCXXXENN

SEQ ID NO: 102 - protein, 13 aa, Artificial Sequence
  Synthesized peptide
  MOD_RES (1)..(1): D-form arginine
  MOD_RES (2)..(2): Abu
  MISC_FEATURE (2)..(7): residues cyclosized
  MOD_RES (8)..(8): 4-(2-aminoethoxy)-L-phenylalanine
  MOD_RES (9)..(9): L-2-Napthylalanine
  MOD_RES (10)..(10): 4-amino-4-carboxy-tetrahydropyran
XXQTWTCXXXENN

SEQ ID NO: 103 - protein, 13 aa, Artificial Sequence
  Synthesized peptide
  MOD_RES (1)..(1): D-form arginine
  MOD_RES (2)..(2): Abu
  MISC_FEATURE (2)..(7): residues cyclosized
  MOD_RES (8)..(8): 4-(2-aminoethoxy)-L-phenylalanine
  MOD_RES (9)..(9): L-2-Napthylalanine
  MOD_RES (10)..(10): 4-amino-4-carboxy-tetrahydropyran
XXQTWVCXXXENN

SEQ ID NO: 104 - protein, 13 aa, Artificial Sequence
  Synthesized peptide
  MOD_RES (1)..(1): D-form arginine
  MOD_RES (2)..(2): Abu
  MISC_FEATURE (2)..(7): residues cyclosized
  MOD_RES (5)..(5): 5-Fluoro-L-tryptophan
  MOD_RES (8)..(8): 4-(2-aminoethoxy)-L-phenylalanine
  MOD_RES (9)..(9): L-2-Napthylalanine
  MOD_RES (10)..(10): 4-amino-4-carboxy-tetrahydropyran
XXQTXQCXXXENN

SEQ ID NO: 105 - protein, 13 aa, Artificial Sequence
  Synthesized peptide
  MOD_RES (1)..(1): D-form arginine
  MOD_RES (2)..(2): Abu
  MISC_FEATURE (2)..(7): residues cyclosized
  MOD_RES (5)..(5): 5-Fluoro-L-tryptophan
  MOD_RES (8)..(8): 4-(2-aminoethoxy)-L-phenylalanine
  MOD_RES (9)..(9): L-2-Napthylalanine
  MOD_RES (10)..(10): alpha-methyl-L-Leucine
XXQTXQCXXXENN

SEQ ID NO: 106 - protein, 12 aa, Artificial Sequence
  Synthesized peptide
  MOD_RES (1)..(1): Abu
  MISC_FEATURE (1)..(6): residues cyclosized
  MOD_RES (4)..(4): 5-Fluoro-L-tryptophan
  MOD_RES (7)..(7): 4-(2-aminoethoxy)-L-phenylalanine
  MOD_RES (8)..(8): L-2-Napthylalanine
  MOD_RES (9)..(9): alpha-methyl-L-Leucine
XQTXQCXXXENN

SEQ ID NO: 107 - protein, 13 aa, Artificial Sequence
  Synthesized peptide
  MOD_RES (1)..(1): D-form arginine
  MOD_RES (2)..(2): Abu
  MISC_FEATURE (2)..(7): residues cyclosized
  MOD_RES (8)..(8): 4-(2-aminoethoxy)-L-phenylalanine
  MOD_RES (9)..(9): L-2-Napthylalanine
  MOD_RES (10)..(10): alpha-methyl-L-Leucine
XXQTWQCXXXENN

SEQ ID NO: 108 - protein, 13 aa, Artificial Sequence
  Synthesized peptide
  MOD_RES (1)..(1): D-form arginine
  MOD_RES (2)..(2): Abu
  MISC_FEATURE (2)..(7): residues cyclosized
  MOD_RES (6)..(6): L-2-Napthylalanine
  MOD_RES (8)..(8): 4-(2-aminoethoxy)-L-phenylalanine
  MOD_RES (9)..(9): L-2-Napthylalanine
  MOD_RES (10)..(10): 4-amino-4-carboxy-tetrahydropyran
XXQTWXCXXXENN

SEQ ID NO: 109 - protein, 13 aa, Artificial Sequence
  Synthesized peptide
  MOD_RES (1)..(1): D-form arginine
  MOD_RES (2)..(2): Abu
  MISC_FEATURE (2)..(7): residues cyclosized
  MOD_RES (6)..(6): L-1-Napthylalanine
  MOD_RES (8)..(8): 4-(2-aminoethoxy)-L-phenylalanine
  MOD_RES (9)..(9): L-2-Napthylalanine
  MOD_RES (10)..(10): 4-amino-4-carboxy-tetrahydropyran
XXQTWXCXXXENN

SEQ ID NO: 110 - protein, 13 aa, Artificial Sequence
  Synthesized peptide
  MOD_RES (1)..(1): D-form arginine
  MOD_RES (2)..(2): Abu
  MISC_FEATURE (2)..(7): residues cyclosized
  MOD_RES (6)..(6): 5-Fluoro-L-tryptophan
  MOD_RES (8)..(8): 4-(2-aminoethoxy)-L-phenylalanine
  MOD_RES (9)..(9): L-2-Napthylalanine
  MOD_RES (10)..(10): 4-amino-4-carboxy-tetrahydropyran
XXQTWXCXXXENN

SEQ ID NO: 111 - protein, 13 aa, Artificial Sequence
  Synthesized peptide
  MOD_RES (1)..(1): Abu
  MISC_FEATURE (1)..(6): residues cyclosized
  MOD_RES (7)..(7): 4-(2-aminoethoxy)-L-phenylalanine
  MOD_RES (8)..(8): L-2-Napthylalanine
  MOD_RES (9)..(9): 4-amino-4-carboxy-tetrahydropyran
  MOD_RES (10)..(10): ACETYLATION
XQTWQCXXXKNNE

SEQ ID NO: 112 - protein, 13 aa, Artificial Sequence
  Synthesized peptide
  MOD_RES (1)..(1): Abu
  MISC_FEATURE (1)..(6): residues cyclosized
  MOD_RES (7)..(7): 4-(2-aminoethoxy)-L-phenylalanine
  MOD_RES (8)..(8): L-2-Napthylalanine
  MOD_RES (9)..(9): 4-amino-4-carboxy-tetrahydropyran
  MOD_RES (10)..(10): ACETYLATION
XQTWQCXXXKNNF

SEQ ID NO: 113 - protein, 13 aa, Artificial Sequence
  Synthesized peptide
  MOD_RES (1)..(1): Abu
  MISC_FEATURE (1)..(6): residues cyclosized
  MOD_RES (7)..(7): 4-(2-aminoethoxy)-L-phenylalanine
  MOD_RES (8)..(8): L-2-Napthylalanine
  MOD_RES (9)..(9): 4-amino-4-carboxy-tetrahydropyran
  MOD_RES (10)..(10): ACETYLATION
XQTWQCXXXKNNK

SEQ ID NO: 114 - protein, 13 aa, Artificial Sequence
  Synthesized peptide
  MOD_RES (1)..(1): Abu
  MISC_FEATURE (1)..(6): residues cyclosized
  MOD_RES (7)..(7): 4-(2-aminoethoxy)-L-phenylalanine
  MOD_RES (8)..(8): L-2-Napthylalanine
  MOD_RES (9)..(9): 4-amino-4-carboxy-tetrahydropyran
  MOD_RES (10)..(10): ACETYLATION
XQTWQCXXXKNNN

SEQ ID NO: 115 - protein, 13 aa, Artificial Sequence
  Synthesized peptide
  MOD_RES (1)..(1): Abu
  MISC_FEATURE (1)..(6): residues cyclosized
  MOD_RES (7)..(7): 4-(2-aminoethoxy)-L-phenylalanine
  MOD_RES (8)..(8): L-2-Napthylalanine
  MOD_RES (9)..(9): 4-amino-4-carboxy-tetrahydropyran
  MOD_RES (10)..(10): ACETYLATION
XQTWQCXXXKNNW

SEQ ID NO: 116 - protein, 13 aa, Artificial Sequence
  Synthesized peptide
  MOD_RES (1)..(1): Abu
  MISC_FEATURE (1)..(6): residues cyclosized
  MOD_RES (7)..(7): 4-(2-aminoethoxy)-L-phenylalanine
  MOD_RES (8)..(8): L-2-Napthylalanine
  MOD_RES (9)..(9): 4-amino-4-carboxy-tetrahydropyran
  MOD_RES (10)..(10): ACETYLATION
XQTWQCXXXKNNT

SEQ ID NO: 117 - protein, 14 aa, Artificial Sequence
  Synthesized peptide
  MOD_RES (1)..(1): Abu
  MISC_FEATURE (1)..(6): residues cyclosized
  MOD_RES (7)..(7): 4-(2-aminoethoxy)-L-phenylalanine
  MOD_RES (8)..(8): L-2-Napthylalanine
  MOD_RES (9)..(9): 4-amino-4-carboxy-tetrahydropyran
  MOD_RES (10)..(10): ACETYLATION
XQTWQCXXXKNNNG

SEQ ID NO: 118 - protein, 14 aa, Artificial Sequence
  Synthesized peptide
  MOD_RES (1)..(1): Abu
  MISC_FEATURE (1)..(6): residues cyclosized
  MOD_RES (7)..(7): 4-(2-aminoethoxy)-L-phenylalanine
  MOD_RES (8)..(8): L-2-Napthylalanine
  MOD_RES (9)..(9): 4-amino-4-carboxy-tetrahydropyran
  MOD_RES (10)..(10): ACETYLATION
XQTWQCXXXKNNPK

SEQ ID NO: 119 - protein, 14 aa, Artificial Sequence
  Synthesized peptide
  MOD_RES (1)..(1): Abu
  MISC_FEATURE (1)..(6): residues cyclosized
  MOD_RES (7)..(7): 4-(2-aminoethoxy)-L-phenylalanine
  MOD_RES (8)..(8): L-2-Napthylalanine
  MOD_RES (9)..(9): 4-amino-4-carboxy-tetrahydropyran
  MOD_RES (10)..(10): ACETYLATION
XQTWQCXXXKNNPG

SEQ ID NO: 120 - protein, 14 aa, Artificial Sequence
  Synthesized peptide
  MOD_RES (1)..(1): Abu
  MISC_FEATURE (1)..(6): residues cyclosized
  MOD_RES (7)..(7): 4-(2-aminoethoxy)-L-phenylalanine
  MOD_RES (8)..(8): L-2-Napthylalanine
  MOD_RES (9)..(9): 4-amino-4-carboxy-tetrahydropyran
  MOD_RES (10)..(10): ACETYLATION
XQTWQCXXXKNNEP

SEQ ID NO: 121 - protein, 14 aa, Artificial Sequence
  Synthesized peptide
  MOD_RES (1)..(1): Abu
  MISC_FEATURE (1)..(6): residues cyclosized
  MOD_RES (7)..(7): 4-(2-aminoethoxy)-L-phenylalanine
  MOD_RES (8)..(8): L-2-Napthylalanine
  MOD_RES (9)..(9): 4-amino-4-carboxy-tetrahydropyran
  MOD_RES (10)..(10): ACETYLATION
XQTWQCXXXKNNGK

SEQ ID NO: 122 - protein, 14 aa, Artificial Sequence
  Synthesized peptide
  MOD_RES (1)..(1): Abu
  MISC_FEATURE (1)..(6): residues cyclosized
  MOD_RES (7)..(7): 4-(2-aminoethoxy)-L-phenylalanine
  MOD_RES (8)..(8): L-2-Napthylalanine
  MOD_RES (9)..(9): 4-amino-4-carboxy-tetrahydropyran
  MOD_RES (10)..(10): ACETYLATION
XQTWQCXXXKNNPT

SEQ ID NO: 123 - protein, 14 aa, Artificial Sequence
  Synthesized peptide
  MOD_RES (1)..(1): Abu
  MISC_FEATURE (1)..(6): residues cyclosized
  MOD_RES (7)..(7): 4-(2-aminoethoxy)-L-phenylalanine
  MOD_RES (8)..(8): L-2-Napthylalanine
  MOD_RES (9)..(9): 4-amino-4-carboxy-tetrahydropyran
  MOD_RES (10)..(10): ACETYLATION
XQTWQCXXXKNNGF

SEQ ID NO: 124 - protein, 14 aa, Artificial Sequence
  Synthesized peptide
  MOD_RES (1)..(1): Abu
  MISC_FEATURE (1)..(6): residues cyclosized
  MOD_RES (7)..(7): 4-(2-aminoethoxy)-L-phenylalanine
  MOD_RES (8)..(8): L-2-Napthylalanine
  MOD_RES (9)..(9): 4-amino-4-carboxy-tetrahydropyran
  MOD_RES (10)..(10): ACETYLATION
XQTWQCXXXKNNGW

SEQ ID NO: 125 - protein, 14 aa, Artificial Sequence
  Synthesized peptide
  MOD_RES (1)..(1): Abu
  MISC_FEATURE (1)..(6): residues cyclosized
  MOD_RES (7)..(7): 4-(2-aminoethoxy)-L-phenylalanine
  MOD_RES (8)..(8): L-2-Napthylalanine
  MOD_RES (9)..(9): 4-amino-4-carboxy-tetrahydropyran
  MOD_RES (10)..(10): ACETYLATION
XQTWQCXXXKNNGQ

SEQ ID NO: 126 - protein, 15 aa, Artificial Sequence
  Synthesized peptide
  MOD_RES (1)..(1): Abu
  MISC_FEATURE (1)..(6): residues cyclosized
  MOD_RES (7)..(7): 4-(2-aminoethoxy)-L-phenylalanine
  MOD_RES (8)..(8): L-2-Napthylalanine
  MOD_RES (9)..(9): 4-amino-4-carboxy-tetrahydropyran
  MOD_RES (10)..(10): ACETYLATION
XQTWQCXXXKNNGGG

SEQ ID NO: 127 - protein, 15 aa, Artificial Sequence
  Synthesized peptide
  MOD_RES (1)..(1): Abu
  MISC_FEATURE (1)..(6): residues cyclosized
  MOD_RES (7)..(7): 4-(2-aminoethoxy)-L-phenylalanine
  MOD_RES (8)..(8): L-2-Napthylalanine
  MOD_RES (9)..(9): 4-amino-4-carboxy-tetrahydropyran
  MOD_RES (10)..(10): ACETYLATION
XQTWQCXXXKNNKKK

SEQ ID NO: 128 - protein, 15 aa, Artificial Sequence
  Synthesized peptide
  MOD_RES (1)..(1): Abu
  MISC_FEATURE (1)..(6): residues cyclosized
  MOD_RES (7)..(7): 4-(2-aminoethoxy)-L-phenylalanine
  MOD_RES (8)..(8): L-2-Napthylalanine
  MOD_RES (9)..(9): 4-amino-4-carboxy-tetrahydropyran
  MOD_RES (10)..(10): ACETYLATION
XQTWQCXXXKNNEEE

SEQ ID NO: 129 - protein, 15 aa, Artificial Sequence
  Synthesized peptide
  MOD_RES (1)..(1): Abu
  MISC_FEATURE (1)..(6): residues cyclosized
  MOD_RES (7)..(7): 4-(2-aminoethoxy)-L-phenylalanine
  MOD_RES (8)..(8): L-2-Napthylalanine
  MOD_RES (9)..(9): 4-amino-4-carboxy-tetrahydropyran
  MOD_RES (10)..(10): ACETYLATION
XQTWQCXXXKNNFFF

SEQ ID NO: 130 - protein, 15 aa, Artificial Sequence
  Synthesized peptide
  MOD_RES (1)..(1): Abu
  MISC_FEATURE (1)..(6): residues cyclosized
  MOD_RES (7)..(7): 4-(2-aminoethoxy)-L-phenylalanine
  MOD_RES (8)..(8): L-2-Napthylalanine
  MOD_RES (9)..(9): 4-amino-4-carboxy-tetrahydropyran
  MOD_RES (10)..(10): ACETYLATION
XQTWQCXXXKNNTTT

SEQ ID NO: 131 - protein, 13 aa, Artificial Sequence
  Synthesized peptide
  MOD_RES (1)..(1): D-form arginine
  MOD_RES (2)..(2): Abu
  MISC_FEATURE (2)..(7): residues cyclosized
  MOD_RES (5)..(5): azatryptophan
  MOD_RES (8)..(8): 4-(2-aminoethoxy)-L-phenylalanine
  MOD_RES (9)..(9): L-2-Napthylalanine
  MOD_RES (10)..(10): alpha-methyl-L-Leucine
XXQTXQCXXXENN

SEQ ID NO: 132 - protein, 13 aa, Artificial Sequence
  Synthesized peptide
  MOD_RES (1)..(1): D-form arginine
  MOD_RES (2)..(2): Abu
  MISC_FEATURE (2)..(7): residues cyclosized
  MOD_RES (5)..(5): Trp(5-CN)
  MOD_RES (8)..(8): 4-(2-aminoethoxy)-L-phenylalanine
  MOD_RES (9)..(9): L-2-Napthylalanine
  MOD_RES (10)..(10): alpha-methyl-L-Leucine
XXQTXQCXXXENN

SEQ ID NO: 133 - protein, 13 aa, Artificial Sequence
  Synthesized peptide
  MOD_RES (1)..(1): D-form arginine
  MOD_RES (2)..(2): Abu
  MISC_FEATURE (2)..(7): residues cyclosized
  MOD_RES (5)..(5): Trp(5-Cl)
  MOD_RES (8)..(8): 4-(2-aminoethoxy)-L-phenylalanine
  MOD_RES (9)..(9): L-2-Napthylalanine
  MOD_RES (10)..(10): alpha-methyl-L-Leucine
XXQTXQCXXXENN

SEQ ID NO: 134 - protein, 13 aa, Artificial Sequence
  Synthesized peptide
  MOD_RES (1)..(1): D-form arginine
  MOD_RES (2)..(2): Abu
  MISC_FEATURE (2)..(7): residues cyclosized
  MOD_RES (5)..(5): Trp(6-OH)
  MOD_RES (8)..(8): 4-(2-aminoethoxy)-L-phenylalanine
  MOD_RES (9)..(9): L-2-Napthylalanine
  MOD_RES (10)..(10): alpha-methyl-L-Leucine
XXQTXQCXXXENN

SEQ ID NO: 135 - protein, 12 aa, Artificial Sequence
  Synthesized peptide
  MOD_RES (1)..(1): D-form Abu
  MISC_FEATURE (1)..(6): residues cyclosized
  MOD_RES (7)..(7): 4-(2-aminoethoxy)-L-phenylalanine
  MOD_RES (8)..(8): L-2-Napthylalanine
  MOD_RES (9)..(9): alpha-methyl-L-Leucine
XQTWQCXXXENN

SEQ ID NO: 136 - protein, 12 aa, Artificial Sequence
  Synthesized peptide
  MOD_RES (1)..(1): D-form Abu
  MISC_FEATURE (1)..(6): residues cyclosized
  MOD_RES (6)..(6): L-Penicillamine
  MOD_RES (7)..(7): 4-(2-aminoethoxy)-L-phenylalanine
  MOD_RES (8)..(8): L-2-Napthylalanine
  MOD_RES (9)..(9): alpha-methyl-L-Leucine
  MOD_RES (10)..(10): ACETYLATION
XNTWQXXXXKNN

SEQ ID NO: 137 - protein, 12 aa, Artificial Sequence
  Synthesized peptide
  MOD_RES (1)..(1): L-Penicillamine
  MISC_FEATURE (1)..(6): residues cyclosized
  MOD_RES (6)..(6): D-form Abu
  MOD_RES (7)..(7): 4-(2-aminoethoxy)-L-phenylalanine
  MOD_RES (8)..(8): L-2-Napthylalanine
  MOD_RES (9)..(9): alpha-methyl-L-Leucine
  MOD_RES (10)..(10): ACETYLATION
XNTWQXXXXKNN

SEQ ID NO: 138 - protein, 13 aa, Artificial Sequence
  Synthesized peptide
  MOD_RES (1)..(1): D-form arginine
  MOD_RES (2)..(2): Abu
  MISC_FEATURE (2)..(7): residues cyclosized
  MOD_RES (8)..(8): 4-(2-aminoethoxy)-L-phenylalanine
  MOD_RES (9)..(9): L-2-Napthylalanine
  MOD_RES (10)..(10): alpha-methyl-L-Leucine
XXQTWQCXXXENN

SEQ ID NO: 139 - protein, 13 aa, Artificial Sequence
  Synthesized peptide
  MOD_RES (1)..(1): D-form arginine
  MOD_RES (2)..(2): Abu
  MISC_FEATURE (2)..(7): residues cyclosized
  MOD_RES (6)..(6): L-2-Napthylalanine
  MOD_RES (8)..(8): 4-(2-aminoethoxy)-L-phenylalanine
  MOD_RES (9)..(9): L-2-Napthylalanine
  MOD_RES (10)..(10): 4-amino-4-carboxy-tetrahydropyran
XXQTWXCXXXENN

SEQ ID NO: 140 - protein, 13 aa, Artificial Sequence
  Synthesized peptide
  MOD_RES (1)..(1): D-form arginine
  MOD_RES (2)..(2): Abu
  MISC_FEATURE (2)..(7): residues cyclosized
  MOD_RES (6)..(6): L-1-Napthylalanine
  MOD_RES (8)..(8): 4-(2-aminoethoxy)-L-phenylalanine
  MOD_RES (9)..(9): L-2-Napthylalanine
  MOD_RES (10)..(10): 4-amino-4-carboxy-tetrahydropyran
XXQTWXCXXXENN

SEQ ID NO: 141 - protein, 13 aa, Artificial Sequence
  Synthesized peptide
  MOD_RES (1)..(1): D-form arginine
  MOD_RES (2)..(2): Abu
  MISC_FEATURE (2)..(7): residues cyclosized
  MOD_RES (6)..(6): Trp(5-F)
  MOD_RES (8)..(8): 4-(2-aminoethoxy)-L-phenylalanine
  MOD_RES (9)..(9): L-2-Napthylalanine
  MOD_RES (10)..(10): 4-amino-4-carboxy-tetrahydropyran
XXQTWXCXXXENN

SEQ ID NO: 142 - protein, 12 aa, Artificial Sequence
  Synthesized peptide
  MOD_RES (1)..(1): L-Penicillamine
  MOD_RES (6)..(6): L-Penicillamine
  MOD_RES (7)..(7): 4-(2-aminoethoxy)-L-phenylalanine
  MOD_RES (8)..(8): L-2-Napthylalanine
  MOD_RES (9)..(9): alpha-methyl-L-Leucine
  MOD_RES (10)..(10): ACETYLATION
XNTWQXXXXKNN

SEQ ID NO: 143 - protein, 12 aa, Artificial Sequence
  Synthesized peptide
  MOD_RES (1)..(1): L-Penicillamine
  MOD_RES (6)..(6): L-Penicillamine
  MOD_RES (7)..(7): 4-(2-aminoethoxy)-L-phenylalanine
  MOD_RES (8)..(8): L-2-Napthylalanine
  MOD_RES (9)..(9): alpha-methyl-L-Leucine
  MOD_RES (10)..(10): ACETYLATION
XNTWQXXXXKND

SEQ ID NO: 144 - protein, 12 aa, Artificial Sequence
  Synthesized peptide
  MOD_RES (1)..(1): L-Penicillamine
  MOD_RES (6)..(6): L-Penicillamine
  MOD_RES (7)..(7): 4-(2-aminoethoxy)-L-phenylalanine
  MOD_RES (8)..(8): L-2-Napthylalanine
  MOD_RES (9)..(9): alpha-methyl-L-Leucine
  MOD_RES (10)..(10): ACETYLATION
XNTWQXXXXKDN

SEQ ID NO: 145 - protein, 12 aa, Artificial Sequence
  Synthesized peptide
  MOD_RES (1)..(1): L-Penicillamine
  MOD_RES (6)..(6): L-Penicillamine
  MOD_RES (7)..(7): 4-(2-aminoethoxy)-L-phenylalanine
  MOD_RES (8)..(8): L-2-Napthylalanine
  MOD_RES (9)..(9): alpha-methyl-L-Leucine
  MOD_RES (10)..(10): ACETYLATION
XNTWEXXXXKNN

SEQ ID NO: 146 - protein, 12 aa, Artificial Sequence
  Synthesized peptide
  MOD_RES (1)..(1): L-Penicillamine
  MOD_RES (6)..(6): L-Penicillamine
  MOD_RES (7)..(7): 4-(2-aminoethoxy)-L-phenylalanine
  MOD_RES (8)..(8): L-2-Napthylalanine
  MOD_RES (9)..(9): alpha-methyl-L-Leucine
  MOD_RES (10)..(10): ACETYLATION
XDTWQXXXXKDN

SEQ ID NO: 147 - protein, 13 aa, Artificial Sequence
  Synthesized peptide
  MOD_RES (1)..(1): D-form arginine
  MOD_RES (2)..(2): Abu
  MISC_FEATURE (2)..(7): residues cyclosized
  MOD_RES (8)..(8): 4-(2-aminoethoxy)-L-phenylalanine
  MOD_RES (9)..(9): L-2-Napthylalanine
  MOD_RES (10)..(10): 3-cyclohexyl-L-alanine
XXQTWQCXXXENN

SEQ ID NO: 148 - protein, 13 aa, Artificial Sequence
  Synthesized peptide
  MOD_RES (1)..(1): D-form arginine
  MOD_RES (2)..(2): Abu
  MISC_FEATURE (2)..(7): residues cyclosized
  MOD_RES (8)..(8): 4-(2-aminoethoxy)-L-phenylalanine
  MOD_RES (9)..(9): L-2-Napthylalanine
  MOD_RES (10)..(10): Aib
XXQTWQCXXXENN

SEQ ID NO: 149 - protein, 13 aa, Artificial Sequence
  Synthesized peptide
  MOD_RES (1)..(1): D-form arginine
  MOD_RES (2)..(2): Abu
  MISC_FEATURE (2)..(7): residues cyclosized
  MOD_RES (8)..(8): 4-(2-aminoethoxy)-L-phenylalanine
  MOD_RES (9)..(9): L-2-Napthylalanine
  MOD_RES (10)..(10): 4-amino-4-carboxy-tetrahydropyran
XXQTWQCXXXENN

SEQ ID NO: 150 - protein, 13 aa, Artificial Sequence
  Synthesized peptide
  MOD_RES (1)..(1): D-form arginine
  MOD_RES (2)..(2): D-form Penicillamine
  MISC_FEATURE (2)..(7): residues cyclosized
  MOD_RES (8)..(8): 4-(2-aminoethoxy)-L-phenylalanine
  MOD_RES (9)..(9): L-2-Napthylalanine
  MOD_RES (10)..(10): 4-amino-4-carboxy-tetrahydropyran
XXQTWQCXXXENN

SEQ ID NO: 151 - protein, 12 aa, Artificial Sequence
  Synthesized peptide
  MOD_RES (1)..(1): D-form Penicillamine
  MISC_FEATURE (1)..(6): residues cyclosized
  MOD_RES (6)..(6): Abu
  MOD_RES (7)..(7): 4-(2-aminoethoxy)-L-phenylalanine
  MOD_RES (8)..(8): L-2-Napthylalanine
  MOD_RES (9)..(9): 4-amino-4-carboxy-tetrahydropyran
XNTWQXXXXENN

SEQ ID NO: 152 - protein, 12 aa, Artificial Sequence
  Synthesized peptide
  MOD_RES (1)..(1): D-form Penicillamine with sulfoxide conjugation
  MISC_FEATURE (1)..(6): residues cyclosized
  MOD_RES (6)..(6): Abu
  MOD_RES (7)..(7): 4-(2-aminoethoxy)-L-phenylalanine
  MOD_RES (8)..(8): L-2-Napthylalanine
  MOD_RES (9)..(9): 4-amino-4-carboxy-tetrahydropyran
XNTWQXXXXENN

SEQ ID NO: 153 - protein, 13 aa, Artificial Sequence
  Synthesized peptide
  MOD_RES (1)..(1): D-form arginine
  MOD_RES (2)..(2): Abu
  MISC_FEATURE (2)..(7): residues cyclosized
  MOD_RES (6)..(6): IsoGlu - Palmityl conjugation
  MOD_RES (8)..(8): 4-(2-aminoethoxy)-L-phenylalanine
  MOD_RES (9)..(9): L-2-Napthylalanine
  MOD_RES (10)..(10): 4-amino-4-carboxy-tetrahydropyran
XXQTWKCXXXENN

SEQ ID NO: 154 - protein, 13 aa, Artificial Sequence
  Synthesized peptide
  MOD_RES (1)..(1): D-form arginine
  MOD_RES (2)..(2): Abu
  MISC_FEATURE (2)..(7): residues cyclosized
  MOD_RES (6)..(6): PEG12 conjugation
  MOD_RES (8)..(8): 4-(2-aminoethoxy)-L-phenylalanine
  MOD_RES (9)..(9): L-2-Napthylalanine
  MOD_RES (10)..(10): 4-amino-4-carboxy-tetrahydropyran
XXQTWKCXXXENN

SEQ ID NO: 155 - protein, 13 aa, Artificial Sequence
  Synthesized peptide
  MOD_RES (1)..(1): D-form arginine
  MOD_RES (2)..(2): Abu
  MISC_FEATURE (2)..(7): residues cyclosized
  MOD_RES (8)..(8): 4-(2-aminoethoxy)-L-phenylalanine
  MOD_RES (9)..(9): L-2-Napthylalanine
  MOD_RES (10)..(10): 4-amino-4-carboxy-tetrahydropyran
  MOD_RES (11)..(11): IsoGlu - Palmityl conjugation
XXQTWQCXXXKNN

SEQ ID NO: 156 - protein, 13 aa, Artificial Sequence
  Synthesized peptide
  MOD_RES (1)..(1): D-form arginine
  MOD_RES (2)..(2): Abu
  MISC_FEATURE (2)..(7): residues cyclosized
  MOD_RES (8)..(8): 4-(2-aminoethoxy)-L-phenylalanine
  MOD_RES (9)..(9): L-2-Napthylalanine
  MOD_RES (10)..(10): 4-amino-4-carboxy-tetrahydropyran
  MOD_RES (11)..(11): PEG12 conjugation
XXQTWQCXXXKNN

SEQ ID NO: 157 - protein, 13 aa, Artificial Sequence
  Synthesized peptide
  MOD_RES (1)..(1): D-form arginine
  MOD_RES (2)..(2): Abu
  MISC_FEATURE (2)..(7): residues cyclosized
  MOD_RES (8)..(8): 4-(2-aminoethoxy)-L-phenylalanine
  MOD_RES (9)..(9): L-2-Napthylalanine
  MOD_RES (10)..(10): PEG12 conjugation
XXQTWQCXXKENN

SEQ ID NO: 158 - protein, 13 aa, Artificial Sequence
  Synthesized peptide
  MOD_RES (1)..(1): L-Penicillamine
  MOD_RES (6)..(6): L-Penicillamine
  MOD_RES (7)..(7): 4-(2-aminoethoxy)-L-phenylalanine
  MOD_RES (8)..(8): L-2-Napthylalanine
  MOD_RES (9)..(9): alpha-methyl-L-Leucine
  MOD_RES (10)..(10): ACETYLATION
XNTWQXXXXKNND

SEQ ID NO: 159 - protein, 13 aa, Artificial Sequence
  Synthesized peptide
  MOD_RES (1)..(1): L-Penicillamine
  MOD_RES (6)..(6): L-Penicillamine
  MOD_RES (7)..(7): 4-(2-aminoethoxy)-L-phenylalanine
  MOD_RES (8)..(8): L-2-Napthylalanine
  MOD_RES (9)..(9): alpha-methyl-L-Leucine
  MOD_RES (10)..(10): ACETYLATION
XNTWQXXXXKNNY

SEQ ID NO: 160 - protein, 13 aa, Artificial Sequence
  Synthesized peptide
  MOD_RES (1)..(1): L-Penicillamine
  MOD_RES (6)..(6): L-Penicillamine
  MOD_RES (7)..(7): 4-(2-aminoethoxy)-L-phenylalanine
  MOD_RES (8)..(8): L-2-Napthylalanine
  MOD_RES (9)..(9): alpha-methyl-L-Leucine
  MOD_RES (10)..(10): ACETYLATION
XNTWQXXXXKNNW

SEQ ID NO: 161 - protein, 13 aa, Artificial Sequence
  Synthesized peptide
  MOD_RES (1)..(1): L-Penicillamine
  MOD_RES (6)..(6): L-Penicillamine
  MOD_RES (7)..(7): 4-(2-aminoethoxy)-L-phenylalanine
  MOD_RES (8)..(8): L-2-Napthylalanine
  MOD_RES (9)..(9): alpha-methyl-L-Leucine
  MOD_RES (10)..(10): ACETYLATION
XNTWQXXXXKNNR

SEQ ID NO: 162 - protein, 13 aa, Artificial Sequence
  Synthesized peptide
  MOD_RES (1)..(1): L-Penicillamine
  MOD_RES (6)..(6): L-Penicillamine
  MOD_RES (7)..(7): 4-(2-aminoethoxy)-L-phenylalanine
  MOD_RES (8)..(8): L-2-Napthylalanine
  MOD_RES (9)..(9): alpha-methyl-L-Leucine
  MOD_RES (10)..(10): ACETYLATION
XNTWQXXXXKNNL

SEQ ID NO: 163 - protein, 13 aa, Artificial Sequence
  Synthesized peptide
  MOD_RES (1)..(1): L-Penicillamine
  MOD_RES (6)..(6): L-Penicillamine
  MOD_RES (7)..(7): 4-(2-aminoethoxy)-L-phenylalanine
  MOD_RES (8)..(8): L-2-Napthylalanine
  MOD_RES (9)..(9): alpha-methyl-L-Leucine
  MOD_RES (10)..(10): ACETYLATION
XNTWQXXXXKNNG

SEQ ID NO: 164 - protein, 13 aa, Artificial Sequence
  Synthesized peptide
  MOD_RES (1)..(1): L-Penicillamine
  MOD_RES (6)..(6): L-Penicillamine
  MOD_RES (7)..(7): 4-(2-aminoethoxy)-L-phenylalanine
  MOD_RES (8)..(8): L-2-Napthylalanine
  MOD_RES (9)..(9): alpha-methyl-L-Leucine
  MOD_RES (10)..(10): ACETYLATION
XNTWQXXXXKNNQ

SEQ ID NO: 165 - protein, 13 aa, Artificial Sequence
  Synthesized peptide
  MOD_RES (1)..(1): L-Penicillamine
  MOD_RES (6)..(6): L-Penicillamine
  MOD_RES (7)..(7): 4-(2-aminoethoxy)-L-phenylalanine
  MOD_RES (8)..(8): L-2-Napthylalanine
  MOD_RES (9)..(9): alpha-methyl-L-Leucine
  MOD_RES (10)..(10): ACETYLATION
XNTWQXXXXKNNS

SEQ ID NO: 166 - protein, 12 aa, Artificial Sequence
  Synthesized peptide
  MOD_RES (1)..(1): L-Penicillamine
  MOD_RES (6)..(6): L-Penicillamine
  MOD_RES (7)..(7): 4-(2-aminoethoxy)-L-phenylalanine
  MOD_RES (8)..(8): L-2-Napthylalanine
  MOD_RES (9)..(9): alpha-methyl-L-Leucine
  MOD_RES (10)..(10): ACETYLATION
  MOD_RES (12)..(12): ACETYLATION
XNTWQXXXXKNK

SEQ ID NO: 167 - protein, 12 aa, Artificial Sequence
  Synthesized peptide
  MOD_RES (1)..(1): L-Penicillamine
  MOD_RES (6)..(6): L-Penicillamine
  MOD_RES (7)..(7): 4-(2-aminoethoxy)-L-phenylalanine
  MOD_RES (8)..(8): L-2-Napthylalanine
  MOD_RES (9)..(9): alpha-methyl-L-Leucine
  MOD_RES (11)..(11): ACETYLATION
  MOD_RES (12)..(12): ACETYLATION
XNTWQXXXXEKK

SEQ ID NO: 168 - protein, 12 aa, Artificial Sequence
  Synthesized peptide
  MOD_RES (1)..(1): L-Penicillamine
  MOD_RES (6)..(6): L-Penicillamine
  MOD_RES (7)..(7): 4-(2-aminoethoxy)-L-phenylalanine
  MOD_RES (8)..(8): L-2-Napthylalanine
  MOD_RES (9)..(9): alpha-methyl-L-Leucine
XNTWQXXXXENN

SEQ ID NO: 169 - protein, 12 aa, Artificial Sequence
  Synthesized peptide
  MOD_RES (1)..(1): L-Penicillamine
  MOD_RES (2)..(2): ACETYLATION
  MOD_RES (6)..(6): L-Penicillamine
  MOD_RES (7)..(7): 4-(2-aminoethoxy)-L-phenylalanine
  MOD_RES (8)..(8): L-2-Napthylalanine
  MOD_RES (9)..(9): alpha-methyl-L-Leucine
  MOD_RES (10)..(10): ACETYLATION
XKTWQXXXXKNN

SEQ ID NO: 170 - protein, 12 aa, Artificial Sequence
  Synthesized peptide
  MOD_RES (1)..(1): L-Penicillamine
  MOD_RES (5)..(5): ACETYLATION
  MOD_RES (6)..(6): L-Penicillamine
  MOD_RES (7)..(7): 4-(2-aminoethoxy)-L-phenylalanine
  MOD_RES (8)..(8): L-2-Napthylalanine
  MOD_RES (9)..(9): alpha-methyl-L-Leucine
  MOD_RES (10)..(10): ACETYLATION
XNTWKXXXXKNN

SEQ ID NO: 171 - protein, 13 aa, Artificial Sequence
  Synthesized peptide
  MOD_RES (1)..(1): L-Penicillamine
  MOD_RES (6)..(6): L-Penicillamine
  MOD_RES (7)..(7): 4-(2-aminoethoxy)-L-phenylalanine
  MOD_RES (8)..(8): L-2-Napthylalanine
  MOD_RES (9)..(9): alpha-methyl-L-Leucine
  MOD_RES (10)..(10): ACETYLATION
  MOD_RES (13)..(13): D-from aspartic acid
XNTWQXXXXKNNX

SEQ ID NO: 172 - protein, 13 aa, Artificial Sequence
  Synthesized peptide
  MOD_RES (1)..(1): L-Penicillamine
  MOD_RES (6)..(6): L-Penicillamine
  MOD_RES (7)..(7): 4-(2-aminoethoxy)-L-phenylalanine
  MOD_RES (8)..(8): L-2-Napthylalanine
  MOD_RES (9)..(9): alpha-methyl-L-Leucine
  MOD_RES (10)..(10): ACETYLATION
  MOD_RES (13)..(13): D-from tyrosine
XNTWQXXXXKNNX

SEQ ID NO: 173 - protein, 13 aa, Artificial Sequence
  Synthesized peptide
  MOD_RES (1)..(1): L-Penicillamine
  MOD_RES (6)..(6): L-Penicillamine
  MOD_RES (7)..(7): 4-(2-aminoethoxy)-L-phenylalanine
  MOD_RES (8)..(8): L-2-Napthylalanine
  MOD_RES (9)..(9): alpha-methyl-L-Leucine
  MOD_RES (10)..(10): ACETYLATION
  MOD_RES (13)..(13): L-2-Napthylalanine
XNTWQXXXXKNNX

SEQ ID NO: 174 - protein, 13 aa, Artificial Sequence
  Synthesized peptide
  MOD_RES (1)..(1): L-Penicillamine
  MOD_RES (6)..(6): L-Penicillamine
  MOD_RES (7)..(7): 4-(2-aminoethoxy)-L-phenylalanine
  MOD_RES (8)..(8): L-2-Napthylalanine
  MOD_RES (9)..(9): alpha-methyl-L-Leucine
  MOD_RES (10)..(10): ACETYLATION
  MOD_RES (13)..(13): D-from arginine
XNTWQXXXXKNNX

SEQ ID NO: 175 - protein, 13 aa, Artificial Sequence
  Synthesized peptide
  MOD_RES (1)..(1): L-Penicillamine
  MOD_RES (6)..(6): L-Penicillamine
  MOD_RES (7)..(7): 4-(2-aminoethoxy)-L-phenylalanine
  MOD_RES (8)..(8): L-2-Napthylalanine
  MOD_RES (9)..(9): alpha-methyl-L-Leucine
  MOD_RES (10)..(10): ACETYLATION
  MOD_RES (13)..(13): D-from isoleucine
XNTWQXXXXKNNX

SEQ ID NO: 176 - protein, 13 aa, Artificial Sequence
  Synthesized peptide
  MOD_RES (1)..(1): L-Penicillamine
  MOD_RES (6)..(6): L-Penicillamine
  MOD_RES (7)..(7): 4-(2-aminoethoxy)-L-phenylalanine
  MOD_RES (8)..(8): L-2-Napthylalanine
  MOD_RES (9)..(9): alpha-methyl-L-Leucine
  MOD_RES (10)..(10): ACETYLATION
  MOD_RES (13)..(13): D-from alanine
XNTWQXXXXKNNX

SEQ ID NO: 177 - protein, 13 aa, Artificial Sequence
  Synthesized peptide
  MOD_RES (1)..(1): L-Penicillamine
  MOD_RES (6)..(6): L-Penicillamine
  MOD_RES (7)..(7): 4-(2-aminoethoxy)-L-phenylalanine
  MOD_RES (8)..(8): L-2-Napthylalanine
  MOD_RES (9)..(9): alpha-methyl-L-Leucine
  MOD_RES (10)..(10): ACETYLATION
  MOD_RES (13)..(13): D-from glutamine
XNTWQXXXXKNNX

SEQ ID NO: 178 - protein, 13 aa, Artificial Sequence
  Synthesized peptide
  MOD_RES (1)..(1): L-Penicillamine
  MOD_RES (6)..(6): L-Penicillamine
  MOD_RES (7)..(7): 4-(2-aminoethoxy)-L-phenylalanine
  MOD_RES (8)..(8): L-2-Napthylalanine
  MOD_RES (9)..(9): alpha-methyl-L-Leucine
  MOD_RES (10)..(10): ACETYLATION
  MOD_RES (13)..(13): D-from Serine
XNTWQXXXXKNNX

SEQ ID NO: 179 - protein, 13 aa, Artificial Sequence
  Synthesized peptide
  MOD_RES (1)..(1): ACETYLATION
  MOD_RES (2)..(2): L-Penicillamine
  MOD_RES (7)..(7): L-Penicillamine
  MOD_RES (8)..(8): 4-(2-aminoethoxy)-L-phenylalanine
  MOD_RES (9)..(9): L-2-Napthylalanine
  MOD_RES (10)..(10): alpha-methyl-L-Leucine
  MOD_RES (11)..(11): ACETYLATION
KXNTWQXXXXKNN

SEQ ID NO: 180 - protein, 13 aa, Artificial Sequence
  Synthesized peptide
  MOD_RES (1)..(1): ACETYLATION
  MOD_RES (2)..(2): L-Penicillamine
  MOD_RES (7)..(7): L-Penicillamine
  MOD_RES (8)..(8): 4-Carbamoyl-L-phenylalanine
  MOD_RES (9)..(9): L-2-Napthylalanine
  MOD_RES (10)..(10): alpha-methyl-L-Leucine
  MOD_RES (11)..(11): ACETYLATION
KXNTWQXXXXKNN

SEQ ID NO: 181 - protein, 13 aa, Artificial Sequence
  Synthesized peptide
  MOD_RES (1)..(1): L-Penicillamine
  MOD_RES (6)..(6): L-Penicillamine
  MOD_RES (7)..(7): 4-(2-aminoethoxy)-L-phenylalanine
  MOD_RES (8)..(8): L-2-Napthylalanine
  MOD_RES (9)..(9): alpha-methyl-L-Leucine
  MOD_RES (10)..(10): ACETYLATION
  MOD_RES (13)..(13): ACETYLATION
XNTWQXXXXKNNK

SEQ ID NO: 182 - protein, 13 aa, Artificial Sequence
  Synthesized peptide
  MOD_RES (1)..(1): L-Penicillamine
  MOD_RES (6)..(6): L-Penicillamine
  MOD_RES (7)..(7): 4-Carbamoyl-L-phenylalanine
  MOD_RES (8)..(8): L-2-Napthylalanine
  MOD_RES (9)..(9): alpha-methyl-L-Leucine
  MOD_RES (10)..(10): ACETYLATION
  MOD_RES (13)..(13): ACETYLATION
XNTWQXXXXKNNK

SEQ ID NO: 183 - protein, 13 aa, Artificial Sequence
  Synthesized peptide
  MOD_RES (1)..(1): L-Penicillamine
  MOD_RES (6)..(6): L-Penicillamine
  MOD_RES (7)..(7): 4-Carbamoyl-L-phenylalanine
  MOD_RES (8)..(8): L-2-Napthylalanine
  MOD_RES (9)..(9): alpha-methyl-L-Leucine
  MOD_RES (10)..(10): ACETYLATION
  MOD_RES (13)..(13): D-form lysine
XNTWQXXXXKNNX

SEQ ID NO: 184 - protein, 13 aa, Artificial Sequence
  Synthesized peptide
  MOD_RES (1)..(1): L-Penicillamine
  MOD_RES (6)..(6): L-Penicillamine
  MOD_RES (7)..(7): 4-Carbamoyl-L-phenylalanine
  MOD_RES (8)..(8): L-2-Napthylalanine
  MOD_RES (9)..(9): alpha-methyl-L-Leucine
  MOD_RES (10)..(10): ACETYLATION
  MOD_RES (13)..(13): D-form lysine
XNTWQXXXXKNNX

SEQ ID NO: 185 - protein, 12 aa, Artificial Sequence
  Synthesized peptide
  MOD_RES (1)..(1): L-Penicillamine
  MOD_RES (4)..(4): Trp(5-F)
  MOD_RES (6)..(6): L-Penicillamine
  MOD_RES (7)..(7): 4-(2-aminoethoxy)-L-phenylalanine
  MOD_RES (8)..(8): L-2-Napthylalanine
  MOD_RES (9)..(9): alpha-methyl-L-Leucine
  MOD_RES (10)..(10): ACETYLATION
XNTXQXXXXKNN

SEQ ID NO: 186 - protein, 12 aa, Artificial Sequence
  Synthesized peptide
  MOD_RES (1)..(1): L-Penicillamine
  MOD_RES (6)..(6): L-Penicillamine
  MOD_RES (7)..(7): 4-(2-aminoethoxy)-L-phenylalanine
  MOD_RES (8)..(8): L-2-Napthylalanine
  MOD_RES (9)..(9): alpha-methyl-L-Leucine
  MOD_RES (10)..(10): L-beta-homoglutamic acid
XNTWQXXXXXNN

SEQ ID NO: 187 - protein, 12 aa, Artificial Sequence
  Synthesized peptide
  MOD_RES (1)..(1): L-Penicillamine
  MOD_RES (6)..(6): L-Penicillamine
  MOD_RES (7)..(7): 4-(2-aminoethoxy)-L-phenylalanine
  MOD_RES (8)..(8): L-2-Napthylalanine
  MOD_RES (9)..(9): alpha-methyl-L-Leucine
XNTWQXXXXDNN

SEQ ID NO: 188 - protein, 12 aa, Artificial Sequence
  Synthesized peptide
  MOD_RES (1)..(1): L-Penicillamine
  MOD_RES (6)..(6): L-Penicillamine
  MOD_RES (7)..(7): 4-(2-aminoethoxy)-L-phenylalanine
  MOD_RES (8)..(8): L-2-Napthylalanine
  MOD_RES (9)..(9): alpha-methyl-L-Leucine
  MOD_RES (10)..(10): ACETYLATION
  MOD_RES (11)..(11): L-Citrulline
XNTWQXXXXKXN

SEQ ID NO: 189 - protein, 12 aa, Artificial Sequence
  Synthesized peptide
  MOD_RES (1)..(1): L-Penicillamine
  MOD_RES (6)..(6): L-Penicillamine
  MOD_RES (7)..(7): 4-(2-aminoethoxy)-L-phenylalanine
  MOD_RES (8)..(8): L-2-Napthylalanine
  MOD_RES (9)..(9): alpha-methyl-L-Leucine
  MOD_RES (10)..(10): ACETYLATION
  MOD_RES (12)..(12): L-Citrulline
XNTWQXXXXKNX

SEQ ID NO: 190 - protein, 12 aa, Artificial Sequence
  Synthesized peptide
  MOD_RES (1)..(1): L-Penicillamine
  MOD_RES (6)..(6): L-Penicillamine
  MOD_RES (7)..(7): 4-(2-aminoethoxy)-L-phenylalanine
  MOD_RES (8)..(8): L-2-Napthylalanine
  MOD_RES (9)..(9): alpha-methyl-L-Leucine
  MOD_RES (10)..(10): ACETYLATION
XNTWQXXXXKNG

SEQ ID NO: 191 - protein, 12 aa, Artificial Sequence
  Synthesized peptide
  MOD_RES (1)..(1): L-Penicillamine
  MOD_RES (5)..(5): L-Citrulline
  MOD_RES (6)..(6): L-Penicillamine
  MOD_RES (7)..(7): 4-(2-aminoethoxy)-L-phenylalanine
  MOD_RES (8)..(8): L-2-Napthylalanine
  MOD_RES (9)..(9): alpha-methyl-L-Leucine
  MOD_RES (10)..(10): ACETYLATION
XNTWXXXXXKNN

SEQ ID NO: 192 - protein, 12 aa, Artificial Sequence
  Synthesized peptide
  MOD_RES (1)..(1): L-Penicillamine
  MOD_RES (6)..(6): L-Penicillamine
  MOD_RES (7)..(7): 4-(2-aminoethoxy)-L-phenylalanine
  MOD_RES (8)..(8): L-2-Napthylalanine
  MOD_RES (9)..(9): alpha-methyl-L-Leucine
  MOD_RES (10)..(10): ACETYLATION
  MOD_RES (12)..(12): Sarcosine
XNTWQXXXXKNX

SEQ ID NO: 193 - protein, 12 aa, Artificial Sequence
  Synthesized peptide
  MOD_RES (1)..(1): L-Penicillamine
  MOD_RES (2)..(2): L-Citrulline
  MOD_RES (5)..(5): L-Citrulline
  MOD_RES (6)..(6): L-Penicillamine
  MOD_RES (7)..(7): 4-(2-aminoethoxy)-L-phenylalanine
  MOD_RES (8)..(8): L-2-Napthylalanine
  MOD_RES (9)..(9): alpha-methyl-L-Leucine
  MOD_RES (10)..(10): ACETYLATION
XXTWXXXXXKNN

SEQ ID NO: 194 - protein, 12 aa, Artificial Sequence
  Synthesized peptide
  MOD_RES (1)..(1): L-Penicillamine
  MOD_RES (6)..(6): L-Penicillamine
  MOD_RES (7)..(7): 4-(2-aminoethoxy)-L-phenylalanine
  MOD_RES (8)..(8): L-2-Napthylalanine
  MOD_RES (9)..(9): Deg
  MOD_RES (10)..(10): ACETYLATION
XNTWQXXXXKNN

SEQ ID NO: 195 - protein, 13 aa, Artificial Sequence
  Synthesized peptide
  MOD_RES (1)..(1): L-Penicillamine
  MOD_RES (5)..(5): ACETYLATION
  MOD_RES (6)..(6): L-Penicillamine
  MOD_RES (7)..(7): 4-(2-aminoethoxy)-L-phenylalanine
  MOD_RES (8)..(8): L-2-Napthylalanine
  MOD_RES (9)..(9): alpha-methyl-L-Leucine
  MOD_RES (10)..(10): ACETYLATION
XNTWKXXXXKNNG

SEQ ID NO: 196 - protein, 13 aa, Artificial Sequence
  Synthesized peptide
  MOD_RES (1)..(1): L-Penicillamine
  MOD_RES (5)..(5): ACETYLATION
  MOD_RES (6)..(6): L-Penicillamine
  MOD_RES (7)..(7): 4-(2-aminoethoxy)-L-phenylalanine
  MOD_RES (8)..(8): L-2-Napthylalanine
  MOD_RES (9)..(9): alpha-methyl-L-Leucine
  MOD_RES (10)..(10): ACETYLATION
  MOD_RES (13)..(13): beta-Alanine
XNTWKXXXXKNNX

SEQ ID NO: 197 - protein, 13 aa, Artificial Sequence
  Synthesized peptide
  MOD_RES (1)..(1): L-Penicillamine
  MOD_RES (5)..(5): ACETYLATION
  MOD_RES (6)..(6): L-Penicillamine
  MOD_RES (7)..(7): 4-(2-aminoethoxy)-L-phenylalanine
  MOD_RES (8)..(8): L-2-Napthylalanine
  MOD_RES (9)..(9): alpha-methyl-L-Leucine
  MOD_RES (10)..(10): ACETYLATION
  MOD_RES (13)..(13): 6-aminohexanoic acid
XNTWKXXXXKNNX

SEQ ID NO: 198 - protein, 13 aa, Artificial Sequence
  Synthesized peptide
  MOD_RES (1)..(1): L-Penicillamine
  MOD_RES (5)..(5): ACETYLATION
  MOD_RES (6)..(6): L-Penicillamine
  MOD_RES (7)..(7): 4-(2-aminoethoxy)-L-phenylalanine
  MOD_RES (8)..(8): L-2-Napthylalanine
  MOD_RES (9)..(9): alpha-methyl-L-Leucine
  MOD_RES (10)..(10): ACETYLATION
  MOD_RES (13)..(13): Sarcosine
XNTWKXXXXKNNX

SEQ ID NO: 199 - protein, 13 aa, Artificial Sequence
  Synthesized peptide
  MOD_RES (1)..(1): L-Penicillamine
  MOD_RES (5)..(5): ACETYLATION
  MOD_RES (6)..(6): L-Penicillamine
  MOD_RES (7)..(7): 4-(2-aminoethoxy)-L-phenylalanine
  MOD_RES (8)..(8): L-2-Napthylalanine
  MOD_RES (9)..(9): alpha-methyl-L-Leucine
  MOD_RES (10)..(10): ACETYLATION
  MOD_RES (13)..(13): D-form arginine
XNTWKXXXXKNNX

SEQ ID NO: 200 - protein, 13 aa, Artificial Sequence
  Synthesized peptide
  MOD_RES (1)..(1): L-Penicillamine
  MOD_RES (5)..(5): ACETYLATION
  MOD_RES (6)..(6): L-Penicillamine
  MOD_RES (7)..(7): 4-(2-aminoethoxy)-L-phenylalanine
  MOD_RES (8)..(8): L-2-Napthylalanine
  MOD_RES (9)..(9): alpha-methyl-L-Leucine
  MOD_RES (10)..(10): ACETYLATION
  MOD_RES (13)..(13): D-form isoleucine
XNTWKXXXXKNNX

SEQ ID NO: 201 - protein, 12 aa, Artificial Sequence
  Synthesized peptide
  MOD_RES (1)..(1): L-Penicillamine
  MOD_RES (6)..(6): L-Penicillamine
  MOD_RES (7)..(7): 4-(2-aminoethoxy)-L-phenylalanine
  MOD_RES (8)..(8): L-2-Napthylalanine
  MOD_RES (9)..(9): alpha-methyl-L-Leucine
XNTWQXXXXDNN

SEQ ID NO: 202 - protein, 12 aa, Artificial Sequence
  Synthesized peptide
  MOD_RES (1)..(1): L-Penicillamine
  MOD_RES (4)..(4): Trp(5-F)
  MOD_RES (5)..(5): ACETYLATION
  MOD_RES (6)..(6): L-Penicillamine
  MOD_RES (7)..(7): 4-(2-aminoethoxy)-L-phenylalanine
  MOD_RES (8)..(8): L-2-Napthylalanine
  MOD_RES (9)..(9): alpha-methyl-L-Leucine
  MOD_RES (10)..(10): ACETYLATION
XNTXKXXXXKNN

SEQ ID NO: 203 - protein, 13 aa, Artificial Sequence
  Synthesized peptide
  MOD_RES (1)..(1): L-Penicillamine
  MOD_RES (4)..(4): Trp(5-F)
  MOD_RES (5)..(5): ACETYLATION
  MOD_RES (6)..(6): L-Penicillamine
  MOD_RES (7)..(7): 4-(2-aminoethoxy)-L-phenylalanine
  MOD_RES (8)..(8): L-2-Napthylalanine
  MOD_RES (9)..(9): alpha-methyl-L-Leucine
  MOD_RES (10)..(10): ACETYLATION
XNTXKXXXXKNNG

SEQ ID NO: 204 - protein, 12 aa, Artificial Sequence
  Synthesized peptide
  MISC_FEATURE (1)..(12): Sequence dimerized via diglycolic acid linker
  MOD_RES (1)..(1): L-Penicillamine
  MOD_RES (5)..(5): ACETYLATION
  MOD_RES (6)..(6): L-Penicillamine
  MOD_RES (7)..(7): 4-(2-aminoethoxy)-L-phenylalanine
  MOD_RES (8)..(8): L-2-Napthylalanine
  MOD_RES (9)..(9): alpha-methyl-L-Leucine
  MOD_RES (10)..(10): ACETYLATION
XNTWKXXXXKNN

SEQ ID NO: 205 - protein, 12 aa, Artificial Sequence
  Synthesized peptide
  MISC_FEATURE (1)..(12): Sequence dimerized via Iminodiacetic acid linker
  MOD_RES (1)..(1): L-Penicillamine
  MOD_RES (5)..(5): ACETYLATION
  MOD_RES (6)..(6): L-Penicillamine
  MOD_RES (7)..(7): 4-(2-aminoethoxy)-L-phenylalanine
  MOD_RES (8)..(8): L-2-Napthylalanine
  MOD_RES (9)..(9): alpha-methyl-L-Leucine
  MOD_RES (10)..(10): ACETYLATION
XNTWKXXXXKNN

SEQ ID NO: 206 - protein, 12 aa, Artificial Sequence
  Synthesized peptide
  MISC_FEATURE (1)..(12): Sequence dimerized via PEG2 linker
  MOD_RES (1)..(1): L-Penicillamine
  MOD_RES (5)..(5): ACETYLATION
  MOD_RES (6)..(6): L-Penicillamine
  MOD_RES (7)..(7): 4-(2-aminoethoxy)-L-phenylalanine
  MOD_RES (8)..(8): L-2-Napthylalanine
  MOD_RES (9)..(9): alpha-methyl-L-Leucine
  MOD_RES (10)..(10): ACETYLATION
XNTWKXXXXKNN

SEQ ID NO: 207 - protein, 12 aa, Artificial Sequence
  Synthesized peptide
  MISC_FEATURE (1)..(12): Sequence dimerized via PEG4 linker
  MOD_RES (1)..(1): L-Penicillamine
  MOD_RES (5)..(5): ACETYLATION
  MOD_RES (6)..(6): L-Penicillamine
  MOD_RES (7)..(7): 4-(2-aminoethoxy)-L-phenylalanine
  MOD_RES (8)..(8): L-2-Napthylalanine
  MOD_RES (9)..(9): alpha-methyl-L-Leucine
  MOD_RES (10)..(10): ACETYLATION
XNTWKXXXXKNN

SEQ ID NO: 208 - protein, 12 aa, Artificial Sequence
  Synthesized peptide
  MISC_FEATURE (1)..(12): Sequence dimerized via PEG13 linker
  MOD_RES (1)..(1): L-Penicillamine
  MOD_RES (5)..(5): ACETYLATION
  MOD_RES (6)..(6): L-Penicillamine
  MOD_RES (7)..(7): 4-(2-aminoethoxy)-L-phenylalanine
  MOD_RES (8)..(8): L-2-Napthylalanine
  MOD_RES (9)..(9): alpha-methyl-L-Leucine
  MOD_RES (10)..(10): ACETYLATION
XNTWKXXXXKNN

SEQ ID NO: 209 - protein, 13 aa, Artificial Sequence
  Synthesized peptide
  MOD_RES (1)..(1): L-Penicillamine
  MOD_RES (5)..(5): ACETYLATION
  MOD_RES (6)..(6): L-Penicillamine
  MOD_RES (7)..(7): 4-(2-aminoethoxy)-L-phenylalanine
  MOD_RES (8)..(8): L-2-Napthylalanine
  MOD_RES (9)..(9): alpha-methyl-L-Leucine
  MOD_RES (10)..(10): acetyl - arginine conjugation
  MOD_RES (13)..(13): D-form isoleucine
XNTWKXXXXKNNX

SEQ ID NO: 210 - protein, 13 aa, Artificial Sequence
  Synthesized peptide
  MOD_RES (1)..(1): L-Penicillamine
  MOD_RES (5)..(5): ACETYLATION
  MOD_RES (6)..(6): L-Penicillamine
  MOD_RES (7)..(7): 4-(2-aminoethoxy)-L-phenylalanine
  MOD_RES (8)..(8): L-2-Napthylalanine
  MOD_RES (9)..(9): alpha-methyl-L-Leucine
  MOD_RES (10)..(10): acetyl - tyrosine conjugation
  MOD_RES (13)..(13): D-form isoleucine
XNTWKXXXXKNNX

SEQ ID NO: 211 - protein, 13 aa, Artificial Sequence
  Synthesized peptide
  MOD_RES (1)..(1): L-Penicillamine
  MOD_RES (5)..(5): ACETYLATION
  MOD_RES (6)..(6): L-Penicillamine
  MOD_RES (7)..(7): 4-(2-aminoethoxy)-L-phenylalanine
  MOD_RES (8)..(8): L-2-Napthylalanine
  MOD_RES (9)..(9): alpha-methyl-L-Leucine
  MOD_RES (10)..(10): acetyl - asparigine conjugation
  MOD_RES (13)..(13): D-form isoleucine
XNTWKXXXXKNNX

SEQ ID NO: 212 - protein, 13 aa, Artificial Sequence
  Synthesized peptide
  MOD_RES (1)..(1): L-Penicillamine
  MOD_RES (5)..(5): ACETYLATION
  MOD_RES (6)..(6): L-Penicillamine
  MOD_RES (7)..(7): 4-(2-aminoethoxy)-L-phenylalanine
  MOD_RES (8)..(8): L-2-Napthylalanine
  MOD_RES (9)..(9): alpha-methyl-L-Leucine
  MOD_RES (10)..(10): acetyl - threonine conjugation
  MOD_RES (13)..(13): D-form isoleucine
XNTWKXXXXKNNX

SEQ ID NO: 213 - protein, 13 aa, Artificial Sequence
  Synthesized peptide
  MOD_RES (1)..(1): L-Penicillamine
  MOD_RES (5)..(5): ACETYLATION
  MOD_RES (6)..(6): L-Penicillamine
  MOD_RES (7)..(7): 4-(2-aminoethoxy)-L-phenylalanine
  MOD_RES (8)..(8): L-2-Napthylalanine
  MOD_RES (9)..(9): alpha-methyl-L-Leucine
  MOD_RES (10)..(10): acetyl - aspartic acid conjugation
  MOD_RES (13)..(13): D-form isoleucine
XNTWKXXXXKNNX

SEQ ID NO: 214 - protein, 13 aa, Artificial Sequence
  Synthesized peptide
  MOD_RES (1)..(1): L-Penicillamine
  MOD_RES (5)..(5): ACETYLATION
  MOD_RES (6)..(6): L-Penicillamine
  MOD_RES (7)..(7): 4-(2-aminoethoxy)-L-phenylalanine
  MOD_RES (8)..(8): L-2-Napthylalanine
  MOD_RES (9)..(9): alpha-methyl-L-Leucine
  MOD_RES (10)..(10): acetyl - leucine conjugation
  MOD_RES (13)..(13): D-form isoleucine
XNTWKXXXXKNNX

SEQ ID NO: 215 - protein, 13 aa, Artificial Sequence
  Synthesized peptide
  MOD_RES (1)..(1): L-Penicillamine
  MOD_RES (5)..(5): ACETYLATION
  MOD_RES (6)..(6): L-Penicillamine
  MOD_RES (7)..(7): 4-(2-aminoethoxy)-L-phenylalanine
  MOD_RES (8)..(8): L-2-Napthylalanine
  MOD_RES (9)..(9): alpha-methyl-L-Leucine
  MOD_RES (10)..(10): acetyl - phenylalanine conjugation
  MOD_RES (13)..(13): D-form isoleucine
XNTWKXXXXKNNX

SEQ ID NO: 216 - protein, 13 aa, Artificial Sequence
  Synthesized peptide
  MOD_RES (1)..(1): L-Penicillamine
  MOD_RES (5)..(5): ACETYLATION
  MOD_RES (6)..(6): L-Penicillamine
  MOD_RES (7)..(7): 4-(2-aminoethoxy)-L-phenylalanine
  MOD_RES (8)..(8): L-2-Napthylalanine
  MOD_RES (9)..(9): alpha-methyl-L-Leucine
  MOD_RES (10)..(10): acetyl - D-form arginine conjugation
  MOD_RES (13)..(13): D-form isoleucine
XNTWKXXXXKNNX

SEQ ID NO: 217 - protein, 13 aa, Artificial Sequence
  Synthesized peptide
  MOD_RES (1)..(1): L-Penicillamine
  MOD_RES (5)..(5): ACETYLATION
  MOD_RES (6)..(6): L-Penicillamine
  MOD_RES (7)..(7): 4-(2-aminoethoxy)-L-phenylalanine
  MOD_RES (8)..(8): L-2-Napthylalanine
  MOD_RES (9)..(9): alpha-methyl-L-Leucine
  MOD_RES (10)..(10): acetyl - D-form tyrosine conjugation
  MOD_RES (13)..(13): D-form isoleucine
XNTWKXXXXKNNX

SEQ ID NO: 218 - protein, 13 aa, Artificial Sequence
  Synthesized peptide
  MOD_RES (1)..(1): L-Penicillamine
  MOD_RES (5)..(5): ACETYLATION
  MOD_RES (6)..(6): L-Penicillamine
  MOD_RES (7)..(7): 4-(2-aminoethoxy)-L-phenylalanine
  MOD_RES (8)..(8): L-2-Napthylalanine
  MOD_RES (9)..(9): alpha-methyl-L-Leucine
  MOD_RES (10)..(10): acetyl - D-form asparigine conjugation
  MOD_RES (13)..(13): D-form isoleucine
XNTWKXXXXKNNX

SEQ ID NO: 219 - protein, 13 aa, Artificial Sequence
  Synthesized peptide
  MOD_RES (1)..(1): L-Penicillamine
  MOD_RES (5)..(5): ACETYLATION
  MOD_RES (6)..(6): L-Penicillamine
  MOD_RES (7)..(7): 4-(2-aminoethoxy)-L-phenylalanine
  MOD_RES (8)..(8): L-2-Napthylalanine
  MOD_RES (9)..(9): alpha-methyl-L-Leucine
  MOD_RES (10)..(10): acetyl - D-form threonine conjugation
  MOD_RES (13)..(13): D-form isoleucine
XNTWKXXXXKNNX

SEQ ID NO: 220 - protein, 13 aa, Artificial Sequence
  Synthesized peptide
  MOD_RES (1)..(1): L-Penicillamine
  MOD_RES (5)..(5): ACETYLATION
  MOD_RES (6)..(6): L-Penicillamine
  MOD_RES (7)..(7): 4-(2-aminoethoxy)-L-phenylalanine
  MOD_RES (8)..(8): L-2-Napthylalanine
  MOD_RES (9)..(9): alpha-methyl-L-Leucine
  MOD_RES (10)..(10): acetyl - D-form aspartic acid conjugation
  MOD_RES (13)..(13): D-form isoleucine
XNTWKXXXXKNNX

SEQ ID NO: 221 - protein, 13 aa, Artificial Sequence
  Synthesized peptide
  MOD_RES (1)..(1): L-Penicillamine
  MOD_RES (5)..(5): ACETYLATION
  MOD_RES (6)..(6): L-Penicillamine
  MOD_RES (7)..(7): 4-(2-aminoethoxy)-L-phenylalanine
  MOD_RES (8)..(8): L-2-Napthylalanine
  MOD_RES (9)..(9): alpha-methyl-L-Leucine
  MOD_RES (10)..(10): acetyl - D-form leucine conjugation
  MOD_RES (13)..(13): D-form isoleucine
XNTWKXXXXKNNX

SEQ ID NO: 222 - protein, 13 aa, Artificial Sequence
  Synthesized peptide
  MOD_RES (1)..(1): L-Penicillamine
  MOD_RES (5)..(5): ACETYLATION
  MOD_RES (6)..(6): L-Penicillamine
  MOD_RES (7)..(7): 4-(2-aminoethoxy)-L-phenylalanine
  MOD_RES (8)..(8): L-2-Napthylalanine
  MOD_RES (9)..(9): alpha-methyl-L-Leucine
  MOD_RES (10)..(10): acetyl - D-form arginine conjugation
  MOD_RES (10)..(10): acetyl - D-form phenylalanine conjugation
  MOD_RES (13)..(13): D-form isoleucine
XNTWKXXXXKNNX

SEQ ID NO: 223 - protein, 13 aa, Artificial Sequence
  Synthesized peptide
  MOD_RES (1)..(1): acetyl - glutamic acid conjugation
  MOD_RES (2)..(2): L-Penicillamine
  MOD_RES (6)..(6): ACETYLATION
  MOD_RES (7)..(7): L-Penicillamine
  MOD_RES (8)..(8): 4-(2-aminoethoxy)-L-phenylalanine
  MOD_RES (9)..(9): L-2-Napthylalanine
  MOD_RES (10)..(10): alpha-methyl-L-Leucine
  MOD_RES (11)..(11): ACETYLATION
KXNTWKXXXXKNN

SEQ ID NO: 224 - protein, 13 aa, Artificial Sequence
  Synthesized peptide
  MOD_RES (1)..(1): acetyl - phenylalanine conjugation
  MOD_RES (2)..(2): L-Penicillamine
  MOD_RES (6)..(6): ACETYLATION
  MOD_RES (7)..(7): L-Penicillamine
  MOD_RES (8)..(8): 4-(2-aminoethoxy)-L-phenylalanine
  MOD_RES (9)..(9): L-2-Napthylalanine
  MOD_RES (10)..(10): alpha-methyl-L-Leucine
  MOD_RES (11)..(11): ACETYLATION
KXNTWKXXXXKNN

SEQ ID NO: 225 - protein, 13 aa, Artificial Sequence
  Synthesized peptide
  MOD_RES (1)..(1): acetyl - tyrosine conjugation
  MOD_RES (2)..(2): L-Penicillamine
  MOD_RES (6)..(6): ACETYLATION
  MOD_RES (7)..(7): L-Penicillamine
  MOD_RES (8)..(8): 4-(2-aminoethoxy)-L-phenylalanine
  MOD_RES (9)..(9): L-2-Napthylalanine
  MOD_RES (10)..(10): alpha-methyl-L-Leucine
  MOD_RES (11)..(11): ACETYLATION
KXNTWKXXXXKNN

SEQ ID NO: 226 - protein, 13 aa, Artificial Sequence
  Synthesized peptide
  MOD_RES (1)..(1): acetyl - Serine conjugation
  MOD_RES (2)..(2): L-Penicillamine
  MOD_RES (6)..(6): ACETYLATION
  MOD_RES (7)..(7): L-Penicillamine
  MOD_RES (8)..(8): 4-(2-aminoethoxy)-L-phenylalanine
  MOD_RES (9)..(9): L-2-Napthylalanine
  MOD_RES (10)..(10): alpha-methyl-L-Leucine
  MOD_RES (11)..(11): ACETYLATION
KXNTWKXXXXKNN

SEQ ID NO: 227 - protein, 13 aa, Artificial Sequence
  Synthesized peptide
  MOD_RES (1)..(1): acetyl - arginine conjugation
  MOD_RES (2)..(2): L-Penicillamine
  MOD_RES (6)..(6): ACETYLATION
  MOD_RES (7)..(7): L-Penicillamine
  MOD_RES (8)..(8): 4-(2-aminoethoxy)-L-phenylalanine
  MOD_RES (9)..(9): L-2-Napthylalanine
  MOD_RES (10)..(10): alpha-methyl-L-Leucine
  MOD_RES (11)..(11): ACETYLATION
KXNTWKXXXXKNN

SEQ ID NO: 228 - protein, 13 aa, Artificial Sequence
  Synthesized peptide
  MOD_RES (1)..(1): acetyl - leucine conjugation
  MOD_RES (2)..(2): L-Penicillamine
  MOD_RES (6)..(6): ACETYLATION
  MOD_RES (7)..(7): L-Penicillamine
  MOD_RES (8)..(8): 4-(2-aminoethoxy)-L-phenylalanine
  MOD_RES (9)..(9): L-2-Napthylalanine
  MOD_RES (10)..(10): alpha-methyl-L-Leucine
  MOD_RES (11)..(11): ACETYLATION
KXNTWKXXXXKNN

SEQ ID NO: 229 - protein, 13 aa, Artificial Sequence
  Synthesized peptide
  MOD_RES (1)..(1): acetyl - proline conjugation
  MOD_RES (2)..(2): L-Penicillamine
  MOD_RES (6)..(6): ACETYLATION
  MOD_RES (7)..(7): L-Penicillamine
  MOD_RES (8)..(8): 4-(2-aminoethoxy)-L-phenylalanine
  MOD_RES (9)..(9): L-2-Napthylalanine
  MOD_RES (10)..(10): alpha-methyl-L-Leucine
  MOD_RES (11)..(11): ACETYLATION
KXNTWKXXXXKNN

SEQ ID NO: 230 - protein, 13 aa, Artificial Sequence
  Synthesized peptide
  MOD_RES (1)..(1): D-form lysine with acetyl - glutamic acid conjugation
  MOD_RES (2)..(2): L-Penicillamine
  MOD_RES (6)..(6): ACETYLATION
  MOD_RES (7)..(7): L-Penicillamine
  MOD_RES (8)..(8): 4-(2-aminoethoxy)-L-phenylalanine
  MOD_RES (9)..(9): L-2-Napthylalanine
  MOD_RES (10)..(10): alpha-methyl-L-Leucine
  MOD_RES (11)..(11): ACETYLATION
XXNTWKXXXXKNN

SEQ ID NO: 231 - protein, 13 aa, Artificial Sequence
  Synthesized peptide
  MOD_RES (1)..(1): D-form lysine with acetyl - phenylalanine conjugation
  MOD_RES (2)..(2): L-Penicillamine
  MOD_RES (6)..(6): ACETYLATION
  MOD_RES (7)..(7): L-Penicillamine
  MOD_RES (8)..(8): 4-(2-aminoethoxy)-L-phenylalanine
  MOD_RES (9)..(9): L-2-Napthylalanine
  MOD_RES (10)..(10): alpha-methyl-L-Leucine
  MOD_RES (11)..(11): ACETYLATION
XXNTWKXXXXKNN

SEQ ID NO: 232 - protein, 13 aa, Artificial Sequence
  Synthesized peptide
  MOD_RES (1)..(1): D-form lysine with acetyl - tyrosine conjugation
  MOD_RES (2)..(2): L-Penicillamine
  MOD_RES (6)..(6): ACETYLATION
  MOD_RES (7)..(7): L-Penicillamine
  MOD_RES (8)..(8): 4-(2-aminoethoxy)-L-phenylalanine
  MOD_RES (9)..(9): L-2-Napthylalanine
  MOD_RES (10)..(10): alpha-methyl-L-Leucine
  MOD_RES (11)..(11): ACETYLATION
XXNTWKXXXXKNN

SEQ ID NO: 233 - protein, 13 aa, Artificial Sequence
  Synthesized peptide
  MOD_RES (1)..(1): D-form lysine with acetyl - serine conjugation
  MOD_RES (2)..(2): L-Penicillamine
  MOD_RES (6)..(6): ACETYLATION
  MOD_RES (7)..(7): L-Penicillamine
  MOD_RES (8)..(8): 4-(2-aminoethoxy)-L-phenylalanine
  MOD_RES (9)..(9): L-2-Napthylalanine
  MOD_RES (10)..(10): alpha-methyl-L-Leucine
  MOD_RES (11)..(11): ACETYLATION
XXNTWKXXXXKNN

SEQ ID NO: 234 - protein, 13 aa, Artificial Sequence
  Synthesized peptide
  MOD_RES (1)..(1): D-form lysine with acetyl - arginine conjugation
  MOD_RES (2)..(2): L-Penicillamine
  MOD_RES (6)..(6): ACETYLATION
  MOD_RES (7)..(7): L-Penicillamine
  MOD_RES (8)..(8): 4-(2-aminoethoxy)-L-phenylalanine
  MOD_RES (9)..(9): L-2-Napthylalanine
  MOD_RES (10)..(10): alpha-methyl-L-Leucine
  MOD_RES (11)..(11): ACETYLATION
XXNTWKXXXXKNN

SEQ ID NO: 235 - protein, 13 aa, Artificial Sequence
  Synthesized peptide
  MOD_RES (1)..(1): D-form lysine with acetyl - leucine conjugation
  MOD_RES (2)..(2): L-Penicillamine
  MOD_RES (6)..(6): ACETYLATION
  MOD_RES (7)..(7): L-Penicillamine
  MOD_RES (8)..(8): 4-(2-aminoethoxy)-L-phenylalanine
  MOD_RES (9)..(9): L-2-Napthylalanine
  MOD_RES (10)..(10): alpha-methyl-L-Leucine
  MOD_RES (11)..(11): ACETYLATION
XXNTWKXXXXKNN

SEQ ID NO: 236 - protein, 13 aa, Artificial Sequence
  Synthesized peptide
  MOD_RES (1)..(1): D-form lysine with acetyl - proline conjugation
  MOD_RES (2)..(2): L-Penicillamine
  MOD_RES (6)..(6): ACETYLATION
  MOD_RES (7)..(7): L-Penicillamine
  MOD_RES (8)..(8): 4-(2-aminoethoxy)-L-phenylalanine
  MOD_RES (9)..(9): L-2-Napthylalanine
  MOD_RES (10)..(10): alpha-methyl-L-Leucine
  MOD_RES (11)..(11): ACETYLATION
XXNTWKXXXXKNN

SEQ ID NO: 237 - protein, 24 aa, Artificial Sequence
  Synthetic peptide motif
  MOD_RES (1)..(1): Xaa is Gly, Arg, Phe, Glu, Gln, Thr, (D)Arg, (D)Phe, (D)Glu, (D)Thr, (D)Leu, (D)Gln, alpha-MeArg, alpha-MePhe, alpha-MeLeu, alpha-MeLys, alpha-MeAsn, alpha-MeTyr, or absent
  MOD_RES (2)..(2): Xaa is Gly, Arg, Phe, Glu, Gln, Thr, (D)Arg, (D)Phe, (D)Glu, (D)Thr, (D)Leu, (D)Gln, alpha-MeArg, alpha-MePheMePhe, alpha-MeLeu, alpha-MeLys, alpha-MeAsn, alpha-MeTyr, or absent
  MOD_RES (3)..(3): Xaa is (D)Asp, Arg, (D)Arg, Phe, (D)Phe, 2-Nal, Thr, Leu, (D)Gln, (D)Asn, IsoGlu, Gly, Arg, Phe, Glu, Gln, Thr, (D)Glu, (D)Thr, (D)Leu, alpha-MeArg, alpha-MePhe, alpha-MeLeu, alpha-MeLys, alpha-MeAsn, alpha-MeTyr, or absent
  MOD_RES (4)..(4): Xaa is ((D)Arg, (D)Tyr, Gly, alpha-MeArg, alpha-MePhe, alpha-MeLeu, alpha-MeLys, alpha-MeAsn, alpha-MeTyr, or absent
  MOD_RES (5)..(5): Xaa is (Abu, Cys, (D)Cys, alpha-MeCys, (D)Abu, (D)Pen, or Pe
  MISC_FEATURE (5)..(10): synthesized peptide inhibitor is cyclized via a bond between postions 5 and 10
  MOD_RES (6)..(6): Xaa is Cit, Glu, Gly, Lys, Asn, Pro, alpha-MeGln, alpha-MeLys, alpha-MeLeu, alpha-MeAsn, Lys(Ac), alpha-MeLys(Ac), Dab(Ac), Dap(Ac), homo-Lys(Ac), or Gln
  MOD_RES (7)..(7): Xaa is Thr, Aib, Asp, Dab, Gly, Pro, Ser, alpha-MeGln, alpha-MeLys, alpha-MeLeu, alpha-MeAsn, alpha-MeThr, alpha-MeSer, or Val
  MOD_RES (8)..(8): Xaa is Trp, Trp(5-F), 1-Nal, 2-Nal, Phe(2-Me), Phe(3-Me), Phe(4-Me), Trp(7-Aza), or Phe(3,4-dimethoxy)
  MOD_RES (9)..(9): Xaa is Gln, alpha-Me-Lys, alpha-MeLeu, alpha-MeLys(Ac), beta-homoGln, Cit, Glu, Phe, Asn, Thr, Val, Aib, alpha-MeGln, alpha-MeAsn, Lys(Ac), alpha-MeLys(Ac), Dab(Ac), Dap(Ac), homo-Lys(Ac),or Trp
  MOD_RES (10)..(10): Xaa is Cys, (D)Cys), alpha-MeCys, (D)Abu, (D)Pen, Pen or Abu
  MOD_RES (11)..(11): Xaa is Phe, Phe[4-(2-aminoethoxy)], Phe[4-(2-acetylaminoethoxy)], alpha-MeTyr, or Phe(4-CONH2)
  MOD_RES (12)..(12): Xaa is 2-Nal, Trp, Trp(5-F), Trp(7-Aza), Phe(2-Me), Phe(3-Me), Phe(4-Me), Phe(3,4-dimethoxy), or 1-Nal
  MOD_RES (13)..(13): Xaa is 4-amino-4-carboxy-tetrahydropyran (THP), alpha-MeLys, alpha-MeLeu, alpha-MeArg, alpha-MePhe, alpha-MeLeu, alpha-MeLys, alpha-MeAsn, alpha-MeTyr, or Aib
  MOD_RES (14)..(14): Xaa is Glu, Cit, Gln, alpha-MeArg, alpha-MeGlu, alpha-MeLeu, alpha-MeLys, alpha-Me-Asn, Lys(Ac), alpha-MeLys(Ac), Dab(Ac), Dap(Ac), homo-Lys(Ac), or Lys
  MOD_RES (15)..(15): Xaa is Asn, 2-Nap, Aib, Arg, Cit, Asp, Phe, Gly, Lys, Leu, Asn, n-Leu, Gln, Ser, Tic, Trp, alpha-MeGln, alpha-MeAsn, alpha-MeLys(Ac), Dab(Ac), Dap(Ac), homo-Lys(Ac),or Lys(Ac)
  MOD_RES (16)..(16): Xaa is Asn, Aib, beta-Ala, Cit, Gln, Asp, alpha-MeGln, alpha-MeAsn, Lys(Ac), alpha-MeLys(Ac), Dab(Ac), Dap(Ac), homo-Lys(Ac),or absent
  MOD_RES (17)..(17): Xaa is Glu, Phe, Lys, Asn, Trp, Gly, Thr, Pro, (D)Arg, (D)Phe, (D)Glu, (D)Thr, (D)Leu, (D)Gln, alpha-MeArg, alpha-MePhe, alpha-MeLeu, alpha-MeLys, alpha-MeAsn, alpha-MeTyr, alpha-MeAsp, or absent
  MOD_RES (18)..(18): Xaa is Lys, Gly, Pro, The, Phe, Trp, Gln, (D)Arg, (D)Phe, (D)Glu, (D)Thr, (D)Leu, (D)Gln, alpha-MeArg, alpha-MePhe, alpha-MeLeu, alpha-MeLys, alpha-MeAsn, alpha-MeTyr, alpha-MeAsp, or absent
  MOD_RES (19)..(19): Xaa is Gly, Lys, Glu, Phe, Thr, Arg, Gln, (D)Arg, (D)Phe, (D)Glu, (D)Thr, (D)Leu, (D)Gln, alpha-MeArg, alpha-MePhe, alpha-MeLeu, alpha-MeLys, alpha-MeAsn, alpha-MeTyr, alpha-MeAsp, or absent
  MOD_RES (20)..(20): Xaa is Arg, Phe, Glu, Gln, Thr, (D)Arg, (D)Phe, (D)Glu, (D)Thr, (D)Leu, (D)Gln , alpha-MeArg, alpha-MePhe, alpha-MeLeu, alpha-MeLys, alpha-MeAsn, alpha-MeTyr, alpha-MeAsp, or absent
  MOD_RES (21)..(21): Xaa is Arg, Phe, Glu, Gln, Thr, (D)Arg, (D)Phe, (D)Glu, (D)Thr, (D)Leu, (D)Gln , alpha-MeArg, alpha-MePhe, alpha-MeLeu, alpha-MeLys, alpha-MeAsn, alpha-MeTyr, alpha-MeAsp, or absent
  MOD_RES (22)..(22): Xaa is Arg, Phe, Glu, Gln, Thr, (D)Arg, (D)Phe, (D)Glu, (D)Thr, (D)Leu, (D)Gln , alpha-MeArg, alpha-MePhe, alpha-MeLeu, alpha-MeLys, alpha-MeAsn, alpha-MeTyr, alpha-MeAsp, or absent
  MOD_RES (23)..(23): Xaa is Arg, Phe, Glu, Gln, Thr, (D)Arg, (D)Phe, (D)Glu, (D)Thr, (D)Leu, (D)Gln , alpha-MeArg, alpha-MePhe, alpha-MeLeu, alpha-MeLys, alpha-MeAsn, alpha-MeTyr, alpha-MeAsp, or absent
  MOD_RES (24)..(24): Xaa is Arg, Phe, Glu, Gln, Thr, (D)Arg, (D)Phe, (D)Glu, (D)Thr, (D)Leu, (D)Gln , alpha-MeArg, alpha-MePhe, alpha-MeLeu, alpha-MeLys, alpha-MeAsn, alpha-MeTyr, alpha-MeAsp, or absent
XXXXXXXXXXXXXXXXXXXXXXXX

SEQ ID NO: 238 - protein, 24 aa, Artificial Sequence
  Synthetic peptide motif
  MOD_RES (1)..(1): Xaa is Gly, Arg, Phe, Glu, Gln, Thr, (D)Arg, (D)Phe, (D)Glu, (D)Thr, (D)Leu, (D)Gln, alpha-MeArg, alpha-MePhe, alpha-MeLeu, alpha-MeLys, alpha-MeAsn, alpha-MeTyr, or absent
  MOD_RES (2)..(2): Xaa is Gly, Arg, Phe, Glu, Gln, Thr, (D)Arg, (D)Phe, (D)Glu, (D)Thr, (D)Leu, (D)Gln, alpha-MeArg, alpha-MePhe, alpha-MeLeu, alpha-MeLys, alpha-MeAsn, alpha-MeTyr, or absent
  MOD_RES (3)..(3): Xaa is (D)Asp, Arg, (D)Arg, Phe, (D)Phe, 2-Nal, Thr, Leu, (D)Gln, (D)Asn, IsoGlu, Gly, Arg, Phe, Glu, Gln, Thr, (D)Glu, (D)Thr, (D)Leu, alpha-MeArg, alpha-MePhe, alpha-MeLeu, alpha-MeLys, alpha-MeAsn, alpha-MeTyr, or absent
  MOD_RES (4)..(4): Xaa is (D)Arg, (D)Tyr, Gly, alpha-MeArg, alpha-MePhe, alpha-MeLeu, alpha-MeLys, alpha-MeAsn, alpha-MeTyr, or absent
  MOD_RES (5)..(5): Abu, Cys, (D)Cys), alpha-MeCys, (D)Abu, (D)Pen, or Pen; or X4 is Pen(sulfoxide)
  MISC_FEATURE (5)..(10): synthesized peptide inhibitor is cyclized via a bond between postions 5 and 10
  MOD_RES (6)..(6): Xaa is Cit, Glu, Gly, Lys, Asn, Pro, alpha-MeGln, alpha-MeLys, alpha-MeLeu, alpha-MeAsn, Lys(Ac), alpha-MeLys(Ac), Dab(Ac), Dap(Ac), homo-Lys(Ac), or Gln; or X5 is Asp, or Cys
  MOD_RES (7)..(7): Xaa is Thr, Aib, Asp, Dab, Gly, Pro, Ser, alpha-MeGln, alpha-MeLys, alpha-MeLeu, alpha-MeAsn, alpha-MeThr, alpha-MeSer, or Val
  MOD_RES (8)..(8): Xaa is Trp, Trp(5-F), 1-Nal, 2-Nal, Phe(2-Me), Phe(3-Me), Phe(4-Me), Trp(7-Aza), or Phe(3,4-dimethoxy)
  MOD_RES (9)..(9): Xaa is Gln, alpha-Me-Lys, alpha-MeLeu, alpha-MeLys(Ac), beta-homoGln, Cit, Glu, Phe, Asn, Thr, Val, Aib, alpha-MeGln, alpha-MeAsn, Lys(Ac), alpha-MeLys(Ac), Dab(Ac), Dap(Ac), homo-Lys(Ac), or Trp; or X8 is 1-Nal, or 2-Nal
  MOD_RES (10)..(10): Xaa is Cys, (D)Cys), alpha-MeCys, (D)Abu, (D)Pen, Pen or Abu
  MOD_RES (11)..(11): Xaa is Phe, Phe[4-(2-aminoethoxy)], Phe[4-(2-acetylaminoethoxy)], alpha-MeTyr, or Phe(4-CONH2)
  MOD_RES (12)..(12): Xaa is 2-Nal, Trp, Trp(5-F), Trp(7-Aza), Phe(2-Me), Phe(3-Me), Phe(4-Me), Phe(3,4-dimethoxy), or 1-Nal
  MOD_RES (13)..(13): Xaa is 4-amino-4-carboxy-tetrahydropyran (THP), alpha-MeLys, alpha-MeLeu, alpha-MeArg, alpha-MePhe, alpha-MeLeu, alpha-MeLys, alpha-MeAsn, alpha-MeTyr, or Aib; or X12 is Ala, or cyclohexylAla, Lys , pegylated Lys, or Deg
  MOD_RES (14)..(14): Xaa is Glu, Cit, Gln, Lys(Ac), alpha-MeArg, alpha-MeGlu, alpha-MeLeu, alpha-MeLys, alpha-Me-Asn, alpha-MeLys(Ac), Dab(Ac), Dap(Ac), homo-Lys(Ac), or Lys; or X13 is Lys, pegylated Lys, b-homoGlu, or Lys(Y2-Ac); ), wherein Y2 is an amino acid
  MOD_RES (15)..(15): Xaa is Asn, 2-Nap, Aib, Arg, Cit, Asp, Phe, Gly, Lys, Leu, Asn, n-Leu, Gln, Ser, Tic, Trp, alpha-MeGln, alpha-MeAsn, alpha-MeLys(Ac), Dab(Ac), Dap(Ac), homo-Lys(Ac), or Lys(Ac)
  MOD_RES (16)..(16): Xaa is Asn, Aib, beta-Ala, Cit, Gln, Asp, alpha-MeGln, alpha-MeAsn, Lys(Ac), alpha-MeLys(Ac), Dab(Ac), Dap(Ac), homo-Lys(Ac), or absent
  MOD_RES (17)..(17): Xaa is Glu, Phe, Lys, Asn, Trp, Gly, Thr, Pro, (D)Arg, (D)Phe, (D)Glu, (D)Thr, (D)Leu, (D)Gln, alpha-MeArg, alpha-MePhe, alpha-MeLeu, alpha-MeLys, alpha-MeAsn, alpha-MeTyr, alpha-MeAsp, or absent; or X16 is Ala, Asp, Tyr, Arg, Leu, Gln, Ser, Ile,
  MOD_RES (17)..(17): Continued: (D)Ala, (D)Asp, (D)Tyr, (D)Arg, (D)Leu, (D)Ser, or (D)Ile
  MOD_RES (18)..(18): Xaa is Lys, Gly, Pro, The, Phe, Trp, Gln, (D)Arg, (D)Phe, (D)Glu, (D)Thr, (D)Leu, (D)Gln, alpha-MeArg, alpha-MePhe, alpha-MeLeu, alpha-MeLys, alpha-MeAsn, alpha-MeTyr, alpha-MeAsp, or absent
  MOD_RES (19)..(19): Xaa is Gly, Lys, Glu, Phe, Thr, Arg, Gln, (D)Arg, (D)Phe, (D)Glu, (D)Thr, (D)Leu, (D)Gln, alpha-MeArg, alpha-MePhe, alpha-MeLeu, alpha-MeLys, alpha-MeAsn, alpha-MeTyr, alpha-MeAsp, or absent
  MOD_RES (20)..(20): Xaa is Arg, Phe, Glu, Gln, Thr, (D)Arg, (D)Phe, (D)Glu, (D)Thr, (D)Leu, (D)Gln , alpha-MeArg, alpha-MePhe, alpha-MeLeu, alpha-MeLys, alpha-MeAsn, alpha-MeTyr, alpha-MeAsp, or absent
  MOD_RES (21)..(21): Xaa is Arg, Phe, Glu, Gln, Thr, (D)Arg, (D)Phe, (D)Glu, (D)Thr, (D)Leu, (D)Gln , alpha-MeArg, alpha-MePhe, alpha-MeLeu, alpha-MeLys, alpha-MeAsn, alpha-MeTyr, alpha-MeAsp, or absent
  MOD_RES (22)..(22): Xaa is Arg, Phe, Glu, Gln, Thr, (D)Arg, (D)Phe, (D)Glu, (D)Thr, (D)Leu, (D)Gln , alpha-MeArg, alpha-MePhe, alpha-MeLeu, alpha-MeLys, alpha-MeAsn, alpha-MeTyr, alpha-MeAsp, or absent
  MOD_RES (23)..(23): Xaa is Arg, Phe, Glu, Gln, Thr, (D)Arg, (D)Phe, (D)Glu, (D)Thr, (D)Leu, (D)Gln , alpha-MeArg, alpha-MePhe, alpha-MeLeu, alpha-MeLys, alpha-MeAsn, alpha-MeTyr, alpha-MeAsp, or absent
  MOD_RES (24)..(24): Xaa is Arg, Phe, Glu, Gln, Thr, (D)Arg, (D)Phe, (D)Glu, (D)Thr, (D)Leu, (D)Gln , alpha-MeArg, alpha-MePhe, alpha-MeLeu, alpha-MeLys, alpha-MeAsn, alpha-MeTyr, alpha-MeAsp, or absent
XXXXXXXXXXXXXXXXXXXXXXXX

SEQ ID NO: 239 - protein, 20 aa, Homo sapiens
NWQPWSSPFVHQTSQETGKR

SEQ ID NO: 240 - protein, 12 aa, Artificial Sequence
  Synthesized peptide
  MOD_RES (1)..(1): L-Penicillamine
  MOD_RES (6)..(6): L-Penicillamine
  MOD_RES (7)..(7): 4-(2-aminoethoxy)-L-phenylalanine
  MOD_RES (8)..(8): L-2-Napthylalanine
  MOD_RES (9)..(9): Aib
  MOD_RES (10)..(10): ACETYLATION
XNTWQXXXXKNN

SEQ ID NO: 241 - protein, 24 aa, Artificial Sequence
  Synthetic peptide motif
  MOD_RES (1)..(4): Xaa is any amino acid or absent
  MOD_RES (5)..(5): Xaa is Cys, (D)Cys), alpha-MeCys, Pen, (D)Pen, Abu, or (D)Abu
  MOD_RES (6)..(9): Xaa is any amino acid
  MOD_RES (10)..(10): Xaa is Cys, (D)Cys), alpha-MeCys, Pen, (D)Pen, Abu, or (D)Abu
  MOD_RES (11)..(11): Xaa is Phe, Phe[4-(2-aminoethoxy)], Phe[4-(2-acetylaminoethoxy)], alpha-MeTyr, or Phe(4-CONH2)
  MOD_RES (12)..(12): Xaa is Trp, Trp(5-F), 1-Nal, Trp(7-Aza), Phe(2-Me), Phe(3-Me), Phe(4-Me), Phe(3,4-dimethoxy), or 2-Nal
  MOD_RES (13)..(13): Xaa is 4-amino-4-carboxy-tetrahydropyran (THP), alpha-MeLys, alpha-MeLeu, alpha-MeArg, alpha-MePhe, alpha-MeLeu, alpha-MeLys, alpha-MeAsn, alpha-MeTyr, or Aib
  MOD_RES (14)..(14): Xaa is Glu, Cit, Gln, alpha-MeArg, alpha-MeGlu, alpha-MeLeu, alpha-MeLys, alpha-Me-Asn, Lys(Ac), alpha-MeLys(Ac), Dab(Ac), Dap(Ac), homo-Lys(Ac),or Lys
  MOD_RES (15)..(15): Xaa is any amino acid
  MOD_RES (16)..(24): Xaa is any amino acid or absent
XXXXXXXXXXXXXXXXXXXXXXXX

SEQ ID NO: 242 - protein, 4 aa, Artificial Sequence
  Synthesized peptide fragment
QTWQ

SEQ ID NO: 243 - protein, 4 aa, Artificial Sequence
  Synthesized peptide fragment
NDWQ

SEQ ID NO: 244 - protein, 4 aa, Artificial Sequence
  Synthesized peptide fragment
  MOD_RES (2)..(2): L-Diaminobutyric acid
NXWQ

SEQ ID NO: 245 - protein, 4 aa, Artificial Sequence
  Synthesized peptide fragment
  MOD_RES (3)..(3): L-1-Napthylalanine
NTXQ

SEQ ID NO: 246 - protein, 4 aa, Artificial Sequence
  Synthesized peptide fragment
  MOD_RES (3)..(3): L-2-Napthylalanine
NTXQ

SEQ ID NO: 247 - protein, 4 aa, Artificial Sequence
  Synthesized peptide fragment
NTWE

SEQ ID NO: 248 - protein, 4 aa, Artificial Sequence
  Synthesized peptide fragment
NTWF

SEQ ID NO: 249 - protein, 4 aa, Artificial Sequence
  Synthesized peptide fragment
NTWQ

SEQ ID NO: 250 - protein, 4 aa, Artificial Sequence
  Synthesized peptide fragment
  MOD_RES (3)..(3): Trp(5-F)
NTXQ

SEQ ID NO: 251 - protein, 4 aa, Artificial Sequence
  Synthesized peptide fragment
QTWE

SEQ ID NO: 252 - protein, 4 aa, Artificial Sequence
  Synthesized peptide fragment
ETWQ

SEQ ID NO: 253 - protein, 4 aa, Artificial Sequence
  Synthesized peptide fragment
ETWE

SEQ ID NO: 254 - protein, 4 aa, Artificial Sequence
  Synthesized peptide fragment
  MOD_RES (4)..(4): alpha-MeLeu
QTWX

SEQ ID NO: 255 - protein, 4 aa, Artificial Sequence
  Synthesized peptide fragment
  MOD_RES (4)..(4): alpha-MeLys
QTWX

SEQ ID NO: 256 - protein, 4 aa, Artificial Sequence
  Synthesized peptide fragment
  MOD_RES (4)..(4): acetylated alpha-MeLys
QTWX

SEQ ID NO: 257 - protein, 4 aa, Artificial Sequence
  Synthesized peptide fragment
  MOD_RES (4)..(4): D-form glutamine
QTWX

SEQ ID NO: 258 - protein, 4 aa, Artificial Sequence
  Synthesized peptide fragment
  MOD_RES (4)..(4): beta homoglutamine
QTWX

SEQ ID NO: 259 - protein, 4 aa, Artificial Sequence
  Synthesized peptide fragment
QTWF

SEQ ID NO: 260 - protein, 4 aa, Artificial Sequence
  Synthesized peptide fragment
QTWW

SEQ ID NO: 261 - protein, 4 aa, Artificial Sequence
  Synthesized peptide fragment
  MOD_RES (4)..(4): Aib
QTWX

SEQ ID NO: 262 - protein, 4 aa, Artificial Sequence
  Synthesized peptide fragment
QTWT

SEQ ID NO: 263 - protein, 4 aa, Artificial Sequence
  Synthesized peptide fragment
QTWV

SEQ ID NO: 264 - protein, 4 aa, Artificial Sequence
  Synthesized peptide fragment
  MOD_RES (3)..(3): Trp(5-F)
QTXQ

SEQ ID NO: 265 - protein, 24 aa, Artificial Sequence
  Synthetic peptide motif
  MOD_RES (1)..(1): Xaa is Gly, Arg, Phe, Glu, Gln, Thr, (D)Arg, (D)Phe, (D)Glu, (D)Thr, (D)Leu, (D)Gln, alpha-MeArg, alpha-MePhe, alpha-MeLeu, alpha-MeLys, alpha-MeAsn, alpha-MeTyr, or absent
  MOD_RES (2)..(2): Xaa is Gly, Arg, Phe, Glu, Gln, Thr, (D)Arg, (D)Phe, (D)Glu, (D)Thr, (D)Leu, (D)Gln, alpha-MeArg, alpha-MePhe, alpha-MeLeu, alpha-MeLys, alpha-MeAsn, alpha-MeTyr, or absent
  MOD_RES (3)..(3): Xaa is (D)Asp, Arg, (D)Arg, Phe, (D)Phe, 2-Nal, Thr, Leu, (D)Gln, (D)Asn, IsoGlu, Gly, Arg, Phe, Glu, Gln, Thr, (D)Glu, (D)Thr, (D)Leu, alpha-MeArg, alpha-MePhe, alpha-MeLeu, alpha-MeLys, alpha-MeAsn, alpha-MeTyr, or absent
  MOD_RES (4)..(4): Xaa is (D)Arg, (D)Tyr, Gly, alpha-MeArg, alpha-MePhe, alpha-MeLeu, alpha-MeLys, alpha-MeAsn, alpha-MeTyr, or absent
  MOD_RES (5)..(5): Cys, (D)Cys), alpha-MeCys, (D)Pen, or Pen
  MOD_RES (6)..(6): Xaa is Cit, Glu, Gly, Lys, Asn, Pro, alpha-MeGln, alpha-MeLys, alpha-MeLeu, alpha-MeAsn, Lys(Ac), alpha-MeLys(Ac), Dab(Ac), Dap(Ac), homo-Lys(Ac), or Gln
  MOD_RES (7)..(7): Xaa is Thr, Aib, Asp, Dab, Gly, Pro, Ser, alpha-MeGln, alpha-MeLys, alpha-MeLeu, alpha-MeAsn, alpha-MeThr, alpha-MeSer, or Val
  MOD_RES (8)..(8): Xaa is Trp, Trp(5-F), 1-Nal, 2-Nal, Phe(2-Me), Phe(3-Me), Phe(4-Me), Trp(7-Aza), or Phe(3,4-dimethoxy)
  MOD_RES (9)..(9): Xaa is Gln, alpha-Me-Lys, alpha-MeLeu, alpha-MeLys(Ac), beta-homoGln, Cit, Glu, Phe, Asn, Thr, Val, Aib, alpha-MeGln, alpha-MeAsn, Lys(Ac), alpha-MeLys(Ac), Dab(Ac), Dap(Ac), homo-Lys(Ac),or Trp
  MOD_RES (10)..(10): Xaa is Cys, (D)Cys), alpha-MeCys, (D)Pen, or Pen
  MOD_RES (11)..(11): Xaa is Phe, Phe[4-(2-aminoethoxy)], Phe[4-(2-acetylaminoethoxy)], alpha-MeTyr, or Phe(4-CONH2)
  MOD_RES (12)..(12): Xaa is 2-Nal, Trp, Trp(5-F), Trp(7-Aza), Phe(2-Me), Phe(3-Me), Phe(4-Me), Phe(3,4-dimethoxy), or 1-Nal
  MOD_RES (13)..(13): Xaa is 4-amino-4-carboxy-tetrahydropyran (THP), alpha-MeLys, alpha-MeLeu, alpha-MeArg, alpha-MePhe, alpha-MeLeu, alpha-MeLys, alpha-MeAsn, alpha-MeTyr, or Aib
  MOD_RES (14)..(14): Xaa is Glu, Cit, Gln, alpha-MeArg, alpha-MeGlu, alpha-MeLeu, alpha-MeLys, alpha-Me-Asn, Lys(Ac), alpha-MeLys(Ac), Dab(Ac), Dap(Ac), homo-Lys(Ac), or Lys
  MOD_RES (15)..(15): Xaa is Asn, 2-Nap, Aib, Arg, Cit, Asp, Phe, Gly, Lys, Leu, Asn, n-Leu, Gln, Ser, Tic, Trp, alpha-MeGln, alpha-MeAsn, alpha-MeLys(Ac), Dab(Ac), Dap(Ac), homo-Lys(Ac), or Lys(Ac)
  MOD_RES (16)..(16): Xaa is Asn, Aib, beta-Ala, Cit, Gln, Asp, alpha-MeGln, alpha-MeAsn, Lys(Ac), alpha-MeLys(Ac), Dab(Ac), Dap(Ac), homo-Lys(Ac),or absent
  MOD_RES (17)..(17): Xaa is Glu, Phe, Lys, Asn, Trp, Gly, Thr, Pro, (D)Arg, (D)Phe, (D)Glu, (D)Thr, (D)Leu, (D)Gln, alpha-MeArg, alpha-MePhe, alpha-MeLeu, alpha-MeLys, alpha-MeAsn, alpha-MeTyr, alpha-MeAsp, or absent
  MOD_RES (18)..(18): Xaa is Lys, Gly, Pro, The, Phe, Trp, Gln, (D)Arg, (D)Phe, (D)Glu, (D)Thr, (D)Leu, (D)Gln, alpha-MeArg, alpha-MePhe, alpha-MeLeu, alpha-MeLys, alpha-MeAsn, alpha-MeTyr, alpha-MeAsp, or abse
  MOD_RES (19)..(19): Xaa is Gly, Lys, Glu, Phe, Thr, Arg, Gln, (D)Arg, (D)Phe, (D)Glu, (D)Thr, (D)Leu, (D)Gln, alpha-MeArg, alpha-MePhe, alpha-MeLeu, alpha-MeLys, alpha-MeAsn, alpha-MeTyr, alpha-MeAsp, or absent
  MOD_RES (20)..(20): Xaa is Arg, Phe, Glu, Gln, Thr, (D)Arg, (D)Phe, (D)Glu, (D)Thr, (D)Leu, (D)Gln , alpha-MeArg, alpha-MePhe, alpha-MeLeu, alpha-MeLys, alpha-MeAsn, alpha-MeTyr, alpha-MeAsp, or absent
  MOD_RES (21)..(21): Arg, Phe, Glu, Gln, Thr, (D)Arg, (D)Phe, (D)Glu, (D)Thr, (D)Leu, (D)Gln , alpha-MeArg, alpha-MePhe, alpha-MeLeu, alpha-MeLys, alpha-MeAsn, alpha-MeTyr, alpha-MeAsp, or absent
  MOD_RES (22)..(22): Xaa is Arg, Phe, Glu, Gln, Thr, (D)Arg, (D)Phe, (D)Glu, (D)Thr, (D)Leu, (D)Gln , alpha-MeArg, alpha-MePhe, alpha-MeLeu, alpha-MeLys, alpha-MeAsn, alpha-MeTyr, alpha-MeAsp, or absent
  MOD_RES (23)..(23): Xaa is Arg, Phe, Glu, Gln, Thr, (D)Arg, (D)Phe, (D)Glu, (D)Thr, (D)Leu, (D)Gln , alpha-MeArg, alpha-MePhe, alpha-MeLeu, alpha-MeLys, alpha-MeAsn, alpha-MeTyr, alpha-MeAsp, or absent
  MOD_RES (24)..(24): Xaa is Arg, Phe, Glu, Gln, Thr, (D)Arg, (D)Phe, (D)Glu, (D)Thr, (D)Leu, (D)Gln , alpha-MeArg, alpha-MePhe, alpha-MeLeu, alpha-MeLys, alpha-MeAsn, alpha-MeTyr, alpha-MeAsp, or absent
XXXXXXXXXXXXXXXXXXXXXXXX

SEQ ID NO: 266 - protein, 9 aa, Artificial Sequence
  Synthetic peptide motif
  MOD_RES (1)..(1): Pen
  MOD_RES (2)..(2): Xaa is Cit, Glu, Gly, Lys, Asn, Pro, alpha-MeGln, alpha-MeLys, alpha-MeLeu, alpha-MeAsn, Lys(Ac), alpha-MeLys(Ac), Dab(Ac), Dap(Ac), homo-Lys(Ac), or Gln
  MOD_RES (3)..(3): Xaa is Thr, Aib, Asp, Dab, Gly, Pro, Ser, alpha-MeGln, alpha-MeLys, alpha-MeLeu, alpha-MeAsn, alpha-MeThr, alpha-MeSer, or Val
  MOD_RES (4)..(4): Xaa is Trp, Trp(5-F), 1-Nal, 2-Nal, Phe(2-Me), Phe(3-Me), Phe(4-Me), Trp(7-Aza), or Phe(3,4-dimethoxy)
  MOD_RES (5)..(5): Xaa is Gln, alpha-Me-Lys, alpha-MeLeu, alpha-MeLys(Ac), beta-homoGln, Cit, Glu, Phe, Asn, Thr, Val, Aib, alpha-MeGln, alpha-MeAsn, Lys(Ac), alpha-MeLys(Ac), Dab(Ac), Dap(Ac), homo-Lys(Ac),or Trp
  MOD_RES (6)..(6): Pen
  MOD_RES (7)..(7): Phe[4-(2-aminoethoxy)
  MOD_RES (8)..(8): 2-Nal
  MOD_RES (9)..(9): 4-amino-4-carboxy-tetrahydropyran (THP)
XXXXXXXXX

SEQ ID NO: 267 - protein, 10 aa, Artificial Sequence
  Synthetic peptide motif
  MOD_RES (1)..(1): Pen
  MOD_RES (2)..(2): Xaa is Cit, Glu, Gly, Lys, Asn, Pro, alpha-MeGln, alpha-MeLys, alpha-MeLeu, alpha-MeAsn, Lys(Ac), alpha-MeLys(Ac), Dab(Ac), Dap(Ac), homo-Lys(Ac), or Gln
  MOD_RES (3)..(3): Xaa is Thr, Aib, Asp, Dab, Gly, Pro, Ser, alpha-MeGln, alpha-MeLys, alpha-MeLeu, alpha-MeAsn, alpha-MeThr, alpha-MeSer, or Val
  MOD_RES (4)..(4): Xaa is Trp, Trp(5-F), 1-Nal, 2-Nal, Phe(2-Me), Phe(3-Me), Phe(4-Me), Trp(7-Aza), or Phe(3,4-dimethoxy)
  MOD_RES (5)..(5): Xaa is Gln, alpha-Me-Lys, alpha-MeLeu, alpha-MeLys(Ac), beta-homoGln, Cit, Glu, Phe, Asn, Thr, Val, Aib, alpha-MeGln, alpha-MeAsn, Lys(Ac), alpha-MeLys(Ac), Dab(Ac), Dap(Ac), homo-Lys(Ac),or Trp
  MOD_RES (6)..(6): Pen
  MOD_RES (7)..(7): Phe[4-(2-aminoethoxy)
  MOD_RES (9)..(9): alpha-MeLeu
  MOD_RES (10)..(10): ACETYLATION
XXXXXXXWXK

SEQ ID NO: 268 - protein, 10 aa, Artificial Sequence
  Synthetic peptide motif
  MOD_RES (1)..(1): Pen
  MOD_RES (2)..(2): Xaa is Cit, Glu, Gly, Lys, Asn, Pro, alpha-MeGln, alpha-MeLys, alpha-MeLeu, alpha-MeAsn, Lys(Ac), alpha-MeLys(Ac), Dab(Ac), Dap(Ac), homo-Lys(Ac), or Gln
  MOD_RES (3)..(3): Xaa is Thr, Aib, Asp, Dab, Gly, Pro, Ser, alpha-MeGln, alpha-MeLys, alpha-MeLeu, alpha-MeAsn, alpha-MeThr, alpha-MeSer, or Val
  MOD_RES (4)..(4): Xaa is Trp, Trp(5-F), 1-Nal, 2-Nal, Phe(2-Me), Phe(3-Me), Phe(4-Me), Trp(7-Aza), or Phe(3,4-dimethoxy)
  MOD_RES (5)..(5): Xaa is Gln, alpha-Me-Lys, alpha-MeLeu, alpha-MeLys(Ac), beta-homoGln, Cit, Glu, Phe, Asn, Thr, Val, Aib, alpha-MeGln, alpha-MeAsn, Lys(Ac), alpha-MeLys(Ac), Dab(Ac), Dap(Ac), homo-Lys(Ac),or Trp
  MOD_RES (6)..(6): Pen
  MOD_RES (7)..(7): Phe[4-(2-aminoethoxy)
  MOD_RES (8)..(8): 2-Nal
  MOD_RES (9)..(9): alpha-MeLeu
  MOD_RES (10)..(10): ACETYLATION
XXXXXXXXXK

SEQ ID NO: 269 - protein, 10 aa, Artificial Sequence
  Synthetic peptide motif
  MOD_RES (1)..(1): Pen
  MOD_RES (2)..(3): Xaa is any amino acid
  MOD_RES (5)..(5): Xaa is any amino acid
  MOD_RES (6)..(6): Pen
  MOD_RES (7)..(10): xaa is any amino acid
XXXWXXXXXK

SEQ ID NO: 270 - protein, 24 aa, Artificial Sequence
  Synthetic peptide motif
  MOD_RES (1)..(1): Xaa is Gly, Arg, Phe, Glu, Gln, Thr, (D)Arg, (D)Phe, (D)Glu, (D)Thr, (D)Leu, (D)Gln, alpha-MeArg, alpha-MePhe, alpha-MeLeu, alpha-MeLys, alpha-MeAsn, alpha-MeTyr, or absent
  MOD_RES (2)..(2): Xaa is Gly, Arg, Phe, Glu, Gln, Thr, (D)Arg, (D)Phe, (D)Glu, (D)Thr, (D)Leu, (D)Gln, alpha-MeArg, alpha-MePhe, alpha-MeLeu, alpha-MeLys, alpha-MeAsn, alpha-MeTyr, or absent
  MOD_RES (3)..(3): Xaa is (D)Asp, Arg, (D)Arg, Phe, (D)Phe, 2-Nal, Thr, Leu, (D)Gln, (D)Asn, IsoGlu, Gly, Arg, Phe, Glu, Gln, Thr, (D)Glu, (D)Thr, (D)Leu, alpha-MeArg, alpha-MePhe, alpha-MeLeu, alpha-MeLys, alpha-MeAsn, alpha-MeTyr, or absent
  MOD_RES (4)..(4): Xaa is (D)Arg, (D)Tyr, Gly, alpha-MeArg, alpha-MePhe, alpha-MeLeu, alpha-MeLys, alpha-MeAsn, alpha-MeTyr, or absent
  MOD_RES (5)..(5): Xaa is Abu, Cys, (D)Cys), alpha-MeCys, (D)Abu, (D)Pen, or Pen
  MISC_FEATURE (5)..(10): synthesized peptide inhibitor is cyclized via a bond between postions 5 and 10
  MOD_RES (6)..(6): Xaa is Cit, Glu, Gly, Lys, Asn, Pro, alpha-MeGln, alpha-MeLys, alpha-MeLeu, alpha-MeAsn, Lys(Ac), alpha-MeLys(Ac), Dab(Ac), Dap(Ac), homo-Lys(Ac), or Gln
  MOD_RES (7)..(7): Xaa is Thr, Aib, Asp, Dab, Gly, Pro, Ser, alpha-MeGln, alpha-MeLys, alpha-MeLeu, alpha-MeAsn, alpha-MeThr, alpha-MeSer, or Val
  MOD_RES (8)..(8): Xaa is Trp, Trp(5-F), 1-Nal, 2-Nal, Phe(2-Me), Phe(3-Me), Phe(4-Me), Trp(7-Aza), or Phe(3,4-dimethoxy)
  MOD_RES (9)..(9): Xaa is Gln, alpha-Me-Lys, alpha-MeLeu, alpha-MeLys(Ac), beta-homoGln, Cit, Glu, Phe, Asn, Thr, Val, Aib, alpha-MeGln, alpha-MeAsn, Lys(Ac), alpha-MeLys(Ac), Dab(Ac), Dap(Ac), homo-Lys(Ac),or Trp
  MOD_RES (10)..(10): Xaa is Cys, (D)Cys), alpha-MeCys, (D)Abu, (D)Pen, Pen or Abu
  MOD_RES (11)..(11): Xaa is Phe, Phe[4-(2-aminoethoxy)], Phe[4-(2-acetylaminoethoxy)], alpha-MeTyr, or Phe(4-CONH2)
  MOD_RES (12)..(12): Xaa is 2-Nal, Trp, Trp(5-F), Trp(7-Aza), Phe(2-Me), Phe(3-Me), Phe(4-Me), Phe(3,4-dimethoxy), or 1-Nal
  MOD_RES (13)..(13): Xaa is 4-amino-4-carboxy-tetrahydropyran (THP), alpha-MeLys, alpha-MeLeu, alpha-MeArg, alpha-MePhe, alpha-MeLeu, alpha-MeLys, alpha-MeAsn, alpha-MeTyr, or Aib
  MOD_RES (14)..(14): Xaa is Glu, Cit, Gln, alpha-MeArg, alpha-MeGlu, alpha-MeLeu, alpha-MeLys, alpha-Me-Asn, Lys(Ac), alpha-MeLys(Ac), Dab(Ac), Dap(Ac), homo-Lys(Ac), or Lys
  MOD_RES (15)..(15): Xaa is Asn, 2-Nap, Aib, Arg, Cit, Asp, Phe, Gly, Lys, Leu, Asn, n-Leu, Gln, Ser, Tic, Trp, alpha-MeGln, alpha-MeAsn, alpha-MeLys(Ac), Dab(Ac), Dap(Ac), homo-Lys(Ac), or Lys(Ac)
  MOD_RES (16)..(16): Xaa is Asn, Aib, beta-Ala, Cit, Gln, Asp, alpha-MeGln, alpha-MeAsn, Lys(Ac), alpha-MeLys(Ac), Dab(Ac), Dap(Ac), homo-Lys(Ac), or absent
  MOD_RES (17)..(17): Xaa is Glu, Phe, Lys, Asn, Trp, Gly, Thr, Pro, (D)Arg, (D)Phe, (D)Glu, (D)Thr, (D)Leu, (D)Gln, alpha-MeArg, alpha-MePhe, alpha-MeLeu, alpha-MeLys, alpha-MeAsn, alpha-MeTyr, alpha-MeAsp, or absent
  MOD_RES (18)..(18): Xaa is Lys, Gly, Pro, The, Phe, Trp, Gln, (D)Arg, (D)Phe, (D)Glu, (D)Thr, (D)Leu, (D)Gln, alpha-MeArg, alpha-MePhe, alpha-MeLeu, alpha-MeLys, alpha-MeAsn, alpha-MeTyr, alpha-MeAsp, or absent
  MOD_RES (19)..(19): Xaa is Gly, Lys, Glu, Phe, Thr, Arg, Gln, (D)Arg, (D)Phe, (D)Glu, (D)Thr, (D)Leu, (D)Gln, alpha-MeArg, alpha-MePhe, alpha-MeLeu, alpha-MeLys, alpha-MeAsn, alpha-MeTyr, alpha-MeAsp, or absent
  MOD_RES (20)..(20): Xaa is Arg, Phe, Glu, Gln, Thr, (D)Arg, (D)Phe, (D)Glu, (D)Thr, (D)Leu, (D)Gln , alpha-MeArg, alpha-MePhe, alpha-MeLeu, alpha-MeLys, alpha-MeAsn, alpha-MeTyr, alpha-MeAsp, or absent
  MOD_RES (21)..(21): Xaa is Arg, Phe, Glu, Gln, Thr, (D)Arg, (D)Phe, (D)Glu, (D)Thr, (D)Leu, (D)Gln , alpha-MeArg, alpha-MePhe, alpha-MeLeu, alpha-MeLys, alpha-MeAsn, alpha-MeTyr, alpha-MeAsp, or absent
  MOD_RES (22)..(22): Xaa is Arg, Phe, Glu, Gln, Thr, (D)Arg, (D)Phe, (D)Glu, (D)Thr, (D)Leu, (D)Gln , alpha-MeArg, alpha-MePhe, alpha-MeLeu, alpha-MeLys, alpha-MeAsn, alpha-MeTyr, alpha-MeAsp, or absent
  MOD_RES (23)..(23): Xaa is Arg, Phe, Glu, Gln, Thr, (D)Arg, (D)Phe, (D)Glu, (D)Thr, (D)Leu, (D)Gln , alpha-MeArg, alpha-MePhe, alpha-MeLeu, alpha-MeLys, alpha-MeAsn, alpha-MeTyr, alpha-MeAsp, or absent
  MOD_RES (24)..(24): Xaa is Arg, Phe, Glu, Gln, Thr, (D)Arg, (D)Phe, (D)Glu, (D)Thr, (D)Leu, (D)Gln , alpha-MeArg, alpha-MePhe, alpha-MeLeu, alpha-MeLys, alpha-MeAsn, alpha-MeTyr, alpha-MeAsp, or absent
XXXXXXXXXXXXXXXXXXXXXXXX

SEQ ID NO: 271 - protein, 9 aa, Artificial Sequence
  Synthetic peptide motif
  MOD_RES (1)..(1): Abu
  MOD_RES (2)..(2): Xaa is Cit, Glu, Gly, Lys, Asn, Pro, alpha-MeGln, alpha-MeLys, alpha-MeLeu, alpha-MeAsn, Lys(Ac), alpha-MeLys(Ac), Dab(Ac), Dap(Ac), homo-Lys(Ac), or Gln
  MOD_RES (3)..(3): Xaa is Thr, Aib, Asp, Dab, Gly, Pro, Ser, alpha-MeGln, alpha-MeLys, alpha-MeLeu, alpha-MeAsn, alpha-MeThr, alpha-MeSer, or Val
  MOD_RES (4)..(4): Xaa is Trp, Trp(5-F), 1-Nal, 2-Nal, Phe(2-Me), Phe(3-Me), Phe(4-Me), Trp(7-Aza), or Phe(3,4-dimethoxy)
  MOD_RES (5)..(5): Xaa is Gln, alpha-Me-Lys, alpha-MeLeu, alpha-MeLys(Ac), beta-homoGln, Cit, Glu, Phe, Asn, Thr, Val, Aib, alpha-MeGln, alpha-MeAsn, Lys(Ac), alpha-MeLys(Ac), Dab(Ac), Dap(Ac), homo-Lys(Ac),or Trp
  MOD_RES (7)..(7): Phe[4-(2-aminoethoxy)
  MOD_RES (8)..(8): 2-Nal
  MOD_RES (9)..(9): 4-amino-4-carboxy-tetrahydropyran (THP)
XXXXXCXXX

SEQ ID NO: 272 - protein, 10 aa, Artificial Sequence
  Synthetic peptide motif
  MOD_RES (1)..(1): Abu
  MOD_RES (2)..(2): Xaa is Cit, Glu, Gly, Lys, Asn, Pro, alpha-MeGln, alpha-MeLys, alpha-MeLeu, alpha-MeAsn, Lys(Ac), alpha-MeLys(Ac), Dab(Ac), Dap(Ac), homo-Lys(Ac), or Gln
  MOD_RES (3)..(3): Xaa is Thr, Aib, Asp, Dab, Gly, Pro, Ser, alpha-MeGln, alpha-MeLys, alpha-MeLeu, alpha-MeAsn, alpha-MeThr, alpha-MeSer, or Val
  MOD_RES (4)..(4): Xaa is Trp, Trp(5-F), 1-Nal, 2-Nal, Phe(2-Me), Phe(3-Me), Phe(4-Me), Trp(7-Aza), or Phe(3,4-dimethoxy)
  MOD_RES (5)..(5): Xaa is Gln, alpha-Me-Lys, alpha-MeLeu, alpha-MeLys(Ac), beta-homoGln, Cit, Glu, Phe, Asn, Thr, Val, Aib, alpha-MeGln, alpha-MeAsn, Lys(Ac), alpha-MeLys(Ac), Dab(Ac), Dap(Ac), homo-Lys(Ac),or Trp
  MOD_RES (7)..(7): Phe[4-(2-aminoethoxy)
  MOD_RES (9)..(9): alpha-MeLeu
  MOD_RES (10)..(10): ACETYLATION
XXXXXCXWXK

SEQ ID NO: 273 - protein, 10 aa, Artificial Sequence
  Synthetic peptide motif
  MOD_RES (1)..(1): Abu
  MOD_RES (2)..(2): Xaa is Cit, Glu, Gly, Lys, Asn, Pro, alpha-MeGln, alpha-MeLys, alpha-MeLeu, alpha-MeAsn, Lys(Ac), alpha-MeLys(Ac), Dab(Ac), Dap(Ac), homo-Lys(Ac), or Gln
  MOD_RES (3)..(3): Xaa is Thr, Aib, Asp, Dab, Gly, Pro, Ser, alpha-MeGln, alpha-MeLys, alpha-MeLeu, alpha-MeAsn, alpha-MeThr, alpha-MeSer, or Val
  MOD_RES (4)..(4): Xaa is Trp, Trp(5-F), 1-Nal, 2-Nal, Phe(2-Me), Phe(3-Me), Phe(4-Me), Trp(7-Aza), or Phe(3,4-dimethoxy)
  MOD_RES (5)..(5): Xaa is Gln, alpha-Me-Lys, alpha-MeLeu, alpha-MeLys(Ac), beta-homoGln, Cit, Glu, Phe, Asn, Thr, Val, Aib, alpha-MeGln, alpha-MeAsn, Lys(Ac), alpha-MeLys(Ac), Dab(Ac), Dap(Ac), homo-Lys(Ac),or Trp
  MOD_RES (7)..(7): Phe[4-(2-aminoethoxy)
  MOD_RES (8)..(8): 2-Nal
  MOD_RES (9)..(9): alpha-MeLeu
  MOD_RES (10)..(10): ACETYLATION
XXXXXCXXXK

SEQ ID NO: 274 - protein, 11 aa, Artificial Sequence
  Synthesized peptide motif
  MOD_RES (1)..(1): Abu
  MISC_FEATURE (1)..(6): Cyclisized
  MOD_RES (2)..(3): Xaa is any amino acid
  MOD_RES (5)..(5): Xaa is any amino acid
  MOD_RES (7)..(7): Phe[4-(2-aminoethoxy)
  MOD_RES (8)..(8): 2-Nal
  MOD_RES (9)..(11): Xaa is any amino acid
XXXWXCXXXXX

SEQ ID NO: 275 - protein, 15 aa, Artificial Sequence
  Synthesized peptide motif
  MOD_RES (1)..(1): Xaa is Arg, (D)Arg, Gln, or absent
  MOD_RES (2)..(2): Xaa is (D)Arg, Phe, (D)Phe, Lys, (D)Lys, Lys(Y1-Ac), (D)Lys(Y1-Ac), or absent; wherein Y1 is an amino acid, or Y1 is absent
  MOD_RES (3)..(3): Xaa is Cys, (D)Cys), alpha-MeCys, Abu, (D)Pen, Pen, (D)Pensulfoxide, or Pensulfoxide
  MOD_RES (4)..(4): Xaa is Cit, Lys, Asn, Asp, Glu, Lys(Ac), or Gln
  MOD_RES (5)..(5): Xaa is Trp, substituted Trp, or 1-Nal
  MOD_RES (7)..(7): Xaa is Gln, Lys, Lys(Ac), a-MeLeu, Cit, Glu, 1-Nal, 2-Nal, Trp, substituted Trp, or Lys(Peg12)
  MOD_RES (8)..(8): Xaa is Cys, Abu, or Pen
  MOD_RES (9)..(9): Xaa is Phe, Phe[4-(2-aminoethoxy)], Phe(Cmd), or Phe[4-(2-acetylaminoethoxy)]
  MOD_RES (10)..(10): Xaa is 2-Nal, Phe(2-Me), Phe(3-Me), Phe(4-Me), Phe(3,4-dimethoxy), or 1-Nal
  MOD_RES (11)..(11): Xaa is alpha-MeLeu, Aib, Lys, cyclohexylAla, tetrahydropyranAla, Lys(Peg12), or Deg
  MOD_RES (12)..(12): Xaa is Glu, b-homoGlu, Lys, (D)Lys, Lys(Y2-Ac), or (D)Lys(Y2-Ac); wherein Y2 is an amino acid, or Y2 is absent
  MOD_RES (13)..(13): Xaa is Asn, Asp, Cit, or Lys(Ac)
  MOD_RES (14)..(14): Xaa is Asn, Lys, Lys(Ac), Cit, Asp, Gly, Ala, b-Ala, or Sarc
  MOD_RES (15)..(15): Xaa is any amino acid, or absent; substituted Trp is Trp substituted with halo, or azaTrp
XXXXXTXXXXXXXXX

SEQ ID NO: 276 - protein, 14 aa, Artificial Sequence
  Synthesized peptide motif
  MOD_RES (1)..(1): Xaa is (D)Arg, Phe, (D)Phe, Lys, (D)Lys, Lys(Y1-Ac), (D)Lys(Y1-Ac), or absent; wherein Y1 is an amino acid, or Y1 is absent
  MOD_RES (2)..(2): Xaa is Cys, (D)Cys), alpha-MeCys, Abu, (D)Pen, Pen, (D)Pensulfoxide, or Pensulfoxide
  MOD_RES (3)..(3): Xaa is Cit, Lys, Asn, Asp, Glu, Lys(Ac), or Gln
  misc_feature (4)..(4): Xaa can be any naturally occurring amino acid
  MOD_RES (6)..(6): Xaa is Gln, Lys, Lys(Ac), a-MeLeu, Cit, Glu, 1-Nal, 2-Nal, Trp, substituted Trp, or Lys(Peg12)
  MOD_RES (7)..(7): Xaa is Cys, Abu, or Pen
  MOD_RES (8)..(8): Phe[4-(2-aminoethoxy)]
  MOD_RES (9)..(9): 2-Nal
  MOD_RES (10)..(10): Xaa is alpha-MeLeu, Aib, Lys, cyclohexylAla, tetrahydropyranAla, Lys(Peg12), or Deg
  MOD_RES (11)..(11): Xaa is Glu, b-homoGlu, Lys, (D)Lys, Lys(Y2-Ac), or (D)Lys(Y2-Ac); wherein Y2 is an amino acid, or Y2 is absent
  MOD_RES (12)..(12): Xaa is Asn, Asp, Cit, or Lys(Ac)
  MOD_RES (14)..(14): Xaa is any amino acid, or absent; substituted Trp is Trp substituted with halo, or azaTrp
XXXXTWXXXXXXNX

SEQ ID NO: 277 - protein, 14 aa, Artificial Sequence
  Synthesized peptide motif
  MOD_RES (1)..(1): Xaa is (D)Arg, Phe, (D)Phe, Lys, (D)Lys, Lys(Y1-Ac), (D)Lys(Y1-Ac), or absent; wherein Y1 is an amino acid, or Y1 is absent
  MOD_RES (2)..(2): Abu
  MOD_RES (3)..(3): Xaa is Cit, Lys, Asn, Asp, Glu, Lys(Ac), or Gln
  misc_feature (4)..(4): Xaa can be any naturally occurring amino acid
  MOD_RES (6)..(6): Xaa is Gln, Lys, Lys(Ac), a-MeLeu, Cit, Glu, 1-Nal, 2-Nal, Trp, substituted Trp, or Lys(Peg12)
  MOD_RES (7)..(7): Xaa is Cys, Abu, or Pen
  MOD_RES (8)..(8): Phe[4-(2-aminoethoxy)]
  MOD_RES (9)..(9): 2-Nal
  MOD_RES (10)..(10): Xaa is alpha-MeLeu, Aib, Lys, cyclohexylAla, tetrahydropyranAla, Lys(Peg12), or Deg
  MOD_RES (11)..(11): Xaa is Glu, b-homoGlu, Lys, (D)Lys, Lys(Y2-Ac), or (D)Lys(Y2-Ac); wherein Y2 is an amino acid, or Y2 is absent
  MOD_RES (12)..(12): Xaa is Asn, Asp, Cit, or Lys(Ac)
  MOD_RES (14)..(14): Xaa is any amino acid, or absent; substituted Trp is Trp substituted with halo, or azaTrp
XXXXTWXXXXXXNX

SEQ ID NO: 278 - protein, 14 aa, Artificial Sequence
  Synthesized peptide motif
  MOD_RES (1)..(1): Xaa is (D)Arg, Phe, (D)Phe, Lys, (D)Lys, Lys(Y1-Ac), (D)Lys(Y1-Ac), or absent; wherein Y1 is an amino acid, or Y1 is absent
  MOD_RES (2)..(2): Pen
  MOD_RES (3)..(3): Xaa is Cit, Lys, Asn, Asp, Glu, Lys(Ac), or Gln
  misc_feature (4)..(4): Xaa can be any naturally occurring amino acid
  MOD_RES (6)..(6): Xaa is Gln, Lys, Lys(Ac), a-MeLeu, Cit, Glu, 1-Nal, 2-Nal, Trp, substituted Trp, or Lys(Peg12)
  MOD_RES (7)..(7): Xaa is Cys, Abu, or Pen
  MOD_RES (8)..(8): Phe[4-(2-aminoethoxy)]
  MOD_RES (9)..(9): 2-Nal
  MOD_RES (10)..(10): Xaa is alpha-MeLeu, Aib, Lys, cyclohexylAla, tetrahydropyranAla, Lys(Peg12), or Deg
  MOD_RES (11)..(11): Xaa is Glu, b-homoGlu, Lys, (D)Lys, Lys(Y2-Ac), or (D)Lys(Y2-Ac); wherein Y2 is an amino acid, or Y2 is absent
  MOD_RES (12)..(12): Xaa is Asn, Asp, Cit, or Lys(Ac)
  MOD_RES (14)..(14): Xaa is any amino acid, or absent; substituted Trp is Trp substituted with halo, or azaTrp
XXXXTWXXXXXXNX

SEQ ID NO: 279 - protein, 14 aa, Artificial Sequence
  Synthesized peptide motif
  MOD_RES (1)..(1): Xaa is (D)Arg, Phe, (D)Phe, Lys, (D)Lys, Lys(Y1-Ac), (D)Lys(Y1-Ac), or absent; wherein Y1 is an amino acid, or Y1 is absent
  MOD_RES (2)..(2): Abu
  MOD_RES (6)..(6): Xaa is Gln, Lys, Lys(Ac), a-MeLeu, Cit, Glu, 1-Nal, 2-Nal, Trp, substituted Trp, or Lys(Peg12)
  MOD_RES (7)..(7): Xaa is Cys, Abu, or Pen
  MOD_RES (8)..(8): Phe[4-(2-aminoethoxy)]
  MOD_RES (9)..(9): 2-Nal
  MOD_RES (10)..(10): Xaa is alpha-MeLeu, Aib, Lys, cyclohexylAla, tetrahydropyranAla, Lys(Peg12), or Deg
  MOD_RES (11)..(11): Xaa is Glu, b-homoGlu, Lys, (D)Lys, Lys(Y2-Ac), or (D)Lys(Y2-Ac); wherein Y2 is an amino acid, or Y2 is absent
  MOD_RES (12)..(12): Xaa is Asn, Asp, Cit, or Lys(Ac)
  MOD_RES (14)..(14): Xaa is any amino acid, or absent; substituted Trp is Trp substituted with halo, or azaTrp
XXNTWXXXXXXXNX

SEQ ID NO: 280 - protein, 14 aa, Artificial Sequence
  Synthesized peptide motif
  MOD_RES (1)..(1): Xaa is (D)Arg, Phe, (D)Phe, Lys, (D)Lys, Lys(Y1-Ac), (D)Lys(Y1-Ac), or absent; wherein Y1 is an amino acid, or Y1 is absent
  MOD_RES (2)..(2): Pen
  MOD_RES (6)..(6): Xaa is Gln, Lys, Lys(Ac), a-MeLeu, Cit, Glu, 1-Nal, 2-Nal, Trp, substituted Trp, or Lys(Peg12)
  MOD_RES (7)..(7): Xaa is Cys, Abu, or Pen
  MOD_RES (8)..(8): Phe[4-(2-aminoethoxy)]
  MOD_RES (9)..(9): 2-Nal
  MOD_RES (10)..(10): Xaa is alpha-MeLeu, Aib, Lys, cyclohexylAla, tetrahydropyranAla, Lys(Peg12), or Deg
  MOD_RES (11)..(11): Xaa is Glu, b-homoGlu, Lys, (D)Lys, Lys(Y2-Ac), or (D)Lys(Y2-Ac); wherein Y2 is an amino acid, or Y2 is absent
  MOD_RES (12)..(12): Xaa is Asn, Asp, Cit, or Lys(Ac)
  MOD_RES (14)..(14): Xaa is any amino acid, or absent; substituted Trp is Trp substituted with halo, or azaTrp
XXNTWXXXXXXXNX

SEQ ID NO: 281 - protein, 14 aa, Artificial Sequence
  Synthesized peptide motif
  MOD_RES (1)..(1): Xaa is (D)Arg, Phe, (D)Phe, Lys, (D)Lys, Lys(Y1-Ac), (D)Lys(Y1-Ac), or absent; wherein Y1 is an amino acid, or Y1 is absent
  MOD_RES (2)..(2): Abu
  MOD_RES (6)..(6): Xaa is Gln, Lys, Lys(Ac), a-MeLeu, Cit, Glu, 1-Nal, 2-Nal, Trp, substituted Trp, or Lys(Peg12)
  MOD_RES (7)..(7): Xaa is Cys, Abu, or Pen
  MOD_RES (8)..(8): Phe[4-(2-aminoethoxy)]
  MOD_RES (9)..(9): 2-Nal
  MOD_RES (10)..(10): Xaa is alpha-MeLeu, Aib, Lys, cyclohexylAla, tetrahydropyranAla, Lys(Peg12), or Deg
  MOD_RES (11)..(11): Xaa is Glu, b-homoGlu, Lys, (D)Lys, Lys(Y2-Ac), or (D)Lys(Y2-Ac); wherein Y2 is an amino acid, or Y2 is absent
  MOD_RES (12)..(12): Xaa is Asn, Asp, Cit, or Lys(Ac)
  MOD_RES (14)..(14): Xaa is any amino acid, or absent; substituted Trp is Trp substituted with halo, or azaTrp
XXQTWXXXXXXXNX

SEQ ID NO: 282 - protein, 14 aa, Artificial Sequence
  Synthesized peptide motif
  MOD_RES (1)..(1): Xaa is (D)Arg, Phe, (D)Phe, Lys, (D)Lys, Lys(Y1-Ac), (D)Lys(Y1-Ac), or absent; wherein Y1 is an amino acid, or Y1 is absent
  MOD_RES (2)..(2): Pen
  MOD_RES (6)..(6): Xaa is Gln, Lys, Lys(Ac), a-MeLeu, Cit, Glu, 1-Nal, 2-Nal, Trp, substituted Trp, or Lys(Peg12)
  MOD_RES (7)..(7): Xaa is Cys, Abu, or Pen
  MOD_RES (8)..(8): Phe[4-(2-aminoethoxy)]
  MOD_RES (9)..(9): 2-Nal
  MOD_RES (10)..(10): Xaa is alpha-MeLeu, Aib, Lys, cyclohexylAla, tetrahydropyranAla, Lys(Peg12), or Deg
  MOD_RES (11)..(11): Xaa is Glu, b-homoGlu, Lys, (D)Lys, Lys(Y2-Ac), or (D)Lys(Y2-Ac); wherein Y2 is an amino acid, or Y2 is absent
  MOD_RES (12)..(12): Xaa is Asn, Asp, Cit, or Lys(Ac)
  MOD_RES (14)..(14): Xaa is any amino acid, or absent; substituted Trp is Trp substituted with halo, or azaTrp
XXQTWXXXXXXXNX

SEQ ID NO: 283 - protein, 14 aa, Artificial Sequence
  Synthesized peptide motif
  MOD_RES (1)..(1): Xaa is (D)Arg, Phe, (D)Phe, Lys, (D)Lys, Lys(Y1-Ac), (D)Lys(Y1-Ac), or absent; wherein Y1 is an amino acid, or Y1 is absent
  MOD_RES (2)..(2): Abu
  MOD_RES (6)..(6): Xaa is Gln, Lys, Lys(Ac), a-MeLeu, Cit, Glu, 1-Nal, 2-Nal, Trp, substituted Trp, or Lys(Peg12)
  MOD_RES (8)..(8): Phe[4-(2-aminoethoxy)]
  MOD_RES (9)..(9): 2-Nal
  MOD_RES (10)..(10): Xaa is alpha-MeLeu, Aib, Lys, cyclohexylAla, tetrahydropyranAla, Lys(Peg12), or Deg
  MOD_RES (11)..(11): Xaa is Glu, b-homoGlu, Lys, (D)Lys, Lys(Y2-Ac), or (D)Lys(Y2-Ac); wherein Y2 is an amino acid, or Y2 is absent
  MOD_RES (12)..(12): Xaa is Asn, Asp, Cit, or Lys(Ac)
  MOD_RES (14)..(14): Xaa is any amino acid, or absent; substituted Trp is Trp substituted with halo, or azaTrp
XXNTWXCXXXXXNX

SEQ ID NO: 284 - protein, 14 aa, Artificial Sequence
  Synthesized peptide motif
  MOD_RES (1)..(1): Xaa is (D)Arg, Phe, (D)Phe, Lys, (D)Lys, Lys(Y1-Ac), (D)Lys(Y1-Ac), or absent; wherein Y1 is an amino acid, or Y1 is absent
  MOD_RES (2)..(2): Pen
  MOD_RES (6)..(6): Xaa is Gln, Lys, Lys(Ac), a-MeLeu, Cit, Glu, 1-Nal, 2-Nal, Trp, substituted Trp, or Lys(Peg12)
  MOD_RES (8)..(8): Phe[4-(2-aminoethoxy)]
  MOD_RES (9)..(9): 2-Nal
  MOD_RES (10)..(10): Xaa is alpha-MeLeu, Aib, Lys, cyclohexylAla, tetrahydropyranAla, Lys(Peg12), or Deg
  MOD_RES (11)..(11): Xaa is Glu, b-homoGlu, Lys, (D)Lys, Lys(Y2-Ac), or (D)Lys(Y2-Ac); wherein Y2 is an amino acid, or Y2 is absent
  MOD_RES (12)..(12): Xaa is Asn, Asp, Cit, or Lys(Ac)
  MOD_RES (14)..(14): Xaa is any amino acid, or absent; substituted Trp is Trp substituted with halo, or azaTrp
XXNTWXCXXXXXNX

SEQ ID NO: 285 - protein, 14 aa, Artificial Sequence
  Synthesized peptide motif
  MOD_RES (1)..(1): Xaa is (D)Arg, Phe, (D)Phe, Lys, (D)Lys, Lys(Y1-Ac), (D)Lys(Y1-Ac), or absent; wherein Y1 is an amino acid, or Y1 is absent
  MOD_RES (2)..(2): Abu
  MOD_RES (6)..(6): Xaa is Gln, Lys, Lys(Ac), a-MeLeu, Cit, Glu, 1-Nal, 2-Nal, Trp, substituted Trp, or Lys(Peg12)
  MOD_RES (8)..(8): Phe[4-(2-aminoethoxy)]
  MOD_RES (9)..(9): 2-Nal
  MOD_RES (10)..(10): Xaa is alpha-MeLeu, Aib, Lys, cyclohexylAla, tetrahydropyranAla, Lys(Peg12), or Deg
  MOD_RES (11)..(11): Xaa is Glu, b-homoGlu, Lys, (D)Lys, Lys(Y2-Ac), or (D)Lys(Y2-Ac); wherein Y2 is an amino acid, or Y2 is absent
  MOD_RES (12)..(12): Xaa is Asn, Asp, Cit, or Lys(Ac)
  MOD_RES (14)..(14): Xaa is any amino acid, or absent; substituted Trp is Trp substituted with halo, or azaTrp
XXQTWXCXXXXXNX

SEQ ID NO: 286 - protein, 14 aa, Artificial Sequence
  Synthesized peptide motif
  MOD_RES (1)..(1): Xaa is (D)Arg, Phe, (D)Phe, Lys, (D)Lys, Lys(Y1-Ac), (D)Lys(Y1-Ac), or absent; wherein Y1 is an amino acid, or Y1 is absent
  MOD_RES (2)..(2): Pen
  MOD_RES (6)..(6): Xaa is Gln, Lys, Lys(Ac), a-MeLeu, Cit, Glu, 1-Nal, 2-Nal, Trp, substituted Trp, or Lys(Peg12)
  MOD_RES (8)..(8): Phe[4-(2-aminoethoxy)]
  MOD_RES (9)..(9): 2-Nal
  MOD_RES (10)..(10): Xaa is alpha-MeLeu, Aib, Lys, cyclohexylAla, tetrahydropyranAla, Lys(Peg12), or Deg
  MOD_RES (11)..(11): Xaa is Glu, b-homoGlu, Lys, (D)Lys, Lys(Y2-Ac), or (D)Lys(Y2-Ac); wherein Y2 is an amino acid, or Y2 is absent
  MOD_RES (12)..(12): Xaa is Asn, Asp, Cit, or Lys(Ac)
  MOD_RES (14)..(14): Xaa is any amino acid, or absent; substituted Trp is Trp substituted with halo, or azaTrp
XXQTWXCXXXXXNX

SEQ ID NO: 287 - protein, 14 aa, Artificial Sequence
  Synthesized peptide motif
  MOD_RES (1)..(1): Xaa is (D)Arg, Phe, (D)Phe, Lys, (D)Lys, Lys(Y1-Ac), (D)Lys(Y1-Ac), or absent; wherein Y1 is an amino acid, or Y1 is absent
  MOD_RES (2)..(2): Abu
  MOD_RES (6)..(6): Xaa is Gln, Lys, Lys(Ac), a-MeLeu, Cit, Glu, 1-Nal, 2-Nal, Trp, substituted Trp, or Lys(Peg12)
  MOD_RES (7)..(7): Pen
  MOD_RES (8)..(8): Phe[4-(2-aminoethoxy)]
  MOD_RES (9)..(9): 2-Nal
  MOD_RES (10)..(10): Xaa is alpha-MeLeu, Aib, Lys, cyclohexylAla, tetrahydropyranAla, Lys(Peg12), or Deg
  MOD_RES (11)..(11): Xaa is Glu, b-homoGlu, Lys, (D)Lys, Lys(Y2-Ac), or (D)Lys(Y2-Ac); wherein Y2 is an amino acid, or Y2 is absent
  MOD_RES (12)..(12): Xaa is Asn, Asp, Cit, or Lys(Ac)
  MOD_RES (14)..(14): Xaa is any amino acid, or absent; substituted Trp is Trp substituted with halo, or azaTrp
XXNTWXXXXXXXNX

SEQ ID NO: 288 - protein, 14 aa, Artificial Sequence
  Synthesized peptide motif
  MOD_RES (1)..(1): Xaa is (D)Arg, Phe, (D)Phe, Lys, (D)Lys, Lys(Y1-Ac), (D)Lys(Y1-Ac), or absent; wherein Y1 is an amino acid, or Y1 is absent
  MOD_RES (2)..(2): Pen
  MOD_RES (6)..(6): Xaa is Gln, Lys, Lys(Ac), a-MeLeu, Cit, Glu, 1-Nal, 2-Nal, Trp, substituted Trp, or Lys(Peg12)
  MOD_RES (7)..(7): Pen
  MOD_RES (8)..(8): Phe[4-(2-aminoethoxy)]
  MOD_RES (9)..(9): 2-Nal
  MOD_RES (10)..(10): Xaa is alpha-MeLeu, Aib, Lys, cyclohexylAla, tetrahydropyranAla, Lys(Peg12), or Deg
  MOD_RES (11)..(11): Xaa is Glu, b-homoGlu, Lys, (D)Lys, Lys(Y2-Ac), or (D)Lys(Y2-Ac); wherein Y2 is an amino acid, or Y2 is absent
  MOD_RES (12)..(12): Xaa is Asn, Asp, Cit, or Lys(Ac)
  MOD_RES (14)..(14): Xaa is any amino acid, or absent; substituted Trp is Trp substituted with halo, or azaTrp
XXNTWXXXXXXXNX

SEQ ID NO: 289 - protein, 14 aa, Artificial Sequence
  Synthesized peptide motif
  MOD_RES (1)..(1): Xaa is (D)Arg, Phe, (D)Phe, Lys, (D)Lys, Lys(Y1-Ac), (D)Lys(Y1-Ac), or absent; wherein Y1 is an amino acid, or Y1 is absent
  MOD_RES (2)..(2): Abu
  MOD_RES (6)..(6): Xaa is Gln, Lys, Lys(Ac), a-MeLeu, Cit, Glu, 1-Nal, 2-Nal, Trp, substituted Trp, or Lys(Peg12)
  MOD_RES (7)..(7): Pen
  MOD_RES (8)..(8): Phe[4-(2-aminoethoxy)]
  MOD_RES (9)..(9): 2-Nal
  MOD_RES (10)..(10): Xaa is alpha-MeLeu, Aib, Lys, cyclohexylAla, tetrahydropyranAla, Lys(Peg12), or Deg
  MOD_RES (11)..(11): Xaa is Glu, b-homoGlu, Lys, (D)Lys, Lys(Y2-Ac), or (D)Lys(Y2-Ac); wherein Y2 is an amino acid, or Y2 is absent
  MOD_RES (12)..(12): Xaa is Asn, Asp, Cit, or Lys(Ac)
  MOD_RES (14)..(14): Xaa is any amino acid, or absent; substituted Trp is Trp substituted with halo, or azaTrp
XXQTWXXXXXXXNX

SEQ ID NO: 290 - protein, 14 aa, Artificial Sequence
  Synthesized peptide motif
  MOD_RES (1)..(1): Xaa is (D)Arg, Phe, (D)Phe, Lys, (D)Lys, Lys(Y1-Ac), (D)Lys(Y1-Ac), or absent; wherein Y1 is an amino acid, or Y1 is absent
  MOD_RES (2)..(2): Pen
  MOD_RES (6)..(6): Xaa is Gln, Lys, Lys(Ac), a-MeLeu, Cit, Glu, 1-Nal, 2-Nal, Trp, substituted Trp, or Lys(Peg12)
  MOD_RES (7)..(7): Pen
  MOD_RES (8)..(8): Phe[4-(2-aminoethoxy)]
  MOD_RES (9)..(9): 2-Nal
  MOD_RES (10)..(10): Xaa is alpha-MeLeu, Aib, Lys, cyclohexylAla, tetrahydropyranAla, Lys(Peg12), or Deg
  MOD_RES (11)..(11): Xaa is Glu, b-homoGlu, Lys, (D)Lys, Lys(Y2-Ac), or (D)Lys(Y2-Ac); wherein Y2 is an amino acid, or Y2 is absent
  MOD_RES (12)..(12): Xaa is Asn, Asp, Cit, or Lys(Ac)
  MOD_RES (14)..(14): Xaa is any amino acid, or absent; substituted Trp is Trp substituted with halo, or azaTrp
XXQTWXXXXXXXNX

SEQ ID NO: 291 - protein, 14 aa, Artificial Sequence
  Synthesized peptide motif
  MOD_RES (1)..(1): Xaa is (D)Arg, Phe, (D)Phe, Lys, (D)Lys, Lys(Y1-Ac), (D)Lys(Y1-Ac), or absent; wherein Y1 is an amino acid, or Y1 is absent
  MOD_RES (2)..(2): Abu
  MOD_RES (6)..(6): Xaa is Gln, Lys, Lys(Ac), a-MeLeu, Cit, Glu, 1-Nal, 2-Nal, Trp, substituted Trp, or Lys(Peg12)
  MOD_RES (8)..(8): Phe[4-(2-aminoethoxy)]
  MOD_RES (9)..(9): 2-Nal
  MOD_RES (10)..(10): tetrahydropyran Ala
  MOD_RES (11)..(11): Xaa is Glu, b-homoGlu, Lys, (D)Lys, Lys(Y2-Ac), or (D)Lys(Y2-Ac); wherein Y2 is an amino acid, or Y2 is absent
  MOD_RES (14)..(14): Xaa is any amino acid, or absent; substituted Trp is Trp substituted with halo, or azaTrp
XXNTWXCXXXXNNX

SEQ ID NO: 292 - protein, 14 aa, Artificial Sequence
  Synthesized peptide motif
  MOD_RES (1)..(1): Xaa is (D)Arg, Phe, (D)Phe, Lys, (D)Lys, Lys(Y1-Ac), (D)Lys(Y1-Ac), or absent; wherein Y1 is an amino acid, or Y1 is absent
  MOD_RES (2)..(2): Pen
  MOD_RES (6)..(6): Xaa is Gln, Lys, Lys(Ac), a-MeLeu, Cit, Glu, 1-Nal, 2-Nal, Trp, substituted Trp, or Lys(Peg12)
  MOD_RES (8)..(8): Phe[4-(2-aminoethoxy)]
  MOD_RES (9)..(9): 2-Nal
  MOD_RES (10)..(10): tetrahydropyran Ala
  MOD_RES (11)..(11): Xaa is Glu, b-homoGlu, Lys, (D)Lys, Lys(Y2-Ac), or (D)Lys(Y2-Ac); wherein Y2 is an amino acid, or Y2 is absent
  misc_feature (12)..(12): Xaa can be any naturally occurring amino acid
  MOD_RES (14)..(14): Xaa is any amino acid, or absent; substituted Trp is Trp substituted with halo, or azaTrp
XXNTWXCXXXXXNX

SEQ ID NO: 293 - protein, 14 aa, Artificial Sequence
  Synthesized peptide motif
  MOD_RES (1)..(1): Xaa is (D)Arg, Phe, (D)Phe, Lys, (D)Lys, Lys(Y1-Ac), (D)Lys(Y1-Ac), or absent; wherein Y1 is an amino acid, or Y1 is absent
  MOD_RES (2)..(2): Abu
  MOD_RES (6)..(6): Xaa is Gln, Lys, Lys(Ac), a-MeLeu, Cit, Glu, 1-Nal, 2-Nal, Trp, substituted Trp, or Lys(Peg12)
  MOD_RES (8)..(8): Phe[4-(2-aminoethoxy)]
  MOD_RES (9)..(9): 2-Nal
  MOD_RES (10)..(10): tetrahydropyran Ala
  MOD_RES (11)..(11): Xaa is Glu, b-homoGlu, Lys, (D)Lys, Lys(Y2-Ac), or (D)Lys(Y2-Ac); wherein Y2 is an amino acid, or Y2 is absent
  MOD_RES (14)..(14): Xaa is any amino acid, or absent; substituted Trp is Trp substituted with halo, or azaTrp
XXQTWXCXXXXNNX

SEQ ID NO: 294 - protein, 14 aa, Artificial Sequence
  Synthesized peptide motif
  MOD_RES (1)..(1): Xaa is (D)Arg, Phe, (D)Phe, Lys, (D)Lys, Lys(Y1-Ac), (D)Lys(Y1-Ac), or absent; wherein Y1 is an amino acid, or Y1 is absent
  MOD_RES (2)..(2): Pen
  MOD_RES (6)..(6): Xaa is Gln, Lys, Lys(Ac), a-MeLeu, Cit, Glu, 1-Nal, 2-Nal, Trp, substituted Trp, or Lys(Peg12)
  MOD_RES (8)..(8): Phe[4-(2-aminoethoxy)]
  MOD_RES (9)..(9): 2-Nal
  MOD_RES (10)..(10): tetrahydropyran Ala
  MOD_RES (11)..(11): Xaa is Glu, b-homoGlu, Lys, (D)Lys, Lys(Y2-Ac), or (D)Lys(Y2-Ac); wherein Y2 is an amino acid, or Y2 is absent
  misc_feature (12)..(12): Xaa can be any naturally occurring amino acid
  MOD_RES (14)..(14): Xaa is any amino acid, or absent; substituted Trp is Trp substituted with halo, or azaTrp
XXQTWXCXXXXXNX

SEQ ID NO: 295 - protein, 14 aa, Artificial Sequence
  Synthesized peptide motif
  MOD_RES (1)..(1): Xaa is (D)Arg, Phe, (D)Phe, Lys, (D)Lys, Lys(Y1-Ac), (D)Lys(Y1-Ac), or absent; wherein Y1 is an amino acid, or Y1 is absent
  MOD_RES (2)..(2): Abu
  MOD_RES (6)..(6): Xaa is Gln, Lys, Lys(Ac), a-MeLeu, Cit, Glu, 1-Nal, 2-Nal, Trp, substituted Trp, or Lys(Peg12)
  MOD_RES (7)..(7): Pen
  MOD_RES (8)..(8): Phe[4-(2-aminoethoxy)]
  MOD_RES (9)..(9): 2-Nal
  MOD_RES (10)..(10): tetrahydropyran Ala
  MOD_RES (11)..(11): Xaa is Glu, b-homoGlu, Lys, (D)Lys, Lys(Y2-Ac), or (D)Lys(Y2-Ac); wherein Y2 is an amino acid, or Y2 is absent
  misc_feature (12)..(12): Xaa can be any naturally occurring amino acid
  MOD_RES (14)..(14): Xaa is any amino acid, or absent; substituted Trp is Trp substituted with halo, or azaTrp
XXNTWXXXXXXXNX

SEQ ID NO: 296 - protein, 14 aa, Artificial Sequence
  Synthesized peptide motif
  MOD_RES (1)..(1): Xaa is (D)Arg, Phe, (D)Phe, Lys, (D)Lys, Lys(Y1-Ac), (D)Lys(Y1-Ac), or absent; wherein Y1 is an amino acid, or Y1 is absent
  MOD_RES (2)..(2): Pen
  MOD_RES (6)..(6): Xaa is Gln, Lys, Lys(Ac), a-MeLeu, Cit, Glu, 1-Nal, 2-Nal, Trp, substituted Trp, or Lys(Peg12)
  MOD_RES (7)..(7): Pen
  MOD_RES (8)..(8): Phe[4-(2-aminoethoxy)]
  MOD_RES (9)..(9): 2-Nal
  MOD_RES (10)..(10): tetrahydropyran Ala
  MOD_RES (11)..(11): Xaa is Glu, b-homoGlu, Lys, (D)Lys, Lys(Y2-Ac), or (D)Lys(Y2-Ac); wherein Y2 is an amino acid, or Y2 is absent
  misc_feature (12)..(12): Xaa can be any naturally occurring amino acid
  MOD_RES (14)..(14): Xaa is any amino acid, or absent; substituted Trp is Trp substituted with halo, or azaTrp
XXNTWXXXXXXXNX

SEQ ID NO: 297 - protein, 14 aa, Artificial Sequence
  Synthesized peptide motif
  MOD_RES (1)..(1): Xaa is (D)Arg, Phe, (D)Phe, Lys, (D)Lys, Lys(Y1-Ac), (D)Lys(Y1-Ac), or absent; wherein Y1 is an amino acid, or Y1 is absent
  MOD_RES (2)..(2): Abu
  MOD_RES (6)..(6): Xaa is Gln, Lys, Lys(Ac), a-MeLeu, Cit, Glu, 1-Nal, 2-Nal, Trp, substituted Trp, or Lys(Peg12)
  MOD_RES (7)..(7): Pen
  MOD_RES (8)..(8): Phe[4-(2-aminoethoxy)]
  MOD_RES (9)..(9): 2-Nal
  MOD_RES (10)..(10): tetrahydropyran Ala
  MOD_RES (11)..(11): Xaa is Glu, b-homoGlu, Lys, (D)Lys, Lys(Y2-Ac), or (D)Lys(Y2-Ac); wherein Y2 is an amino acid, or Y2 is absent
  misc_feature (12)..(12): Xaa can be any naturally occurring amino acid
  MOD_RES (14)..(14): Xaa is any amino acid, or absent; substituted Trp is Trp substituted with halo, or azaTrp
XXQTWXXXXXXXNX

SEQ ID NO: 298 - protein, 14 aa, Artificial Sequence
  Synthesized peptide motif
  MOD_RES (1)..(1): Xaa is (D)Arg, Phe, (D)Phe, Lys, (D)Lys, Lys(Y1-Ac), (D)Lys(Y1-Ac), or absent; wherein Y1 is an amino acid, or Y1 is absent
  MOD_RES (2)..(2): Pen
  MOD_RES (6)..(6): Xaa is Gln, Lys, Lys(Ac), a-MeLeu, Cit, Glu, 1-Nal, 2-Nal, Trp, substituted Trp, or Lys(Peg12)
  MOD_RES (7)..(7): Pen
  MOD_RES (8)..(8): Phe[4-(2-aminoethoxy)]
  MOD_RES (9)..(9): 2-Nal
  MOD_RES (10)..(10): tetrahydropyran Ala
  MOD_RES (11)..(11): Xaa is Glu, b-homoGlu, Lys, (D)Lys, Lys(Y2-Ac), or (D)Lys(Y2-Ac); wherein Y2 is an amino acid, or Y2 is absent
  misc_feature (12)..(12): Xaa can be any naturally occurring amino acid
  MOD_RES (14)..(14): Xaa is any amino acid, or absent; substituted Trp is Trp substituted with halo, or azaTrp
XXQTWXXXXXXXNX

SEQ ID NO: 299 - protein, 14 aa, Artificial Sequence
  Synthesized peptide motif
  MOD_RES (1)..(1): Xaa is (D)Arg, Phe, (D)Phe, Lys, (D)Lys, Lys(Y1-Ac), (D)Lys(Y1-Ac), or absent; wherein Y1 is an amino acid, or Y1 is absent
  MOD_RES (2)..(2): Abu
  MOD_RES (6)..(6): Xaa is Gln, Lys, Lys(Ac), a-MeLeu, Cit, Glu, 1-Nal, 2-Nal, Trp, substituted Trp, or Lys(Peg12)
  MOD_RES (8)..(8): Phe[4-(2-aminoethoxy)]
  MOD_RES (9)..(9): 2-Nal
  MOD_RES (10)..(10): alpha-MeLeu
  MOD_RES (11)..(11): Xaa is Glu, b-homoGlu, Lys, (D)Lys, Lys(Y2-Ac), or (D)Lys(Y2-Ac); wherein Y2 is an amino acid, or Y2 is absent
  MOD_RES (14)..(14): Xaa is any amino acid, or absent; substituted Trp is Trp substituted with halo, or azaTrp
XXNTWXCXXXXNNX

SEQ ID NO: 300 - protein, 14 aa, Artificial Sequence
  Synthesized peptide motif
  MOD_RES (1)..(1): Xaa is (D)Arg, Phe, (D)Phe, Lys, (D)Lys, Lys(Y1-Ac), (D)Lys(Y1-Ac), or absent; wherein Y1 is an amino acid, or Y1 is absent
  MOD_RES (2)..(2): Pen
  MOD_RES (6)..(6): Xaa is Gln, Lys, Lys(Ac), a-MeLeu, Cit, Glu, 1-Nal, 2-Nal, Trp, substituted Trp, or Lys(Peg12)
  MOD_RES (8)..(8): Phe[4-(2-aminoethoxy)]
  MOD_RES (9)..(9): 2-Nal
  MOD_RES (10)..(10): alpha-MeLeu
  MOD_RES (11)..(11): Xaa is Glu, b-homoGlu, Lys, (D)Lys, Lys(Y2-Ac), or (D)Lys(Y2-Ac); wherein Y2 is an amino acid, or Y2 is absent
  misc_feature (12)..(12): Xaa can be any naturally occurring amino acid
  MOD_RES (14)..(14): Xaa is any amino acid, or absent; substituted Trp is Trp substituted with halo, or azaTrp
XXNTWXCXXXXXNX

SEQ ID NO: 301 - protein, 14 aa, Artificial Sequence
  Synthesized peptide motif
  MOD_RES (1)..(1): Xaa is (D)Arg, Phe, (D)Phe, Lys, (D)Lys, Lys(Y1-Ac), (D)Lys(Y1-Ac), or absent; wherein Y1 is an amino acid, or Y1 is absent
  MOD_RES (2)..(2): Abu
  MOD_RES (6)..(6): Xaa is Gln, Lys, Lys(Ac), a-MeLeu, Cit, Glu, 1-Nal, 2-Nal, Trp, substituted Trp, or Lys(Peg12)
  MOD_RES (8)..(8): Phe[4-(2-aminoethoxy)]
  MOD_RES (9)..(9): 2-Nal
  MOD_RES (10)..(10): alpha-MeLeu
  MOD_RES (11)..(11): Xaa is Glu, b-homoGlu, Lys, (D)Lys, Lys(Y2-Ac), or (D)Lys(Y2-Ac); wherein Y2 is an amino acid, or Y2 is absent
  MOD_RES (14)..(14): Xaa is any amino acid, or absent; substituted Trp is Trp substituted with halo, or azaTrp
XXQTWXCXXXXNNX

SEQ ID NO: 302 - protein, 14 aa, Artificial Sequence
  Synthesized peptide motif
  MOD_RES (1)..(1): Xaa is (D)Arg, Phe, (D)Phe, Lys, (D)Lys, Lys(Y1-Ac), (D)Lys(Y1-Ac), or absent; wherein Y1 is an amino acid, or Y1 is absent
  MOD_RES (2)..(2): Pen
  MOD_RES (6)..(6): Xaa is Gln, Lys, Lys(Ac), a-MeLeu, Cit, Glu, 1-Nal, 2-Nal, Trp, substituted Trp, or Lys(Peg12)
  MOD_RES (8)..(8): Phe[4-(2-aminoethoxy)]
  MOD_RES (9)..(9): 2-Nal
  MOD_RES (10)..(10): alpha-MeLeu
  MOD_RES (11)..(11): Xaa is Glu, b-homoGlu, Lys, (D)Lys, Lys(Y2-Ac), or (D)Lys(Y2-Ac); wherein Y2 is an amino acid, or Y2 is absent
  misc_feature (12)..(12): Xaa can be any naturally occurring amino acid
  MOD_RES (14)..(14): Xaa is any amino acid, or absent; substituted Trp is Trp substituted with halo, or azaTrp
XXQTWXCXXXXXNX

SEQ ID NO: 303 - protein, 14 aa, Artificial Sequence
  Synthesized peptide motif
  MOD_RES (1)..(1): Xaa is (D)Arg, Phe, (D)Phe, Lys, (D)Lys, Lys(Y1-Ac), (D)Lys(Y1-Ac), or absent; wherein Y1 is an amino acid, or Y1 is absent
  MOD_RES (2)..(2): Abu
  MOD_RES (6)..(6): Xaa is Gln, Lys, Lys(Ac), a-MeLeu, Cit, Glu, 1-Nal, 2-Nal, Trp, substituted Trp, or Lys(Peg12)
  MOD_RES (7)..(7): Pen
  MOD_RES (8)..(8): Phe[4-(2-aminoethoxy)]
  MOD_RES (9)..(9): 2-Nal
  MOD_RES (10)..(10): alpha-MeLeu
  MOD_RES (11)..(11): Xaa is Glu, b-homoGlu, Lys, (D)Lys, Lys(Y2-Ac), or (D)Lys(Y2-Ac); wherein Y2 is an amino acid, or Y2 is absent
  misc_feature (12)..(12): Xaa can be any naturally occurring amino acid
  MOD_RES (14)..(14): Xaa is any amino acid, or absent; substituted Trp is Trp substituted with halo, or azaTrp
XXNTWXXXXXXXNX

SEQ ID NO: 304 - protein, 14 aa, Artificial Sequence
  Synthesized peptide motif
  MOD_RES (1)..(1): Xaa is (D)Arg, Phe, (D)Phe, Lys, (D)Lys, Lys(Y1-Ac), (D)Lys(Y1-Ac), or absent; wherein Y1 is an amino acid, or Y1 is absent
  MOD_RES (2)..(2): Pen
  MOD_RES (6)..(6): Xaa is Gln, Lys, Lys(Ac), a-MeLeu, Cit, Glu, 1-Nal, 2-Nal, Trp, substituted Trp, or Lys(Peg12)
  MOD_RES (7)..(7): Pen
  MOD_RES (8)..(8): Phe[4-(2-aminoethoxy)]
  MOD_RES (9)..(9): 2-Nal
  MOD_RES (10)..(10): alpha-MeLeu
  MOD_RES (11)..(11): Xaa is Glu, b-homoGlu, Lys, (D)Lys, Lys(Y2-Ac), or (D)Lys(Y2-Ac); wherein Y2 is an amino acid, or Y2 is absent
  misc_feature (12)..(12): Xaa can be any naturally occurring amino acid
  MOD_RES (14)..(14): Xaa is any amino acid, or absent; substituted Trp is Trp substituted with halo, or azaTrp
XXNTWXXXXXXXNX

SEQ ID NO: 305 - protein, 14 aa, Artificial Sequence
  Synthesized peptide motif
  MOD_RES (1)..(1): Xaa is (D)Arg, Phe, (D)Phe, Lys, (D)Lys, Lys(Y1-Ac), (D)Lys(Y1-Ac), or absent; wherein Y1 is an amino acid, or Y1 is absent
  MOD_RES (2)..(2): Abu
  MOD_RES (6)..(6): Xaa is Gln, Lys, Lys(Ac), a-MeLeu, Cit, Glu, 1-Nal, 2-Nal, Trp, substituted Trp, or Lys(Peg12)
  MOD_RES (7)..(7): Pen
  MOD_RES (8)..(8): Phe[4-(2-aminoethoxy)]
  MOD_RES (9)..(9): 2-Nal
  MOD_RES (10)..(10): alpha-MeLeu
  MOD_RES (11)..(11): Xaa is Glu, b-homoGlu, Lys, (D)Lys, Lys(Y2-Ac), or (D)Lys(Y2-Ac); wherein Y2 is an amino acid, or Y2 is absent
  misc_feature (12)..(12): Xaa can be any naturally occurring amino acid
  MOD_RES (14)..(14): Xaa is any amino acid, or absent; substituted Trp is Trp substituted with halo, or azaTrp
XXQTWXXXXXXXNX

SEQ ID NO: 306 - protein, 14 aa, Artificial Sequence
  Synthesized peptide motif
  MOD_RES (1)..(1): Xaa is (D)Arg, Phe, (D)Phe, Lys, (D)Lys, Lys(Y1-Ac), (D)Lys(Y1-Ac), or absent; wherein Y1 is an amino acid, or Y1 is absent
  MOD_RES (2)..(2): Pen
  MOD_RES (6)..(6): Xaa is Gln, Lys, Lys(Ac), a-MeLeu, Cit, Glu, 1-Nal, 2-Nal, Trp, substituted Trp, or Lys(Peg12)
  MOD_RES (7)..(7): Pen
  MOD_RES (8)..(8): Phe[4-(2-aminoethoxy)]
  MOD_RES (9)..(9): 2-Nal
  MOD_RES (10)..(10): tetrahydropyran Ala
  MOD_RES (10)..(10): alpha-MeLeu
  MOD_RES (11)..(11): Xaa is Glu, b-homoGlu, Lys, (D)Lys, Lys(Y2-Ac), or (D)Lys(Y2-Ac); wherein Y2 is an amino acid, or Y2 is absent
  misc_feature (12)..(12): Xaa can be any naturally occurring amino acid
  MOD_RES (14)..(14): Xaa is any amino acid, or absent; substituted Trp is Trp substituted with halo, or azaTrp
XXQTWXXXXXXXNX

SEQ ID NO: 307 - protein, 12 aa, Artificial Sequence
  Synthesized peptide
  MOD_RES (1)..(1): Penicilamine
  MOD_RES (6)..(6): Penicilamine
  MOD_RES (7)..(7): Phe (4-OMe)
  MOD_RES (8)..(8): 2-Nal
  MOD_RES (9)..(9): alpha-MeLys
  MOD_RES (10)..(10): ACETYLATION
XQTWQXXXXKNG

SEQ ID NO: 308 - protein, 13 aa, Artificial Sequence
  Synthesized peptide
  MOD_RES (1)..(1): D-form arginine
  MOD_RES (2)..(2): Abu
  MISC_FEATURE (2)..(7): residues cyclosized
  MOD_RES (5)..(5): L-2-Napthylalanine
  MOD_RES (8)..(8): 4-(2-aminoethoxy)-L-phenylalanine
  MOD_RES (9)..(9): L-2-Napthylalanine
  MOD_RES (10)..(10): 4-amino-4-carboxy-tetrahydropyran
XXQTXQCXXXENN

SEQ ID NO: 309 - protein, 13 aa, Artificial Sequence
  Synthesized peptide
  MOD_RES (1)..(1): D-form arginine
  MOD_RES (2)..(2): Abu
  MISC_FEATURE (2)..(7): residues cyclosized
  MOD_RES (5)..(5): L-1-Napthylalanine
  MOD_RES (8)..(8): 4-(2-aminoethoxy)-L-phenylalanine
  MOD_RES (9)..(9): L-2-Napthylalanine
  MOD_RES (10)..(10): 4-amino-4-carboxy-tetrahydropyran
XXQTXQCXXXENN

SEQ ID NO: 310 - protein, 13 aa, Artificial Sequence
  Synthesized peptide
  MOD_RES (1)..(1): D-form arginine
  MOD_RES (2)..(2): Abu
  MISC_FEATURE (2)..(7): residues cyclosized
  MOD_RES (5)..(5): 5-Fluoro-L-tryptophan
  MOD_RES (8)..(8): 4-(2-aminoethoxy)-L-phenylalanine
  MOD_RES (9)..(9): L-2-Napthylalanine
  MOD_RES (10)..(10): 4-amino-4-carboxy-tetrahydropyran
XXQTXQCXXXENN